European Patent Specification EP 3 795 591 B1, published September 27, 2023. Title: CYS80 CONJUGATED IMMUNOGLOBULINS. Applicant: EISAI R&D MANAGEMENT CO., LTD. The sequence listing filed with the application follows.

SEQUENCE LISTING (491 sequences)

SEQ ID NO: 1 - DNA, 76 bp, Artificial Sequence
  source: /note="Description of Artificial Sequence: Synthetic primer"
gatcaagcttgccgccaccatgggctggtcctgcatcatcctgtttctggtggcggccgccaccggcgtgcactcc

SEQ ID NO: 2 - DNA, 40 bp, Artificial Sequence
  source: /note="Description of Artificial Sequence: Synthetic primer"
gtgcctttggctggcctgargagayggtgaccagggtgcc

SEQ ID NO: 3 - DNA, 76 bp, Artificial Sequence; identical to SEQ ID NO: 1
  source: /note="Description of Artificial Sequence: Synthetic primer"

SEQ ID NO: 4 - DNA, 31 bp, Artificial Sequence
  source: /note="Description of Artificial Sequence: Synthetic primer"
gatcggcgcgcctcacttgccggggctccgg

SEQ ID NO: 5 - DNA, 41 bp, Artificial Sequence
  source: /note="Description of Artificial Sequence: Synthetic primer"
gccaccggcgtgcactcccagtcggtgraggagtccrgggg

SEQ ID NO: 6 - DNA, 41 bp, Artificial Sequence
  source: /note="Description of Artificial Sequence: Synthetic primer"
gggcccttggtggatgctgargagayggtgaccagggtgcc

SEQ ID NO: 7 - DNA, 42 bp, Artificial Sequence
  source: /note="Description of Artificial Sequence: Synthetic primer"
gccaccggcgtgcactccgagctcgtgatgacccagactcca

SEQ ID NO: 8 - DNA, 33 bp, Artificial Sequence
  source: /note="Description of Artificial Sequence: Synthetic primer"
agccacagttcgtttgacsaccacctcggtccc

SEQ ID NO: 9 - DNA, 24 bp, Artificial Sequence
  source: /note="Description of Artificial Sequence: Synthetic primer"
cagtcgctgctcgagtccgggggt

SEQ ID NO: 10 - DNA, 17 bp, Artificial Sequence
  source: /note="Description of Artificial Sequence: Synthetic primer"
ctctggcacaggagctc

SEQ ID NO: 11 - DNA, 21 bp, Artificial Sequence
  source: /note="Description of Artificial Sequence: Synthetic primer"
ggagacgagcgggtacagagt

SEQ ID NO: 12 - DNA, 20 bp, Artificial Sequence
  source: /note="Description of Artificial Sequence: Synthetic primer"
cgtgggcttgctgcatgtcg

SEQ ID NO: 13 - DNA, 18 bp, Artificial Sequence
  source: /note="Description of Artificial Sequence: Synthetic primer"
gtgatgacccagactcca

SEQ ID NO: 14 - DNA, 25 bp, Artificial Sequence
  source: /note="Description of Artificial Sequence: Synthetic primer"
acagtcacccctattgaagctctgg

SEQ ID NO: 15 - DNA, 24 bp, Artificial Sequence
  source: /note="Description of Artificial Sequence: Synthetic primer"
gcagtcacccctgttgaagctctg

SEQ ID NO: 16 - DNA, 41 bp, Artificial Sequence; identical to SEQ ID NO: 5
  source: /note="Description of Artificial Sequence: Synthetic primer"

SEQ ID NO: 17 - DNA, 41 bp, Artificial Sequence; identical to SEQ ID NO: 6
  source: /note="Description of Artificial Sequence: Synthetic primer"

SEQ ID NO: 18 - DNA, 42 bp, Artificial Sequence; identical to SEQ ID NO: 7
  source: /note="Description of Artificial Sequence: Synthetic primer"

SEQ ID NO: 19 - DNA, 33 bp, Artificial Sequence
  source: /note="Description of Artificial Sequence: Synthetic primer"
agccacagttcgtttgatctccagctcggtccc

SEQ ID NO: 20 - DNA, 33 bp, Artificial Sequence
  source: /note="Description of Artificial Sequence: Synthetic primer"
agccacagttcgtttgatttccacattggtgcc

SEQ ID NO: 21 - DNA, 33 bp, Artificial Sequence; identical to SEQ ID NO: 8
  source: /note="Description of Artificial Sequence: Synthetic primer"

SEQ ID NO: 22 - protein, 14 aa, Oryctolagus cuniculus
DCTYNLSSTLSLTK

SEQ ID NO: 23 - protein, 11 aa, Oryctolagus cuniculus
FTLTITGVQCD

SEQ ID NO: 24 - protein, 10 aa, Artificial Sequence
  source: /note="Description of Artificial Sequence: Synthetic peptide"
FTLTITGVQC

SEQ ID NO: 25 - protein, 9 aa, Artificial Sequence
  source: /note="Description of Artificial Sequence: Synthetic peptide"
TLTITGVQC

SEQ ID NO: 26 - protein, 8 aa, Artificial Sequence
  source: /note="Description of Artificial Sequence: Synthetic peptide"
LTITGVQC

SEQ ID NO: 27 - protein, 7 aa, Artificial Sequence
  source: /note="Description of Artificial Sequence: Synthetic peptide"
TITGVQC

SEQ ID NO: 28 - protein, 6 aa, Artificial Sequence
  source: /note="Description of Artificial Sequence: Synthetic peptide"
ITGVQC

SEQ ID NO: 29 - protein, 5 aa, Artificial Sequence
  source: /note="Description of Artificial Sequence: Synthetic peptide"
TGVQC

SEQ ID NO: 30 - protein, 4 aa, Artificial Sequence
  source: /note="Description of Artificial Sequence: Synthetic peptide"
GVQC

SEQ ID NO: 31 - protein, 2 aa, Artificial Sequence
  source: /note="Description of Artificial Sequence: Synthetic peptide"
QC

SEQ ID NO: 32 - protein, 23 aa, Artificial Sequence
  source: /note="Description of Artificial Sequence: Synthetic peptide"
DIQMTQSPSTLSASVGDRVTITC

SEQ ID NO: 33 - protein, 15 aa, Artificial Sequence
  source: /note="Description of Artificial Sequence: Synthetic peptide"
WYQQKPGKAPKLLIY

SEQ ID NO: 34 - protein, 32 aa, Artificial Sequence
  source: /note="Description of Artificial Sequence: Synthetic polypeptide"
GVPSRFSGSGSGTEFTLTISSLQCDDFATYYC

SEQ ID NO: 35 - protein, 10 aa, Artificial Sequence
  source: /note="Description of Artificial Sequence: Synthetic peptide"
FGGGTKVEIK

SEQ ID NO: 36 - protein, 23 aa, Artificial Sequence
  source: /note="Description of Artificial Sequence: Synthetic peptide"
DIQMTQSPSTVSAAVGGTVTITC

SEQ ID NO: 37 - protein, 32 aa, Artificial Sequence
  source: /note="Description of Artificial Sequence: Synthetic polypeptide"
GVPSRFSGSGSGTEFTLTITGVQCDDFATYYC

SEQ ID NO: 38 - protein, 10 aa, Artificial Sequence
  source: /note="Description of Artificial Sequence: Synthetic peptide"
FGGGTELEIK

SEQ ID NO: 39 - protein, 32 aa, Artificial Sequence
  source: /note="Description of Artificial Sequence: Synthetic polypeptide"
GVPSRFKGSGSGTEFTLTITGVQCDDAATYYC

SEQ ID NO: 40 - protein, 16 aa, Artificial Sequence
  source: /note="Description of Artificial Sequence: Synthetic peptide"
DAEFRHDSGYEVHHQK

SEQ ID NO: 41 - DNA, 2274 bp, Artificial Sequence
  source: /note="Description of Artificial Sequence: Synthetic polynucleotide"
atgctgctgcgcctgttgctggcctgggcggccgcagggcccacactgggccaggacccctgggctgctgagccccgtgccgcctgcggccccagcagctgctacgctctcttcccacggcgccgcaccttcctggaggcctggcgggcctgccgcgagctggggggcgacctggccactcctcggacccccgaggaggcccagcgtgtggacagcctggtgggtgcgggcccagccagccggctgctgtggatcgggctgcagcggcaggcccggcaatgccagctgcagcgcccactgcgcggcttcacgtggaccacaggggaccaggacacggctttcaccaactgggcccagccagcctctggaggcccctgcccggcccagcgctgtgtggccctggaggcaagtggcgagcaccgctggctggagggctcgtgcacgctggctgtcgacggctacctgtgccagtttggcttcgagggcgcctgcccggcgctgcaagatgaggcgggccaggccggcccagccgtgtataccacgcccttccacctggtctccacagagtttgagtggctgcccttcggctctgtggccgctgtgcagtgccaggctggcaggggagcctctctgctctgcgtgaagcagcctgagggaggtgtgggctggtcacgggctgggcccctgtgcctggggactggctgcagccctgacaacgggggctgcgaacacgaatgtgtggaggaggtggatggtcacgtgtcctgccgctgcactgagggcttccggctggcagcagacgggcgcagttgcgaggacccctgtgcccaggctccgtgcgagcagcagtgtgagcccggtgggccacaaggctacagctgccactgtcgcctgggtttccggccagcggaggatgatccgcaccgctgtgtggacacagatgagtgccagattgccggtgtgtgccagcagatgtgtgtcaactacgttggtggcttcgagtgttattgtagcgagggacatgagctggaggctgatggcatcagctgcagccctgcaggggccatgggtgcccaggcttcccaggacctcggagatgagttgctggatgacggggaggatgaggaagatgaagacgaggcctggaaggccttcaacggtggctggacggagatgcctgggatcctgtggatggagcctacgcagccgcctgactttgccctggcctatagaccgagcttcccagaggacagagagccacagataccctacccggagcccacctggccacccccgctcagtgcccccagggtcccctaccactcctcagtgctctccgtcacccggcctgtggtggtctctgccacgcatcccacactgccttctgcccaccagcctcctgtgatccctgccacacacccagctttgtcccgtgaccaccagatccccgtgatcgcagccaactatccagatctgccttctgcctaccaacccggtattctctctgtctctcattcagcacagcctcctgcccaccagccccctatgatctcaaccaaatatccggagctcttccctgcccaccagtcccccatgtttccagacacccgggtcgctggcacccagaccaccactcatttgcctggaatcccacctaaccatgcccctctggtcaccaccctcggtgcccagctaccccctcaagccccagatgcccttgtcctcagaacccaggccacccagcttcccattatcccaactgcccagccctctctgaccaccacctccaggtcccctgtgtctcctgcccatcaaatctctgtgcctgctgccacccagcccgcagccctccccaccctcctgccctctcagagccccactaaccagacctcacccatcagccctacacatccccattccaaagccccccaaatcccaagggaagatggccccagtcccaagttggccctgtggctgccctcaccagctcccacagcagccccaacagccctgggggaggctggtcttgccgagcacagccagagggatgaccggtggctgctggtggcactcctggtgccaacgtgtgtctttttggtggtcctgcttgcactgggcatcgtgtactgcacccgctgtggcccccatgcacccaacaagcgcatcactgactgctatcgctgggtcatccatgctgggagcaagagcccaacagaacccatgccccccaggggcagcctcacaggggtgcagacctgcagaaccagcgtgtga

SEQ ID NO: 42 - protein, 757 aa, Artificial Sequence
  source: /note="Description of Artificial Sequence: Synthetic polypeptide"
MLLRLLLAWAAAGPTLGQDPWAAEPRAACGPSSCYALFPRRRTFLEAWRACRELGGDLATPRTPEEAQRVDSLVGAGPASRLLWIGLQRQARQCQLQRPLRGFTWTTGDQDTAFTNWAQPASGGPCPAQRCVALEASGEHRWLEGSCTLAVDGYLCQFGFEGACPALQDEAGQAGPAVYTTPFHLVSTEFEWLPFGSVAAVQCQAGRGASLLCVKQPEGGVGWSRAGPLCLGTGCSPDNGGCEHECVEEVDGHVSCRCTEGFRLAADGRSCEDPCAQAPCEQQCEPGGPQGYSCHCRLGFRPAEDDPHRCVDTDECQIAGVCQQMCVNYVGGFECYCSEGHELEADGISCSPAGAMGAQASQDLGDELLDDGEDEEDEDEAWKAFNGGWTEMPGILWMEPTQPPDFALAYRPSFPEDREPQIPYPEPTWPPPLSAPRVPYHSSVLSVTRPVVVSATHPTLPSAHQPPVIPATHPALSRDHQIPVIAANYPDLPSAYQPGILSVSHSAQPPAHQPPMISTKYPELFPAHQSPMFPDTRVAGTQTTTHLPGIPPNHAPLVTTLGAQLPPQAPDALVLRTQATQLPIIPTAQPSLTTTSRSPVSPAHQISVPAATQPAALPTLLPSQSPTNQTSPISPTHPHSKAPQIPREDGPSPKLALWLPSPAPTAAPTALGEAGLAEHSQRDDRWLLVALLVPTCVFLVVLLALGIVYCTRCGPHAPNKRITDCYRWVIHAGSKSPTEPMPPRGSLTGVQTCRTSV

SEQ ID NO: 43 - DNA, 2796 bp, Artificial Sequence
  source: /note="Description of Artificial Sequence: Synthetic polynucleotide"
atgctgctgcgcctgttgctggcctgggcggccgcagggcccacactgggccaggacccctgggctgctgagccccgtgccgcctgcggccccagcagctgctacgctctcttcccacggcgccgcaccttcctggaggcctggcgggcctgccgcgagctggggggcgacctggccactcctcggacccccgaggaggcccagcgtgtggacagcctggtgggtgcgggcccagccagccggctgctgtggatcgggctgcagcggcaggcccggcaatgccagctgcagcgcccactgcgcggcttcacgtggaccacaggggaccaggacacggctttcaccaactgggcccagccagcctctggaggcccctgcccggcccagcgctgtgtggccctggaggcaagtggcgagcaccgctggctggagggctcgtgcacgctggctgtcgacggctacctgtgccagtttggcttcgagggcgcctgcccggcgctgcaagatgaggcgggccaggccggcccagccgtgtataccacgcccttccacctggtctccacagagtttgagtggctgcccttcggctctgtggccgctgtgcagtgccaggctggcaggggagcctctctgctctgcgtgaagcagcctgagggaggtgtgggctggtcacgggctgggcccctgtgcctggggactggctgcagccctgacaacgggggctgcgaacacgaatgtgtggaggaggtggatggtcacgtgtcctgccgctgcactgagggcttccggctggcagcagacgggcgcagttgcgaggacccctgtgcccaggctccgtgcgagcagcagtgtgagcccggtgggccacaaggctacagctgccactgtcgcctgggtttccggccagcggaggatgatccgcaccgctgtgtggacacagatgagtgccagattgccggtgtgtgccagcagatgtgtgtcaactacgttggtggcttcgagtgttattgtagcgagggacatgagctggaggctgatggcatcagctgcagccctgcaggggccatgggtgcccaggcttcccaggacctcggagatgagttgctggatgacggggaggatgaggaagatgaagacgaggcctggaaggccttcaacggtggctggacggagatgcctgggatcctgtggatggagcctacgcagccgcctgactttgccctggcctatagaccgagcttcccagaggacagagagccacagataccctacccggagcccacctggccacccccgctcagtgcccccagggtcccctaccactcctcagtgctctccgtcacccggcctgtggtggtctctgccacgcatcccacactgccttctgcccaccagcctcctgtgatccctgccacacacccagctttgtcccgtgaccaccagatccccgtgatcgcagccaactatccagatctgccttctgcctaccaacccggtattctctctgtctctcattcagcacagcctcctgcccaccagccccctatgatctcaaccaaatatccggagctcttccctgcccaccagtcccccatgtttccagacacccgggtcgctggcacccagaccaccactcatttgcctggaatcccacctaaccatgcccctctggtcaccaccctcggtgcccagctaccccctcaagccccagatgcccttgtcctcagaacccaggccacccagcttcccattatcccaactgcccagccctctctgaccaccacctccaggtcccctgtgtctcctgcccatcaaatctctgtgcctgctgccacccagcccgcagccctccccaccctcctgccctctcagagccccactaaccagacctcacccatcagccctacacatccccattccaaagccccccaaatcccaagggaagatggccccagtcccaagttggccctgtggctgccctcaccagctcccacagcagccccaacagccctgggggaggctggtcttgccgagcacagccagagggatgaccgggttaacgacgacgacgacaaagagcccagcggaccaatttcaacaatcaacccctctcctccatccaaggagtctcacaaaagcccagctcctaacctcgagggtggaccatccgtcttcatcttccctccaaatatcaaggatgtactcatgatctccctgacacccaaggtcacgtgtgtggtggtggatgtgagcgaggatgacccagacgtccagatcagctggtttgtgaacaacgtggaagtacacacagcycagacacaaacccatagagaggattacaacagtactatccgggtggtcagcaccctccccatccagcaccaggactggatgagtggcaaggagttcaaatgcaaggtcaacaacaaagacctcccatcacccatcgagagaaccatctcaaaaattaaagggctagtcagagctccacaagtatacatcttgccgccaccagcagagcagttgtccaggaaagatgtcagtctcacttgcctggtcgtgggcttcaaccctggagacatcagtgtggagtggaccagcaatgggcatacagaggagaactacaaggacaccgcaccagtcctggactctgacggttcttacttcatatatagcaagctcaatatgaaaacaagcaagtgggagaaaacagattccttctcatgcaacgtgagacacgagggtctgaaaaattactacctgaagaagaccatctcccggtctccgggtaaatga

SEQ ID NO: 44 - protein, 931 aa, Artificial Sequence
  source: /note="Description of Artificial Sequence: Synthetic polypeptide"
MLLRLLLAWAAAGPTLGQDPWAAEPRAACGPSSCYALFPRRRTFLEAWRACRELGGDLATPRTPEEAQRVDSLVGAGPASRLLWIGLQRQARQCQLQRPLRGFTWTTGDQDTAFTNWAQPASGGPCPAQRCVALEASGEHRWLEGSCTLAVDGYLCQFGFEGACPALQDEAGQAGPAVYTTPFHLVSTEFEWLPFGSVAAVQCQAGRGASLLCVKQPEGGVGWSRAGPLCLGTGCSPDNGGCEHECVEEVDGHVSCRCTEGFRLAADGRSCEDPCAQAPCEQQCEPGGPQGYSCHCRLGFRPAEDDPHRCVDTDECQIAGVCQQMCVNYVGGFECYCSEGHELEADGISCSPAGAMGAQASQDLGDELLDDGEDEEDEDEAWKAFNGGWTEMPGILWMEPTQPPDFALAYRPSFPEDREPQIPYPEPTWPPPLSAPRVPYHSSVLSVTRPVVVSATHPTLPSAHQPPVIPATHPALSRDHQIPVIAANYPDLPSAYQPGILSVSHSAQPPAHQPPMISTKYPELFPAHQSPMFPDTRVAGTQTTTHLPGIPPNHAPLVTTLGAQLPPQAPDALVLRTQATQLPIIPTAQPSLTTTSRSPVSPAHQISVPAATQPAALPTLLPSQSPTNQTSPISPTHPHSKAPQIPREDGPSPKLALWLPSPAPTAAPTALGEAGLAEHSQRDDRVNDDDDKEPSGPISTINPSPPSKESHKSPAPNLEGGPSVFIFPPNIKDVLMISLTPKVTCVVVDVSEDDPDVQISWFVNNVEVHTAQTQTHREDYNSTIRVVSTLPIQHQDWMSGKEFKCKVNNKDLPSPIERTISKIKGLVRAPQVYILPPPAEQLSRKDVSLTCLVVGFNPGDISVEWTSNGHTEENYKDTAPVLDSDGSYFIYSKLNMKTSKWEKTDSFSCNVRHEGLKNYYLKKTISRSPGK

SEQ ID NO: 45 - DNA, 1380 bp, Artificial Sequence
  source: /note="Description of Artificial Sequence: Synthetic polynucleotide"
atggcaccactgtgcccaagcccatggctgccactgctgatcccagcaccagcaccaggactgaccgtgcagctgctgctgagcctgctgctgctggtgcccgtgcacccccagcggctgccccggatgcaggaggacagccccctgggcggcggcagcagcggcgaggacgaccccctgggcgaggaggacctgcccagcgaggaggacagcccccgggaggaggacccccccggagaagaggacctgcccggcgaggaggacctgccaggagaggaggacctgccagaggtgaagccaaagagcgaggaggagggaagcctgaagctggaggacctgccaaccgtggaggcaccaggcgacccacaggagccccagaacaacgcccaccgggacaaggagggcgacgaccagagccactggagatacggaggcgacccaccatggccacgggtgagcccagcatgcgcaggacggttccagagccccgtggacatccggccccagctggccgccttctgccccgccctgcggcccctggagctgctgggcttccagctgccccccctgcccgagctgcggctgcggaacaacggccacagcgtgcagctgaccctgccccccggcctggagatggccctgggccccggccgggagtaccgggccctgcagctgcacctgcactggggcgccgccggccggcccggcagcgagcacaccgtggagggacacaggttcccagcagagatccacgtggtgcacctgagcaccgcattcgcaagggtggacgaggcactgggaaggccaggaggactggcagtgctggcagccttcctggaggagggaccagaggagaacagcgcatacgagcagctgctgagccggctggaggagatcgcagaggagggaagcgagacccaggtgccaggcctggacatcagcgcactgctgccaagcgacttcagccggtacttccagtacgagggcagcctgaccacccccccctgcgcccagggcgtgatctggaccgtgttcaaccagaccgtgatgctgagcgcaaagcagctgcacaccctgagcgacaccctgtggggaccaggcgacagccggctgcagctgaacttcagggcaacccagcccctgaacggaagagtgatcgaggcaagcttcccagcaggagtggacagcagcccaagggcagcagagccagtgcagctgaacagctgcctggcagcaggcgacatcctggcactggtgttcggactgctgttcgcagtgaccagcgtggccttcctggtgcagatgcggcggcagcaccggcggggcaccaagggcggcgtgagctaccggcccgccgaggtggccgagaccggcgcctga

SEQ ID NO: 46 - protein, 459 aa, Artificial Sequence
  source: /note="Description of Artificial Sequence: Synthetic polypeptide"
MAPLCPSPWLPLLIPAPAPGLTVQLLLSLLLLVPVHPQRLPRMQEDSPLGGGSSGEDDPLGEEDLPSEEDSPREEDPPGEEDLPGEEDLPGEEDLPEVKPKSEEEGSLKLEDLPTVEAPGDPQEPQNNAHRDKEGDDQSHWRYGGDPPWPRVSPACAGRFQSPVDIRPQLAAFCPALRPLELLGFQLPPLPELRLRNNGHSVQLTLPPGLEMALGPGREYRALQLHLHWGAAGRPGSEHTVEGHRFPAEIHVVHLSTAFARVDEALGRPGGLAVLAAFLEEGPEENSAYEQLLSRLEEIAEEGSETQVPGLDISALLPSDFSRYFQYEGSLTTPPCAQGVIWTVFNQTVMLSAKQLHTLSDTLWGPGDSRLQLNFRATQPLNGRVIEASFPAGVDSSPRAAEPVQLNSCLAAGDILALVFGLLFAVTSVAFLVQMRRQHRRGTKGGVSYRPAEVAETGA

SEQ ID NO: 47 - DNA, 1203 bp, Artificial Sequence
  source: /note="Description of Artificial Sequence: Synthetic polynucleotide"
atgggctggagctgcatcatcctgttcctggtggcaaccgcaaccggagtgcacagccagaggctgccacggatgcaggaggacagccccctgggcggcggcagcagcggcgaggacgaccccctgggcgaggaggacctgcccagcgaggaggacagcccaagggaggaggacccaccaggagaggaggacctgcctggcgaggaggacctgcctggggaggaggacctgccagaggtgaagccaaagagcgaagaggagggaagcctgaagctggaggacctgccaaccgtggaggcaccaggcgacccacaggagccccagaacaacgcccaccgggacaaggagggcgacgaccagagccactggagatacggaggcgacccaccatggccacgggtgagcccagcatgcgcaggacggttccagagccccgtggacatccggccccagctggccgccttctgccccgccctgcggcccctggagctgctgggcttccagctgccccccctgcccgagctgcggctgcggaacaacggccacagcgtgcagctgaccctgccccccggcctggagatggccctgggccccggccgggagtaccgggccctgcagctgcacctgcactggggcgccgccggccggcccggcagcgagcacaccgtggagggacacaggttcccagcagagatccacgtggtgcacctgagcaccgcattcgcaagggtggacgaggcactgggaaggccaggaggactggcagtgctggcagccttcctggaggagggaccagaggagaacagcgcatacgagcagctgctgagccggctggaggagatcgcagaggagggaagcgagacccaggtgccaggcctggacatcagcgcactgctgccaagcgacttcagccggtacttccagtacgagggcagcctgaccacccccccctgcgcccagggcgtgatctggaccgtgttcaaccagaccgtgatgctgagcgcaaagcagctgcacaccctgagcgacaccctgtggggaccaggcgacagccggctgcagctgaacttcagggcaacccagcccctgaacggaagagtgatcgaggcaagcttcccagcaggagtggacagcagcccaagggcagcagagccagtgcagctgaacagctgcctggccggccaccaccaccaccaccactga

SEQ ID NO: 48 - protein, 400 aa, Artificial Sequence
  source: /note="Description of Artificial Sequence: Synthetic polypeptide"
MGWSCIILFLVATATGVHSQRLPRMQEDSPLGGGSSGEDDPLGEEDLPSEEDSPREEDPPGEEDLPGEEDLPGEEDLPEVKPKSEEEGSLKLEDLPTVEAPGDPQEPQNNAHRDKEGDDQSHWRYGGDPPWPRVSPACAGRFQSPVDIRPQLAAFCPALRPLELLGFQLPPLPELRLRNNGHSVQLTLPPGLEMALGPGREYRALQLHLHWGAAGRPGSEHTVEGHRFPAEIHVVHLSTAFARVDEALGRPGGLAVLAAFLEEGPEENSAYEQLLSRLEEIAEEGSETQVPGLDISALLPSDFSRYFQYEGSLTTPPCAQGVIWTVFNQTVMLSAKQLHTLSDTLWGPGDSRLQLNFRATQPLNGRVIEASFPAGVDSSPRAAEPVQLNSCLAGHHHHHH

SEQ ID NO: 49 - DNA, 1041 bp, Artificial Sequence
  source: /note="Description of Artificial Sequence: Synthetic polynucleotide"
atgggatggagctgtatcatcctcttcttggtagcaacagctacaggtgtacacagcgaagtggagaagacagcctgtccttcaggcaagaaggcccgcgagatagacgagagcctcatcttctacaagaagtgggagctggaagcctgcgtggatgcggccctgctggccacccagatggaccgcgtgaacgccatccccttcacctacgagcagctggacgtcctaaagcataaactggatgagctctacccacaaggttaccccgagtctgtgatccagcacctgggctacctcttcctcaagatgagccctgaggacattcgcaagtggaatgtgacgtccctggagaccctgaaggctttgcttgaagtcaacaaagggcacgaaatgagtcctcaggtggccaccctgatcgaccgctttgtgaagggaaggggccagctagacaaagacaccctagacaccctgaccgccttctaccctgggtacctgtgctccctcagccccgaggagctgagctccgtgccccccagcagcatctgggcggtcaggccccaggacctggacacgtgtgacccaaggcagctggacgtcctctatcccaaggcccgccttgctttccagaacatgaacgggtccgaatacttcgtgaagatccagtccttcctgggtggggcccccacggaggatttgaaggcgctcagtcagcagaatgtgagcatggacttggccacgttcatgaagctgcggacggatgcggtgctgccgttgactgtggctgaggtgcagaaacttctgggaccccacgtggagggcctgaaggcggaggagcggcaccgcccggtgcgggactggatcctacggcagcggcaggacgacctggacacgctggggctggggctacagggcggcatccccaacggctacctggtcctagacctcagcatgcaagaggccctctcggggacgccctgcctcctaggacctggacctgttctcaccgtcctggcactgctcctagcctccaccctggcctga

SEQ ID NO: 50 - protein, 346 aa, Artificial Sequence
  source: /note="Description of Artificial Sequence: Synthetic polypeptide"
MGWSCIILFLVATATGVHSEVEKTACPSGKKAREIDESLIFYKKWELEACVDAALLATQMDRVNAIPFTYEQLDVLKHKLDELYPQGYPESVIQHLGYLFLKMSPEDIRKWNVTSLETLKALLEVNKGHEMSPQVATLIDRFVKGRGQLDKDTLDTLTAFYPGYLCSLSPEELSSVPPSSIWAVRPQDLDTCDPRQLDVLYPKARLAFQNMNGSEYFVKIQSFLGGAPTEDLKALSQQNVSMDLATFMKLRTDAVLPLTVAEVQKLLGPHVEGLKAEERHRPVRDWILRQRQDDLDTLGLGLQGGIPNGYLVLDLSMQEALSGTPCLLGPGPVLTVLALLLASTLA

SEQ ID NO: 51 - DNA, 1416 bp, Artificial Sequence
  source: /note="Description of Artificial Sequence: Synthetic polynucleotide"
atgggctggtcctgcatcatcctgtttctggtggccaccgccaccggcgtgcacagccagtcggtgaaggagtccgggggtcgcctggtcacgcctgggacacccctgacactcacctgcacagtctctggattctccctcaatagctatgcgatgatctgggtccgccaggctccaggggaggggctggaatacatcggattcattactactggtggtaccacatactacgcgagctgggcaaaaggccgattcaccatctccagaacctcgaccacggtggatctgaagctcacccgtccgacaaccgaggacacggccacctatttctgtgccagagatcgggttaaaagctacgatgactatggtgatttagatgctttcgagccctggggcccaggcaccctggtcaccatctcctcagcatccaccaagggcccatcggtcttccccctggcaccctcctccaagagcacctctgggggcacagcggccctgggctgcctggtcaaggactacttccccgaaccggtgacggtgtcgtggaactcaggcgccctgaccagcggcgtgcacaccttcccggctgtcctacagtcctcaggactctactccctcagcagcgtggtgaccgtgccctccagcagcttgggcacccagacctacatctgcaacgtgaatcacaagcccagcaacaccaaggtggacaagaaagttgagcccaaatcttgtgacaaaactcacacatgcccaccgtgcccagcacctgaactcctggggggaccgtcagtcttcctcttccccccaaaacccaaggacaccctcatgatctcccggacccctgaggtcacatgcgtggtggtggacgtgagccacgaagaccctgaggtcaagttcaactggtacgtggacggcgtggaggtgcataatgccaagacaaagccgcgggaggagcagtacaacagcacgtaccgtgtggtcagcgtcctcaccgtcctgcaccaggactggctgaatggcaaggagtacaagtgcaaggtctccaacaaagccctcccagcccccatcgagaaaaccatctccaaagccaaagggcagccccgagaaccacaggtgtacaccctgcccccatcccgggatgagctgaccaagaaccaggtcagcctgacctgcctggtcaaaggcttctatcccagcgacatcgccgtggagtgggagagcaatgggcagccggagaacaactacaagaccacgcctcccgtgctggactccgacggctccttcttcttatattcaaagctcaccgtggacaagagcaggtggcagcaggggaacgtcttctcatgctccgtgatgcatgaggctctgcacaaccactacacgcagaagagcctctccctgtctcccgggaaatga

SEQ ID NO: 52 - protein, 471 aa, Artificial Sequence
  source: /note="Description of Artificial Sequence: Synthetic polypeptide"
MGWSCIILFLVATATGVHSQSVKESGGRLVTPGTPLTLTCTVSGFSLNSYAMIWVRQAPGEGLEYIGFITTGGTTYYASWAKGRFTISRTSTTVDLKLTRPTTEDTATYFCARDRVKSYDDYGDLDAFEPWGPGTLVTISSASTKGPSVFPLAPSSKSTSGGTAALGCLVKDYFPEPVTVSWNSGALTSGVHTFPAVLQSSGLYSLSSVVTVPSSSLGTQTYICNVNHKPSNTKVDKKVEPKSCDKTHTCPPCPAPELLGGPSVFLFPPKPKDTLMISRTPEVTCVVVDVSHEDPEVKFNWYVDGVEVHNAKTKPREEQYNSTYRVVSVLTVLHQDWLNGKEYKCKVSNKALPAPIEKTISKAKGQPREPQVYTLPPSRDELTKNQVSLTCLVKGFYPSDIAVEWESNGQPENNYKTTPPVLDSDGSFFLYSKLTVDKSRWQQGNVFSCSVMHEALHNHYTQKSLSLSPGK

SEQ ID NO: 53 - DNA, 1425 bp, Artificial Sequence
  source: /note="Description of Artificial Sequence: Synthetic polynucleotide"
atgggttggagttgcatcattctgttcctggtggccacagctactggcgtgcactcacaggtgcagctggtggagtccggaggaggactggtgcagccaggtggctctctgcgactgtcttgtagtgcttcaggcttttccctgaacagctacgctatgatctgggtcaggcaggcacctggcaagggcctggaatatatcggattcattaccacaggagggactacctactatgccgactccgtgaaggggagattcactatctctcgcgataacagtaagaataccctgtacctgcagatgaatagcctgagagcagaggacacagccgtgtactattgcgccagggatcgggtgaaatcttacgacgattatggagacctggatgctttcgaaccatggggacaggggaccctggtgacagtgtccagcgcatccaccaagggcccatcggtcttccccctggcaccctcctccaagagcacctctgggggcacagcggccctgggctgcctggtcaaggactacttccccgaaccggtgacggtgtcgtggaactcaggcgccctgaccagcggcgtgcacaccttcccggctgtcctacagtcctcaggactctactccctcagcagcgtggtgaccgtgccctccagcagcttgggcacccagacctacatctgcaacgtgaatcacaagcccagcaacaccaaggtggacaagaaagttgagcccaaatcttgtgacaaaactcacacatgcccaccgtgcccagcacctgaactcctggggggaccgtcagtcttcctcttccccccaaaacccaaggacaccctcatgatctcccggacccctgaggtcacatgcgtggtggtggacgtgagccacgaagaccctgaggtcaagttcaactggtacgtggacggcgtggaggtgcataatgccaagacaaagccgcgggaggagcagtacaacagcacgtaccgtgtggtcagcgtcctcaccgtcctgcaccaggactggctgaatggcaaggagtacaagtgcaaggtctccaacaaagccctcccagcccccatcgagaaaaccatctccaaagccaaagggcagccccgagaaccacaggtgtacaccctgcccccatcccgggatgagctgaccaagaaccaggtcagcctgacctgcctggtcaaaggcttctatcccagcgacatcgccgtggagtgggagagcaatgggcagccggagaacaactacaagaccacgcctcccgtgctggactccgacggctccttcttcttatattcaaagctcaccgtggacaagagcaggtggcagcaggggaacgtcttctcatgctccgtgatgcatgaggctctgcacaaccactacacgcagaagagcctctccctgtctcccgggaaatga

SEQ ID NO: 54 - protein, 474 aa, Artificial Sequence
  source: /note="Description of Artificial Sequence: Synthetic polypeptide"
MGWSCIILFLVATATGVHSQVQLVESGGGLVQPGGSLRLSCSASGFSLNSYAMIWVRQAPGKGLEYIGFITTGGTTYYADSVKGRFTISRDNSKNTLYLQMNSLRAEDTAVYYCARDRVKSYDDYGDLDAFEPWGQGTLVTVSSASTKGPSVFPLAPSSKSTSGGTAALGCLVKDYFPEPVTVSWNSGALTSGVHTFPAVLQSSGLYSLSSVVTVPSSSLGTQTYICNVNHKPSNTKVDKKVEPKSCDKTHTCPPCPAPELLGGPSVFLFPPKPKDTLMISRTPEVTCVVVDVSHEDPEVKFNWYVDGVEVHNAKTKPREEQYNSTYRVVSVLTVLHQDWLNGKEYKCKVSNKALPAPIEKTISKAKGQPREPQVYTLPPSRDELTKNQVSLTCLVKGFYPSDIAVEWESNGQPENNYKTTPPVLDSDGSFFLYSKLTVDKSRWQQGNVFSCSVMHEALHNHYTQKSLSLSPGK

SEQ ID NO: 55 - DNA, 1410 bp, Artificial Sequence
  source: /note="Description of Artificial Sequence: Synthetic polynucleotide"
atgggctggtcctgcatcatcctgtttctggtggccaccgccaccggcgtgcactcccagtcggtggaggagtccgggggagacctggtcaagcctgagggatccctgacactcacctgcacagcctctggattctccttcagtagcagctactggggatgctgggtccgccaggctccagggaaggggcctgagtggatcgcatgcatttatggtggtagtagtggtaccacttattacccgaactgggcgaaaggccgattctccatctccaaaacctcgtcgaccacggtgactctgcaaatggccagtctgacagccgcggacacggccacctatttctgtgcgagagtgactaatggtggtgattgggattttaaattgtggggcccaggcaccctggtcaccatctcctcagcatccaccaagggcccatcggtcttccccctggcaccctcctccaagagcacctctgggggcacagcggccctgggctgcctggtcaaggactacttccccgaaccggtgacggtgtcgtggaactcaggcgccctgaccagcggcgtgcacaccttcccggctgtcctacagtcctcaggactctactccctcagcagcgtggtgaccgtgccctccagcagcttgggcacccagacctacatctgcaacgtgaatcacaagcccagcaacaccaaggtggacaagaaagttgagcccaaatcttgtgacaaaactcacacatgcccaccgtgcccagcacctgaactcctggggggaccgtcagtcttcctcttccccccaaaacccaaggacaccctcatgatctcccggacccctgaggtcacatgcgtggtggtggacgtgagccacgaagaccctgaggtcaagttcaactggtacgtggacggcgtggaggtgcataatgccaagacaaagccgcgggaggagcagtacaacagcacgtaccgtgtggtcagcgtcctcaccgtcctgcaccaggactggctgaatggcaaggagtacaagtgcaaggtctccaacaaagccctcccagcccccatcgagaaaaccatctccaaagccaaagggcagccccgagaaccacaggtgtacaccctgcccccatcccgggatgagctgaccaagaaccaggtcagcctgacctgcctggtcaaaggcttctatcccagcgacatcgccgtggagtgggagagcaatgggcagccggagaacaactacaagaccacgcctcccgtgctggactccgacggctccttcttcttatattcaaagctcaccgtggacaagagcaggtggcagcaggggaacgtcttctcatgctccgtgatgcatgaggctctgcacaaccactacacgcagaagagcctctccctgtctcccgggaaatga

SEQ ID NO: 56 - protein, 469 aa, Artificial Sequence
  source: /note="Description of Artificial Sequence: Synthetic polypeptide"
MGWSCIILFLVATATGVHSQSVEESGGDLVKPEGSLTLTCTASGFSFSSSYWGCWVRQAPGKGPEWIACIYGGSSGTTYYPNWAKGRFSISKTSSTTVTLQMASLTAADTATYFCARVTNGGDWDFKLWGPGTLVTISSASTKGPSVFPLAPSSKSTSGGTAALGCLVKDYFPEPVTVSWNSGALTSGVHTFPAVLQSSGLYSLSSVVTVPSSSLGTQTYICNVNHKPSNTKVDKKVEPKSCDKTHTCPPCPAPELLGGPSVFLFPPKPKDTLMISRTPEVTCVVVDVSHEDPEVKFNWYVDGVEVHNAKTKPREEQYNSTYRVVSVLTVLHQDWLNGKEYKCKVSNKALPAPIEKTISKAKGQPREPQVYTLPPSRDELTKNQVSLTCLVKGFYPSDIAVEWESNGQPENNYKTTPPVLDSDGSFFLYSKLTVDKSRWQQGNVFSCSVMHEALHNHYTQKSLSLSPGK

SEQ ID NO: 57 - DNA, 1407 bp, Artificial Sequence
  source: /note="Description of Artificial Sequence: Synthetic polynucleotide"
atgggctggtcctgcatcatcctgtttctggtggccaccgccaccggcgtgcacagccagtcggtggaggagtccaggggtcgcctggtcacgcctgggacacccctgacactcacctgcacagtctctggaatcgacctcagtaattatgcaatgacctgggtccgccaggctccagggaaggggctggaatggatcggaatcattagtagtaatgataagacatggtacgcgagctgggtgaaaggccggttcaccatctcaaaaacctcgtcgaccacggtggatctgaaaatgaccagtctgacaaccgaggacacggccacctatttctgtgccagagctgctatgcctggtggtttaaagaatgctttcgatccctggggcccaggcaccctggtcaccgtctcttcagcatccaccaagggcccatcggtcttccccctggcaccctcctccaagagcacctctgggggcacagcggccctgggctgcctggtcaaggactacttccccgaaccggtgacggtgtcgtggaactcaggcgccctgaccagcggcgtgcacaccttcccggctgtcctacagtcctcaggactctactccctcagcagcgtggtgaccgtgccctccagcagcttgggcacccagacctacatctgcaacgtgaatcacaagcccagcaacaccaaggtggacaagaaagttgagcccaaatcttgtgacaaaactcacacatgcccaccgtgcccagcacctgaactcctggggggaccgtcagtcttcctcttccccccaaaacccaaggacaccctcatgatctcccggacccctgaggtcacatgcgtggtggtggacgtgagccacgaagaccctgaggtcaagttcaactggtacgtggacggcgtggaggtgcataatgccaagacaaagccgcgggaggagcagtacaacagcacgtaccgtgtggtcagcgtcctcaccgtcctgcaccaggactggctgaatggcaaggagtacaagtgcaaggtctccaacaaagccctcccagcccccatcgagaaaaccatctccaaagccaaagggcagccccgagaaccacaggtgtacaccctgcccccatcccgggatgagctgaccaagaaccaggtcagcctgacctgcctggtcaaaggcttctatcccagcgacatcgccgtggagtgggagagcaatgggcagccggagaacaactacaagaccacgcctcccgtgctggactccgacggctccttcttcttatattcaaagctcaccgtggacaagagcaggtggcagcaggggaacgtcttctcatgctccgtgatgcatgaggctctgcacaaccactacacgcagaagagcctctccctgtctcccgggaaatga

SEQ ID NO: 58 - protein, 468 aa, Artificial Sequence
  source: /note="Description of Artificial Sequence: Synthetic polypeptide"
MGWSCIILFLVATATGVHSQSVEESRGRLVTPGTPLTLTCTVSGIDLSNYAMTWVRQAPGKGLEWIGIISSNDKTWYASWVKGRFTISKTSSTTVDLKMTSLTTEDTATYFCARAAMPGGLKNAFDPWGPGTLVTVSSASTKGPSVFPLAPSSKSTSGGTAALGCLVKDYFPEPVTVSWNSGALTSGVHTFPAVLQSSGLYSLSSVVTVPSSSLGTQTYICNVNHKPSNTKVDKKVEPKSCDKTHTCPPCPAPELLGGPSVFLFPPKPKDTLMISRTPEVTCVVVDVSHEDPEVKFNWYVDGVEVHNAKTKPREEQYNSTYRVVSVLTVLHQDWLNGKEYKCKVSNKALPAPIEKTISKAKGQPREPQVYTLPPSRDELTKNQVSLTCLVKGFYPSDIAVEWESNGQPENNYKTTPPVLDSDGSFFLYSKLTVDKSRWQQGNVFSCSVMHEALHNHYTQKSLSLSPGK

SEQ ID NO: 59 - DNA, 1413 bp, Artificial Sequence
  source: /note="Description of Artificial Sequence: Synthetic polynucleotide"
atgggctggtcctgcatcatcctgtttctggtggccaccgccaccggcgtgcacagcgaggtccagctgctggaatcagggggaggactggtgcagcccggagggtcactgcgactgtcttgtgccgcttcaggcattgatctgtctaactacgctatgacttgggtgaggcaggcacccggcaagggactggagtgggtcggaatcattagctccaatgacaagacctggtacgccgattcagtgaaaggccggttcaccatctctagagacaacagtaagaatacactgtatctgcagatgaacagcctgcgggcagaagatacagccgtctactattgcgctaaagccgctatgcctggcggactgaagaacgcatttgatccttggggacagggaactctggtcaccgtctcatctgcatccaccaagggcccatcggtcttccccctggcaccctcctccaagagcacctctgggggcacagcggccctgggctgcctggtcaaggactacttccccgaaccggtgacggtgtcgtggaactcaggcgccctgaccagcggcgtgcacaccttcccggctgtcctacagtcctcaggactctactccctcagcagcgtggtgaccgtgccctccagcagcttgggcacccagacctacatctgcaacgtgaatcacaagcccagcaacaccaaggtggacaagaaagttgagcccaaatcttgtgacaaaactcacacatgcccaccgtgcccagcacctgaactcctggggggaccgtcagtcttcctcttccccccaaaacccaaggacaccctcatgatctcccggacccctgaggtcacatgcgtggtggtggacgtgagccacgaagaccctgaggtcaagttcaactggtacgtggacggcgtggaggtgcataatgccaagacaaagccgcgggaggagcagtacaacagcacgtaccgtgtggtcagcgtcctcaccgtcctgcaccaggactggctgaatggcaaggagtacaagtgcaaggtctccaacaaagccctcccagcccccatcgagaaaaccatctccaaagccaaagggcagccccgagaaccacaggtgtacaccctgcccccatcccgggatgagctgaccaagaaccaggtcagcctgacctgcctggtcaaaggcttctatcccagcgacatcgccgtggagtgggagagcaatgggcagccggagaacaactacaagaccacgcctcccgtgctggactccgacggctccttcttcttatattcaaagctcaccgtggacaagagcaggtggcagcaggggaacgtcttctcatgctccgtgatgcatgaggctctgcacaaccactacacgcagaagagcctctccctgtctcccgggaaatga

SEQ ID NO: 60 - protein, 470 aa, Artificial Sequence
  source: /note="Description of Artificial Sequence: Synthetic polypeptide"
MGWSCIILFLVATATGVHSEVQLLESGGGLVQPGGSLRLSCAASGIDLSNYAMTWVRQAPGKGLEWVGIISSNDKTWYADSVKGRFTISRDNSKNTLYLQMNSLRAEDTAVYYCAKAAMPGGLKNAFDPWGQGTLVTVSSASTKGPSVFPLAPSSKSTSGGTAALGCLVKDYFPEPVTVSWNSGALTSGVHTFPAVLQSSGLYSLSSVVTVPSSSLGTQTYICNVNHKPSNTKVDKKVEPKSCDKTHTCPPCPAPELLGGPSVFLFPPKPKDTLMISRTPEVTCVVVDVSHEDPEVKFNWYVDGVEVHNAKTKPREEQYNSTYRVVSVLTVLHQDWLNGKEYKCKVSNKALPAPIEKTISKAKGQPREPQVYTLPPSRDELTKNQVSLTCLVKGFYPSDIAVEWESNGQPENNYKTTPPVLDSDGSFFLYSKLTVDKSRWQQGNVFSCSVMHEALHNHYTQKSLSLSPGK

SEQ ID NO: 61 - DNA, 1419 bp, Artificial Sequence
  source: /note="Description of Artificial Sequence: Synthetic polynucleotide"
atgggctggtcctgcatcatcctgtttctggtggccaccgccaccggcgtgcactcccagtcggtggaggagtccgggggtcgcctggtcacgcctgggacacccctgacactcacctgcaccgtctctggaatctccctcagtagcgatgcaataagctgggtccgccaggctccagggaaggggctcgaatacatcggaatcattaatggtggtggtaacacatactacgcgagctgggcgaaaggccgattcaccatctccaaaacctcgaccacggtggatctgaaaatcaccagtccgacaaccgaggacacggccacctatttctgtgccagaggcattcaacatggtggtggtaatagtgattattattattacggcatggacctctggggcccaggcaccctggtcactgtctcttcagcatccaccaagggcccatcggtcttccccctggcaccctcctccaagagcacctctgggggcacagcggccctgggctgcctggtcaaggactacttccccgaaccggtgacggtgtcgtggaactcaggcgccctgaccagcggcgtgcacaccttcccggctgtcctacagtcctcaggactctactccctcagcagcgtggtgaccgtgccctccagcagcttgggcacccagacctacatctgcaacgtgaatcacaagcccagcaacaccaaggtggacaagaaagttgagcccaaatcttgtgacaaaactcacacatgcccaccgtgcccagcacctgaactcctggggggaccgtcagtcttcctcttccccccaaaacccaaggacaccctcatgatctcccggacccctgaggtcacatgcgtggtggtggacgtgagccacgaagaccctgaggtcaagttcaactggtacgtggacggcgtggaggtgcataatgccaagacaaagccgcgggaggagcagtacaacagcacgtaccgtgtggtcagcgtcctcaccgtcctgcaccaggactggctgaatggcaaggagtacaagtgcaaggtctccaacaaagccctcccagcccccatcgagaaaaccatctccaaagccaaagggcagccccgagaaccacaggtgtacaccctgcccccatcccgggatgagctgaccaagaaccaggtcagcctgacctgcctggtcaaaggcttctatcccagcgacatcgccgtggagtgggagagcaatgggcagccggagaacaactacaagaccacgcctcccgtgctggactccgacggctccttcttcttatattcaaagctcaccgtggacaagagcaggtggcagcaggggaacgtcttctcatgctccgtgatgcatgaggctctgcacaaccactacacgcagaagagcctctccctgtctcccgggaaatga

SEQ ID NO: 62 - protein, 472 aa, Artificial Sequence
  source: /note="Description of Artificial Sequence: Synthetic polypeptide"
MGWSCIILFLVATATGVHSQSVEESGGRLVTPGTPLTLTCTVSGISLSSDAISWVRQAPGKGLEYIGIINGGGNTYYASWAKGRFTISKTSTTVDLKITSPTTEDTATYFCARGIQHGGGNSDYYYYGMDLWGPGTLVTVSSASTKGPSVFPLAPSSKSTSGGTAALGCLVKDYFPEPVTVSWNSGALTSGVHTFPAVLQSSGLYSLSSVVTVPSSSLGTQTYICNVNHKPSNTKVDKKVEPKSCDKTHTCPPCPAPELLGGPSVFLFPPKPKDTLMISRTPEVTCVVVDVSHEDPEVKFNWYVDGVEVHNAKTKPREEQYNSTYRVVSVLTVLHQDWLNGKEYKCKVSNKALPAPIEKTISKAKGQPREPQVYTLPPSRDELTKNQVSLTCLVKGFYPSDIAVEWESNGQPENNYKTTPPVLDSDGSFFLYSKLTVDKSRWQQGNVFSCSVMHEALHNHYTQKSLSLSPGK

SEQ ID NO: 63 - DNA, 1428 bp, Artificial Sequence
  source: /note="Description of Artificial Sequence: Synthetic polynucleotide"
atgggctggtcctgcatcatcctgtttctggtggccaccgccaccggcgtgcacagcgaagtccaactggtggaaagcgggggaggactggtgcagccgggcggatccctccggctgtcatgtgctgcatcgggaatttccctctcctccgacgcgattagctgggtcagacaggcccccggaaaggggctggagtacatcggtatcatcaacggcggcggaaacacctactacgcctcctgggccaagggccgcttcaccatctcgcggcataattccaagaacactctgtacttgcaaatgaactccctgagggccgaggacaccgccgtgtactactgcgcgcgcggcatccagcacggtggtggaaacagcgactactactactatgggatggatctgtggggccagggaactcttgtgaccgtgtcgtcagcatccaccaagggcccatcggtcttccccctggcaccctcctccaagagcacctctgggggcacagcggccctgggctgcctggtcaaggactacttccccgaaccggtgacggtgtcgtggaactcaggcgccctgaccagcggcgtgcacaccttcccggctgtcctacagtcctcaggactctactccctcagcagcgtggtgaccgtgccctccagcagcttgggcacccagacctacatctgcaacgtgaatcacaagcccagcaacaccaaggtggacaagaaagttgagcccaaatcttgtgacaaaactcacacatgcccaccgtgcccagcacctgaactcctggggggaccgtcagtcttcctcttccccccaaaacccaaggacaccctcatgatctcccggacccctgaggtcacatgcgtggtggtggacgtgagccacgaagaccctgaggtcaagttcaactggtacgtggacggcgtggaggtgcataatgccaagacaaagccgcgggaggagcagtacaacagcacgtaccgtgtggtcagcgtcctcaccgtcctgcaccaggactggctgaatggcaaggagtacaagtgcaaggtctccaacaaagccctcccagcccccatcgagaaaaccatctccaaagccaaagggcagccccgagaaccacaggtgtacaccctgcccccatcccgggatgagctgaccaagaaccaggtcagcctgacctgcctggtcaaaggcttctatcccagcgacatcgccgtggagtgggagagcaatgggcagccggagaacaactacaagaccacgcctcccgtgctggactccgacggctccttcttcttatattcaaagctcaccgtggacaagagcaggtggcagcaggggaacgtcttctcatgctccgtgatgcatgaggctctgcacaaccactacacgcagaagagcctctccctgtctcccgggaaatga

SEQ ID NO: 64 - protein, 475 aa, Artificial Sequence
  source: /note="Description of Artificial Sequence: Synthetic polypeptide"
MGWSCIILFLVATATGVHSEVQLVESGGGLVQPGGSLRLSCAASGISLSSDAISWVRQAPGKGLEYIGIINGGGNTYYASWAKGRFTISRHNSKNTLYLQMNSLRAEDTAVYYCARGIQHGGGNSDYYYYGMDLWGQGTLVTVSSASTKGPSVFPLAPSSKSTSGGTAALGCLVKDYFPEPVTVSWNSGALTSGVHTFPAVLQSSGLYSLSSVVTVPSSSLGTQTYICNVNHKPSNTKVDKKVEPKSCDKTHTCPPCPAPELLGGPSVFLFPPKPKDTLMISRTPEVTCVVVDVSHEDPEVKFNWYVDGVEVHNAKTKPREEQYNSTYRVVSVLTVLHQDWLNGKEYKCKVSNKALPAPIEKTISKAKGQPREPQVYTLPPSRDELTKNQVSLTCLVKGFYPSDIAVEWESNGQPENNYKTTPPVLDSDGSFFLYSKLTVDKSRWQQGNVFSCSVMHEALHNHYTQKSLSLSPGK

SEQ ID NO: 65 - DNA, 1404 bp, Artificial Sequence
  source: /note="Description of Artificial Sequence: Synthetic polynucleotide"
atgggctggtcctgcatcatcctgtttctggtggccaccgccaccggcgtgcactcccagtcgctggaggagtccgggggtcgcctggtcacgcctgggacacccctgacactcacctgcacagcctctggattctccctcagtaactatgcaatgacctgggtccgccaggctccagggaaggggctagaatacatcggaatcattagtactggcggtatcacatactatatggactcggcaaaaggccgattcaccatctccagaacctcgaccacggtggatctgaaaatgaccagtctgacaaccgaggacacggccacctatttctgtggcagaaatgctggtggtagttatattttctattattttgacttgtggggccaaggcaccctggtcactgtctcttcagcatccaccaagggcccatcggtcttccccctggcaccctcctccaagagcacctctgggggcacagcggccctgggctgcctggtcaaggactacttccccgaaccggtgacggtgtcgtggaactcaggcgccctgaccagcggcgtgcacaccttcccggctgtcctacagtcctcaggactctactccctcagcagcgtggtgaccgtgccctccagcagcttgggcacccagacctacatctgcaacgtgaatcacaagcccagcaacaccaaggtggacaagaaagttgagcccaaatcttgtgacaaaactcacacatgcccaccgtgcccagcacctgaactcctggggggaccgtcagtcttcctcttccccccaaaacccaaggacaccctcatgatctcccggacccctgaggtcacatgcgtggtggtggacgtgagccacgaagaccctgaggtcaagttcaactggtacgtggacggcgtggaggtgcataatgccaagacaaagccgcgggaggagcagtacaacagcacgtaccgtgtggtcagcgtcctcaccgtcctgcaccaggactggctgaatggcaaggagtacaagtgcaaggtctccaacaaagccctcccagcccccatcgagaaaaccatctccaaagccaaagggcagccccgagaaccacaggtgtacaccctgcccccatcccgggatgagctgaccaagaaccaggtcagcctgacctgcctggtcaaaggcttctatcccagcgacatcgccgtggagtgggagagcaatgggcagccggagaacaactacaagaccacgcctcccgtgctggactccgacggctccttcttcttatattcaaagctcaccgtggacaagagcaggtggcagcaggggaacgtcttctcatgctccgtgatgcatgaggctctgcacaaccactacacgcagaagagcctctccctgtctcccgggaaatga

SEQ ID NO: 66 - protein, 467 aa, Artificial Sequence
  source: /note="Description of Artificial Sequence: Synthetic polypeptide"
MGWSCIILFLVATATGVHSQSLEESGGRLVTPGTPLTLTCTASGFSLSNYAMTWVRQAPGKGLEYIGIISTGGITYYMDSAKGRFTISRTSTTVDLKMTSLTTEDTATYFCGRNAGGSYIFYYFDLWGQGTLVTVSSASTKGPSVFPLAPSSKSTSGGTAALGCLVKDYFPEPVTVSWNSGALTSGVHTFPAVLQSSGLYSLSSVVTVPSSSLGTQTYICNVNHKPSNTKVDKKVEPKSCDKTHTCPPCPAPELLGGPSVFLFPPKPKDTLMISRTPEVTCVVVDVSHEDPEVKFNWYVDGVEVHNAKTKPREEQYNSTYRVVSVLTVLHQDWLNGKEYKCKVSNKALPAPIEKTISKAKGQPREPQVYTLPPSRDELTKNQVSLTCLVKGFYPSDIAVEWESNGQPENNYKTTPPVLDSDGSFFLYSKLTVDKSRWQQGNVFSCSVMHEALHNHYTQKSLSLSPGK

SEQ ID NO: 67 - DNA, 1404 bp, Artificial Sequence
  source: /note="Description of Artificial Sequence: Synthetic polynucleotide"
atgggctggtcctgcatcatcctgtttctggtggccaccgccaccggcgtgcactcccagtcgttggaggagtccgggggtcgcctggtcacgcctgggacacccctgacactcacctgcacagcctctggattctccctcagtaactatgcaatgacctgggtccgccaggctccagggaaggggctagaatacatcggaatcattagtactggcggtatcacatactatatggactcggcaaaaggccgattcaccatctccagaacctcgaccacggtggatctgaaaatgaccagtctgacaaccgaggacacggccacctatttctgtggcagaaatgctggtggtagttatattttctattatttcgacttgtggggccaagggaccctcgtcactgtctcttcagcatccaccaagggcccatcggtcttccccctggcaccctcctccaagagcacctctgggggcacagcggccctgggctgcctggtcaaggactacttccccgaaccggtgacggtgtcgtggaactcaggcgccctgaccagcggcgtgcacaccttcccggctgtcctacagtcctcaggactctactccctcagcagcgtggtgaccgtgccctccagcagcttgggcacccagacctacatctgcaacgtgaatcacaagcccagcaacaccaaggtggacaagaaagttgagcccaaatcttgtgacaaaactcacacatgcccaccgtgcccagcacctgaactcctggggggaccgtcagtcttcctcttccccccaaaacccaaggacaccctcatgatctcccggacccctgaggtcacatgcgtggtggtggacgtgagccacgaagaccctgaggtcaagttcaactggtacgtggacggcgtggaggtgcataatgccaagacaaagccgcgggaggagcagtacaacagcacgtaccgtgtggtcagcgtcctcaccgtcctgcaccaggactggctgaatggcaaggagtacaagtgcaaggtctccaacaaagccctcccagcccccatcgagaaaaccatctccaaagccaaagggcagccccgagaaccacaggtgtacaccctgcccccatcccgggatgagctgaccaagaaccaggtcagcctgacctgcctggtcaaaggcttctatcccagcgacatcgccgtggagtgggagagcaatgggcagccggagaacaactacaagaccacgcctcccgtgctggactccgacggctccttcttcttatattcaaagctcaccgtggacaagagcaggtggcagcaggggaacgtcttctcatgctccgtgatgcatgaggctctgcacaaccactacacgcagaagagcctctccctgtctcccgggaaatga

SEQ ID NO: 68 - protein, 467 aa, Artificial Sequence; identical to SEQ ID NO: 66
  source: /note="Description of Artificial Sequence: Synthetic polypeptide"

SEQ ID NO: 69 - DNA, 1389 bp, Artificial Sequence
  source: /note="Description of Artificial Sequence: Synthetic polynucleotide"
atgggctggtcctgcatcatcctgtttctggtggccaccgccaccggcgtgcactcccagtcgctggaggagtccgggggtcgcctggtcgcgcctgggacacccctgacactcacctgcacagtctctggattctccctcagtagttaccacatgagctgggtccgccaggctccaggggaggggctggaatggatcggaggcattactgctatgagtcgcacatactacgcgagctgggcgaaaggccgattcaccatctccaaaacctcgaccacggtccatctgaaaatcaccagtccgacaaccgaggacacggccacctatttctgtgccagggaacctggttttgttagtaacatctggggcccaggcaccctggtcaccgtctccttagcatccaccaagggcccatcggtcttccccctggcaccctcctccaagagcacctctgggggcacagcggccctgggctgcctggtcaaggactacttccccgaaccggtgacggtgtcgtggaactcaggcgccctgaccagcggcgtgcacaccttcccggctgtcctacagtcctcaggactctactccctcagcagcgtggtgaccgtgccctccagcagcttgggcacccagacctacatctgcaacgtgaatcacaagcccagcaacaccaaggtggacaagaaagttgagcccaaatcttgtgacaaaactcacacatgcccaccgtgcccagcacctgaactcctggggggaccgtcagtcttcctcttccccccaaaacccaaggacaccctcatgatctcccggacccctgaggtcacatgcgtggtggtggacgtgagccacgaagaccctgaggtcaagttcaactggtacgtggacggcgtggaggtgcataatgccaagacaaagccgcgggaggagcagtacaacagcacgtaccgtgtggtcagcgtcctcaccgtcctgcaccaggactggctgaatggcaaggagtacaagtgcaaggtctccaacaaagccctcccagcccccatcgagaaaaccatctccaaagccaaagggcagccccgagaaccacaggtgtacaccctgcccccatcccgggatgagctgaccaagaaccaggtcagcctgacctgcctggtcaaaggcttctatcccagcgacatcgccgtggagtgggagagcaatgggcagccggagaacaactacaagaccacgcctcccgtgctggactccgacggctccttcttcttatattcaaagctcaccgtggacaagagcaggtggcagcaggggaacgtcttctcatgctccgtgatgcatgaggctctgcacaaccactacacgcagaagagcctctccctgtctcccgggaaatga

SEQ ID NO: 70 - protein, 462 aa, Artificial Sequence
  source: /note="Description of Artificial Sequence: Synthetic polypeptide"
MGWSCIILFLVATATGVHSQSLEESGGRLVAPGTPLTLTCTVSGFSLSSYHMSWVRQAPGEGLEWIGGITAMSRTYYASWAKGRFTISKTSTTVHLKITSPTTEDTATYFCAREPGFVSNIWGPGTLVTVSLASTKGPSVFPLAPSSKSTSGGTAALGCLVKDYFPEPVTVSWNSGALTSGVHTFPAVLQSSGLYSLSSVVTVPSSSLGTQTYICNVNHKPSNTKVDKKVEPKSCDKTHTCPPCPAPELLGGPSVFLFPPKPKDTLMISRTPEVTCVVVDVSHEDPEVKFNWYVDGVEVHNAKTKPREEQYNSTYRVVSVLTVLHQDWLNGKEYKCKVSNKALPAPIEKTISKAKGQPREPQVYTLPPSRDELTKNQVSLTCLVKGFYPSDIAVEWESNGQPENNYKTTPPVLDSDGSFFLYSKLTVDKSRWQQGNVFSCSVMHEALHNHYTQKSLSLSPGK

SEQ ID NO: 71 - DNA, 1404 bp, Artificial Sequence
  source: /note="Description of Artificial Sequence: Synthetic polynucleotide"
atgggctggtcctgcatcatcctgtttctggtggccaccgccaccggcgtgcactcccagtcggtggaggagtccgggggtcgcctggtcacgcctgggacacccctgacactcacctgcacagtctctggattctccctcagtagctatgcaatgggctgggtccgccaggctccaggggaggggctggaatggatcggaaccattagtactggtggtattacatactacgcgagctgggcgaaaggccgattcaccatctccaaaacctcgaccacggtggatctgaaaatcaccagtccgacaaccgaggacacggccacctatttctgtgccagagtgggtagtagtggttatcttttctacttctttaacttgtggggccaaggcaccctcgtcactgtctcctcagcatccaccaagggcccatcggtcttccccctggcaccctcctccaagagcacctctgggggcacagcggccctgggctgcctggtcaaggactacttccccgaaccggtgacggtgtcgtggaactcaggcgccctgaccagcggcgtgcacaccttcccggctgtcctacagtcctcaggactctactccctcagcagcgtggtgaccgtgccctccagcagcttgggcacccagacctacatctgcaacgtgaatcacaagcccagcaacaccaaggtggacaagaaagttgagcccaaatcttgtgacaaaactcacacatgcccaccgtgcccagcacctgaactcctggggggaccgtcagtcttcctcttccccccaaaacccaaggacaccctcatgatctcccggacccctgaggtcacatgcgtggtggtggacgtgagccacgaagaccctgaggtcaagttcaactggtacgtggacggcgtggaggtgcataatgccaagacaaagccgcgggaggagcagtacaacagcacgtaccgtgtggtcagcgtcctcaccgtcctgcaccaggactggctgaatggcaaggagtacaagtgcaaggtctccaacaaagccctcccagcccccatcgagaaaaccatctccaaagccaaagggcagccccgagaaccacaggtgtacaccctgcccccatcccgggatgagctgaccaagaaccaggtcagcctgacctgcctggtcaaaggcttctatcccagcgacatcgccgtggagtgggagagcaatgggcagccggagaacaactacaagaccacgcctcccgtgctggactccgacggctccttcttcttatattcaaagctcaccgtggacaagagcaggtggcagcaggggaacgtcttctcatgctccgtgatgcatgaggctctgcacaaccactacacgcagaagagcctctccctgtctcccgggaaatga

SEQ ID NO: 72 - protein, 467 aa, Artificial Sequence
  source: /note="Description of Artificial Sequence: Synthetic polypeptide"
MGWSCIILFLVATATGVHSQSVEESGGRLVTPGTPLTLTCTVSGFSLSSYAMGWVRQAPGEGLEWIGTISTGGITYYASWAKGRFTISKTSTTVDLKITSPTTEDTATYFCARVGSSGYLFYFFNLWGQGTLVTVSSASTKGPSVFPLAPSSKSTSGGTAALGCLVKDYFPEPVTVSWNSGALTSGVHTFPAVLQSSGLYSLSSVVTVPSSSLGTQTYICNVNHKPSNTKVDKKVEPKSCDKTHTCPPCPAPELLGGPSVFLFPPKPKDTLMISRTPEVTCVVVDVSHEDPEVKFNWYVDGVEVHNAKTKPREEQYNSTYRVVSVLTVLHQDWLNGKEYKCKVSNKALPAPIEKTISKAKGQPREPQVYTLPPSRDELTKNQVSLTCLVKGFYPSDIAVEWESNGQPENNYKTTPPVLDSDGSFFLYSKLTVDKSRWQQGNVFSCSVMHEALHNHYTQKSLSLSPGK

SEQ ID NO: 73 - DNA, 1419 bp, Artificial Sequence
  source: /note="Description of Artificial Sequence: Synthetic polynucleotide"
atgggctggtcctgcatcatcctgtttctggtggccaccgccaccggcgtgcacagccagtcggtgaaggagtccaggggtcgcctggtcacgcctgggacacccctgacactcacctgcacagtctctggattctccctcagtaggtatacattgatctgggtccgccaggctccagggaaggggctggaatggatcggaatcatagatagtagtagtagtgcatactacgcgaggtgggcgaaaggccgattcaccatctccaaaacctcgaccacggtggatctgaaaatcaccagtccgacaaccgaggacacggccacctatttctgtgccagagacagagtcctaagctacgatgactatggtgatttgcccgatggtttcgatccctggggcccaggcaccctggtcaccgtctcctcagcatccaccaagggcccatcggtcttccccctggcaccctcctccaagagcacctctgggggcacagcggccctgggctgcctggtcaaggactacttccccgaaccggtgacggtgtcgtggaactcaggcgccctgaccagcggcgtgcacaccttcccggctgtcctacagtcctcaggactctactccctcagcagcgtggtgaccgtgccctccagcagcttgggcacccagacctacatctgcaacgtgaatcacaagcccagcaacaccaaggtggacaagaaagttgagcccaaatcttgtgacaaaactcacacatgcccaccgtgcccagcacctgaactcctggggggaccgtcagtcttcctcttccccccaaaacccaaggacaccctcatgatctcccggacccctgaggtcacatgcgtggtggtggacgtgagccacgaagaccctgaggtcaagttcaactggtacgtggacggcgtggaggtgcataatgccaagacaaagccgcgggaggagcagtacaacagcacgtaccgtgtggtcagcgtcctcaccgtcctgcaccaggactggctgaatggcaaggagtacaagtgcaaggtctccaacaaagccctcccagcccccatcgagaaaaccatctccaaagccaaagggcagccccgagaaccacaggtgtacaccctgcccccatcccgggatgagctgaccaagaaccaggtcagcctgacctgcctggtcaaaggcttctatcccagcgacatcgccgtggagtgggagagcaatgggcagccggagaacaactacaagaccacgcctcccgtgctggactccgacggctccttcttcttatattcaaagctcaccgtggacaagagcaggtggcagcaggggaacgtcttctcatgctccgtgatgcatgaggctctgcacaaccactacacgcagaagagcctctccctgtctcccgggaaatga

SEQ ID NO: 74 - protein, 472 aa, Artificial Sequence
  source: /note="Description of Artificial Sequence: Synthetic polypeptide"
MGWSCIILFLVATATGVHSQSVKESRGRLVTPGTPLTLTCTVSGFSLSRYTLIWVRQAPGKGLEWIGIIDSSSSAYYARWAKGRFTISKTSTTVDLKITSPTTEDTATYFCARDRVLSYDDYGDLPDGFDPWGPGTLVTVSSASTKGPSVFPLAPSSKSTSGGTAALGCLVKDYFPEPVTVSWNSGALTSGVHTFPAVLQSSGLYSLSSVVTVPSSSLGTQTYICNVNHKPSNTKVDKKVEPKSCDKTHTCPPCPAPELLGGPSVFLFPPKPKDTLMISRTPEVTCVVVDVSHEDPEVKFNWYVDGVEVHNAKTKPREEQYNSTYRVVSVLTVLHQDWLNGKEYKCKVSNKALPAPIEKTISKAKGQPREPQVYTLPPSRDELTKNQVSLTCLVKGFYPSDIAVEWESNGQPENNYKTTPPVLDSDGSFFLYSKLTVDKSRWQQGNVFSCSVMHEALHNHYTQKSLSLSPGK

SEQ ID NO: 75 - DNA, 1428 bp, Artificial Sequence
  source: /note="Description of Artificial Sequence: Synthetic polynucleotide"
atgggctggtcctgcatcatcctgtttctggtggccaccgccaccggcgtgcacagcgaagtgcagctggtcgaatctggaggaggactggtgcagcctggagggagcctgagactgagttgcgcagcaagcgggtttagcctgtcccgatacaccctgatctgggtgagacaggcccccggcaagggactggagtgggtctctatcattgacagctcctctagtgcctactatgctgatagtgtgaagggcaggttcaccatttcacgcgacaacgctaaaaatagcctgtatctgcagatgaactccctgcgggcagaagacacagccgtgtactattgcgcacgggatagagtcctgagctacgacgattatggggacctgcctgacggctttgatccttggggacagggaactctggtgacagtgagcagcgcatccaccaagggcccatcggtcttccccctggcaccctcctccaagagcacctctgggggcacagcggccctgggctgcctggtcaaggactacttccccgaaccggtgacggtgtcgtggaactcaggcgccctgaccagcggcgtgcacaccttcccggctgtcctacagtcctcaggactctactccctcagcagcgtggtgaccgtgccctccagcagcttgggcacccagacctacatctgcaacgtgaatcacaagcccagcaacaccaaggtggacaagaaagttgagcccaaatcttgtgacaaaactcacacatgcccaccgtgcccagcacctgaactcctggggggaccgtcagtcttcctcttccccccaaaacccaaggacaccctcatgatctcccggacccctgaggtcacatgcgtggtggtggacgtgagccacgaagaccctgaggtcaagttcaactggtacgtggacggcgtggaggtgcataatgccaagacaaagccgcgggaggagcagtacaacagcacgtaccgtgtggtcagcgtcctcaccgtcctgcaccaggactggctgaatggcaaggagtacaagtgcaaggtctccaacaaagccctcccagcccccatcgagaaaaccatctccaaagccaaagggcagccccgagaaccacaggtgtacaccctgcccccatcccgggatgagctgaccaagaaccaggtcagcctgacctgcctggtcaaaggcttctatcccagcgacatcgccgtggagtgggagagcaatgggcagccggagaacaactacaagaccacgcctcccgtgctggactccgacggctccttcttcttatattcaaagctcaccgtggacaagagcaggtggcagcaggggaacgtcttctcatgctccgtgatgcatgaggctctgcacaaccactacacgcagaagagcctctccctgtctcccgggaaatga

SEQ ID NO: 76 - protein, 475 aa, Artificial Sequence
  source: /note="Description of Artificial Sequence: Synthetic polypeptide"
MGWSCIILFLVATATGVHSEVQLVESGGGLVQPGGSLRLSCAASGFSLSRYTLIWVRQAPGKGLEWVSIIDSSSSAYYADSVKGRFTISRDNAKNSLYLQMNSLRAEDTAVYYCARDRVLSYDDYGDLPDGFDPWGQGTLVTVSSASTKGPSVFPLAPSSKSTSGGTAALGCLVKDYFPEPVTVSWNSGALTSGVHTFPAVLQSSGLYSLSSVVTVPSSSLGTQTYICNVNHKPSNTKVDKKVEPKSCDKTHTCPPCPAPELLGGPSVFLFPPKPKDTLMISRTPEVTCVVVDVSHEDPEVKFNWYVDGVEVHNAKTKPREEQYNSTYRVVSVLTVLHQDWLNGKEYKCKVSNKALPAPIEKTISKAKGQPREPQVYTLPPSRDELTKNQVSLTCLVKGFYPSDIAVEWESNGQPENNYKTTPPVLDSDGSFFLYSKLTVDKSRWQQGNVFSCSVMHEALHNHYTQKSLSLSPGK

SEQ ID NO: 77 - DNA, 714 bp, Artificial Sequence
  source: /note="Description of Artificial Sequence: Synthetic polynucleotide"
atgggctggtcctgcatcatcctgtttctggtggccaccgccaccggcgtgcacagcgagctcgtgatgacccagactccatcctccgtgtctgcagctgtgggaggcacagtcaccatcaattgccaggccagtcagagcattagtagctacttagcctggtatcagcagaaaccagggcagcctcccaagctcctgatctattatgcatccactctggcgtctggggtcccatcgcggttcaaaggcagtggctctgggacagagttcactctcaccatcaccggcgtgcagtgtgacgatgctgccacttactactgtctaggtgtttatggttatagttttgatgatggtattgctttcggcggagggaccgagctggagatcaaacgaactgtggctgcaccatctgtcttcatcttcccgccatctgatgagcagttgaaatctggaactgcctctgttgtgtgcctgctgaataacttctatcccagagaggccaaagtacagtggaaggtggataacgccctccaatcgggtaactcccaggagagtgtcacagagcaggacagcaaggacagcacctacagcctcagcagcaccctgacgctgagcaaagcagactacgagaaacacaaagtctacgcctgcgaagtcacccatcagggcctgagctcgcccgtcacaaagagcttcaacaggggagagtgttga

SEQ ID NO: 78 - protein, 237 aa, Artificial Sequence
  source: /note="Description of Artificial Sequence: Synthetic polypeptide"
MGWSCIILFLVATATGVHSELVMTQTPSSVSAAVGGTVTINCQASQSISSYLAWYQQKPGQPPKLLIYYASTLASGVPSRFKGSGSGTEFTLTITGVQCDDAATYYCLGVYGYSFDDGIAFGGGTELEIKRTVAAPSVFIFPPSDEQLKSGTASVVCLLNNFYPREAKVQWKVDNALQSGNSQESVTEQDSKDSTYSLSSTLTLSKADYEKHKVYACEVTHQGLSSPVTKSFNRGEC

SEQ ID NO: 79 - DNA, 714 bp, Artificial Sequence
  source: /note="Description of Artificial Sequence: Synthetic polynucleotide"
atggggtggtcttgcatcattctgttcctggtggcaaccgccacaggtgtgcactccgacatccagatgactcagagtccatcaaccctgtccgctagcgtgggagatagagtgactatcacctgtcaggcctctcagagtatttccagctacctggcttggtatcagcagaagccaggcaaagcacccaagctgctgatctactatgctagtacactggcatcaggagtgccttcccgcttctcaggttccggcagcggaactgagtttacactgactatttctagtctgcagtgcgacgatttcgctacctactattgcctgggggtgtacggttattctttcgacgatggcatcgcatttggcggagggacaaaagtggagattaagaggactgtggccgctcccagtgtgttcatttttccccctagcgacgaacagctgaaaagcgggacagcctctgtggtgtgtctgctgaacaatttttaccctcgggaggccaaagtgcagtggaaggtggataacgctctgcagtctggcaatagtcaggagtcagtgaccgaacaggactccaaagatagcacatattctctgtcatccaccctgacactgtccaaggcagactacgagaagcacaaagtgtatgcctgcgaagtgactcatcagggcctgagctctcccgtgaccaagagctttaacaggggagaatgttga

SEQ ID NO: 80 - protein, 237 aa, Artificial Sequence
  source: /note="Description of Artificial Sequence: Synthetic polypeptide"
MGWSCIILFLVATATGVHSDIQMTQSPSTLSASVGDRVTITCQASQSISSYLAWYQQKPGKAPKLLIYYASTLASGVPSRFSGSGSGTEFTLTISSLQCDDFATYYCLGVYGYSFDDGIAFGGGTKVEIKRTVAAPSVFIFPPSDEQLKSGTASVVCLLNNFYPREAKVQWKVDNALQSGNSQESVTEQDSKDSTYSLSSTLTLSKADYEKHKVYACEVTHQGLSSPVTKSFNRGEC

SEQ ID NO: 81 - DNA, 714 bp, Artificial Sequence
  source: /note="Description of Artificial Sequence: Synthetic polynucleotide"
atggggtggtcttgcatcattctgttcctggtggcaaccgccacaggtgtgcactccgacatccagatgactcagagtccatcaaccctgtccgctagcgtgggagatagagtgactatcacctgtcaggcctctcagagtatttccagctacctggcttggtatcagcagaagccaggcaaagcacccaagctgctgatctactatgctagtacactggcatcaggagtgccttcccgcttctcaggttccggcagcggaactgagtttacactgactattactggtgtgcagtgcgacgatttcgctacctactattgcctgggggtgtacggttattctttcgacgatggcatcgcatttggcggagggacaaaagtggagattaagaggactgtggccgctcccagtgtgttcatttttccccctagcgacgaacagctgaaaagcgggacagcctctgtggtgtgtctgctgaacaatttttaccctcgggaggccaaagtgcagtggaaggtggataacgctctgcagtctggcaatagtcaggagtcagtgaccgaacaggactccaaagatagcacatattctctgtcatccaccctgacactgtccaaggcagactacgagaagcacaaagtgtatgcctgcgaagtgactcatcagggcctgagctctcccgtgaccaagagctttaacaggggagaatgttga

SEQ ID NO: 82 - protein, 237 aa, Artificial Sequence
  source: /note="Description of Artificial Sequence: Synthetic polypeptide"
MGWSCIILFLVATATGVHSDIQMTQSPSTLSASVGDRVTITCQASQSISSYLAWYQQKPGKAPKLLIYYASTLASGVPSRFSGSGSGTEFTLTITGVQCDDFATYYCLGVYGYSFDDGIAFGGGTKVEIKRTVAAPSVFIFPPSDEQLKSGTASVVCLLNNFYPREAKVQWKVDNALQSGNSQESVTEQDSKDSTYSLSSTLTLSKADYEKHKVYACEVTHQGLSSPVTKSFNRGEC

SEQ ID NO: 83 - DNA, 714 bp, Artificial Sequence
  source: /note="Description of Artificial Sequence: Synthetic polynucleotide"
atggggtggtcttgcatcattctgttcctggtggcaaccgccacaggtgtgcactccgacatccagatgactcagagtccatcaaccctgtccgctagcgtgggagatagagtgactatcacctgtcaggcctctcagagtatttccagctacctggcttggtatcagcagaagccaggcaaagcacccaagctgctgatctactatgctagtacactggcatcaggagtgccttcccgcttctcaggttccggcagcggaactgagtttacactgactatttctagtctgcagtgcgacgatgccgctacctactattgcctgggggtgtacggttattctttcgacgatggcatcgcatttggcggagggacaaaagtggagattaagaggactgtggccgctcccagtgtgttcatttttccccctagcgacgaacagctgaaaagcgggacagcctctgtggtgtgtctgctgaacaatttttaccctcgggaggccaaagtgcagtggaaggtggataacgctctgcagtctggcaatagtcaggagtcagtgaccgaacaggactccaaagatagcacatattctctgtcatccaccctgacactgtccaaggcagactacgagaagcacaaagtgtatgcctgcgaagtgactcatcagggcctgagctctcccgtgaccaagagctttaacaggggagaatgttga

SEQ ID NO: 84 - protein, 237 aa, Artificial Sequence
  source: /note="Description of Artificial Sequence: Synthetic polypeptide"
MGWSCIILFLVATATGVHSDIQMTQSPSTLSASVGDRVTITCQASQSISSYLAWYQQKPGKAPKLLIYYASTLASGVPSRFSGSGSGTEFTLTISSLQCDDAATYYCLGVYGYSFDDGIAFGGGTKVEIKRTVAAPSVFIFPPSDEQLKSGTASVVCLLNNFYPREAKVQWKVDNALQSGNSQESVTEQDSKDSTYSLSSTLTLSKADYEKHKVYACEVTHQGLSSPVTKSFNRGEC

SEQ ID NO: 85 - DNA, 714 bp, Artificial Sequence
  source: /note="Description of Artificial Sequence: Synthetic polynucleotide"
atggggtggtcttgcatcattctgttcctggtggcaaccgccacaggtgtgcactccgacatccagatgactcagagtccatcaaccctgtccgctagcgtgggagatagagtgactatcacctgtcaggcctctcagagtatttccagctacctggcttggtatcagcagaagccaggcaaagcacccaagctgctgatctactatgctagtacactggcatcaggagtgccttcccgcttctcaggttccggcagcggaactgagtttacactgactattactggtgtgcagtgcgacgatgccgctacctactattgcctgggggtgtacggttattctttcgacgatggcatcgcatttggcggagggacaaaagtggagattaagaggactgtggccgctcccagtgtgttcatttttccccctagcgacgaacagctgaaaagcgggacagcctctgtggtgtgtctgctgaacaatttttaccctcgggaggccaaagtgcagtggaaggtggataacgctctgcagtctggcaatagtcaggagtcagtgaccgaacaggactccaaagatagcacatattctctgtcatccaccctgacactgtccaaggcagactacgagaagcacaaagtgtatgcctgcgaagtgactcatcagggcctgagctctcccgtgaccaagagctttaacaggggagaatgttga

SEQ ID NO: 86 - protein, 237 aa, Artificial Sequence
  source: /note="Description of Artificial Sequence: Synthetic polypeptide"
MGWSCIILFLVATATGVHSDIQMTQSPSTLSASVGDRVTITCQASQSISSYLAWYQQKPGKAPKLLIYYASTLASGVPSRFSGSGSGTEFTLTITGVQCDDAATYYCLGVYGYSFDDGIAFGGGTKVEIKRTVAAPSVFIFPPSDEQLKSGTASVVCLLNNFYPREAKVQWKVDNALQSGNSQESVTEQDSKDSTYSLSSTLTLSKADYEKHKVYACEVTHQGLSSPVTKSFNRGEC

SEQ ID NO: 87 - DNA, 714 bp, Artificial Sequence
  source: /note="Description of Artificial Sequence: Synthetic polynucleotide"
atggggtggtcttgcatcattctgttcctggtggcaaccgccacaggtgtgcactccgacatccagatgactcagagtccatcaaccctgtccgctagcgtgggagatagagtgactatcacctgtcaggcctctcagagtatttccagctacctggcttggtatcagcagaagccaggcaaagcacccaagctgctgatctactatgctagtacactggcatcaggagtgccttcccgcttcaaaggttccggcagcggaactgagtttacactgactattactggtgtgcagtgcgacgatgccgctacctactattgcctgggggtgtacggttattctttcgacgatggcatcgcatttggcggagggacaaaagtggagattaagaggactgtggccgctcccagtgtgttcatttttccccctagcgacgaacagctgaaaagcgggacagcctctgtggtgtgtctgctgaacaatttttaccctcgggaggccaaagtgcagtggaaggtggataacgctctgcagtctggcaatagtcaggagtcagtgaccgaacaggactccaaagatagcacatattctctgtcatccaccctgacactgtccaaggcagactacgagaagcacaaagtgtatgcctgcgaagtgactcatcagggcctgagctctcccgtgaccaagagctttaacaggggagaatgttga

SEQ ID NO: 88 - protein, 237 aa, Artificial Sequence
  source: /note="Description of Artificial Sequence: Synthetic polypeptide"
MGWSCIILFLVATATGVHSDIQMTQSPSTLSASVGDRVTITCQASQSISSYLAWYQQKPGKAPKLLIYYASTLASGVPSRFKGSGSGTEFTLTITGVQCDDAATYYCLGVYGYSFDDGIAFGGGTKVEIKRTVAAPSVFIFPPSDEQLKSGTASVVCLLNNFYPREAKVQWKVDNALQSGNSQESVTEQDSKDSTYSLSSTLTLSKADYEKHKVYACEVTHQGLSSPVTKSFNRGEC

SEQ ID NO: 89 - DNA, 714 bp, Artificial Sequence
  source: /note="Description of Artificial Sequence: Synthetic polynucleotide"
atggggtggtcttgcatcattctgttcctggtggcaaccgccacaggtgtgcactccgacatccagatgactcagagtccatcaaccgtgtccgctgcagtgggaggtacagtgactatcacctgtcaggcctctcagagtatttccagctacctggcttggtatcagcagaagccaggcaaagcacccaagctgctgatctactatgctagtacactggcatcaggagtgccttcccgcttctcaggttccggcagcggaactgagtttacactgactattactggtgtgcagtgcgacgatgccgctacctactattgcctgggggtgtacggttattctttcgacgatggcatcgcatttggcggagggacaaaagtggagattaagaggactgtggccgctcccagtgtgttcatttttccccctagcgacgaacagctgaaaagcgggacagcctctgtggtgtgtctgctgaacaatttttaccctcgggaggccaaagtgcagtggaaggtggataacgctctgcagtctggcaatagtcaggagtcagtgaccgaacaggactccaaagatagcacatattctctgtcatccaccctgacactgtccaaggcagactacgagaagcacaaagtgtatgcctgcgaagtgactcatcagggcctgagctctcccgtgaccaagagctttaacaggggagaatgttga

SEQ ID NO: 90 - protein, 237 aa, Artificial Sequence
  source: /note="Description of Artificial Sequence: Synthetic polypeptide"
MGWSCIILFLVATATGVHSDIQMTQSPSTVSAAVGGTVTITCQASQSISSYLAWYQQKPGKAPKLLIYYASTLASGVPSRFSGSGSGTEFTLTITGVQCDDAATYYCLGVYGYSFDDGIAFGGGTKVEIKRTVAAPSVFIFPPSDEQLKSGTASVVCLLNNFYPREAKVQWKVDNALQSGNSQESVTEQDSKDSTYSLSSTLTLSKADYEKHKVYACEVTHQGLSSPVTKSFNRGEC

SEQ ID NO: 91 - DNA, 714 bp, Artificial Sequence
  source: /note="Description of Artificial Sequence: Synthetic polynucleotide"
atggggtggtcttgcatcattctgttcctggtggcaaccgccacaggtgtgcactccgacatccagatgactcagagtccatcaaccctgtccgctagcgtgggagatagagtgactatcacctgtcaggcctctcagagtatttccagctacctggcttggtatcagcagaagccaggcaaagcacccaagctgctgatctactatgctagtacactggcatcaggagtgccttcccgcttctcaggttccggcagcggaactgagtttacactgactattactggtgtgcagtgcgacgatgccgctacctactattgcctgggggtgtacggttattctttcgacgatggcatcgcatttggcggagggacagagctggagattaagaggactgtggccgctcccagtgtgttcatttttccccctagcgacgaacagctgaaaagcgggacagcctctgtggtgtgtctgctgaacaatttttaccctcgggaggccaaagtgcagtggaaggtggataacgctctgcagtctggcaatagtcaggagtcagtgaccgaacaggactccaaagatagcacatattctctgtcatccaccctgacactgtccaaggcagactacgagaagcacaaagtgtatgcctgcgaagtgactcatcagggcctgagctctcccgtgaccaagagctttaacaggggagaatgttga

SEQ ID NO: 92 - protein, 237 aa, Artificial Sequence
  source: /note="Description of Artificial Sequence: Synthetic polypeptide"
MGWSCIILFLVATATGVHSDIQMTQSPSTLSASVGDRVTITCQASQSISSYLAWYQQKPGKAPKLLIYYASTLASGVPSRFSGSGSGTEFTLTITGVQCDDAATYYCLGVYGYSFDDGIAFGGGTELEIKRTVAAPSVFIFPPSDEQLKSGTASVVCLLNNFYPREAKVQWKVDNALQSGNSQESVTEQDSKDSTYSLSSTLTLSKADYEKHKVYACEVTHQGLSSPVTKSFNRGEC

SEQ ID NO: 93 - DNA, 714 bp, Artificial Sequence
  source: /note="Description of Artificial Sequence: Synthetic polynucleotide"
atgggctggtcctgcatcatcctgtttctggtggccaccgccaccggcgtgcacagcgacattcagatgactcagtccccctcctccctttcggcctccgtcggcgaccgcgtgaccattacctgtcaagccagccagtccatctcctcctacttggcctggtaccaacagaagccaggaaaagctcctaagctgctcatctactacgcctccactctggcgtctggtgtcccgtcacggttcagcgggtccggatcaggaactgacttcaccctgacgatcagcagcctccagtgcgaggattttgcgacctactactgcctgggggtgtatggttactcgttcgacgatggaatcgcattcggctcgggcaccaaggtggaaatcaaacgaactgtggctgcaccatctgtcttcatcttcccgccatctgatgagcagttgaaatctggaactgcctctgttgtgtgcctgctgaataacttctatcccagagaggccaaagtacagtggaaggtggataacgccctccaatcgggtaactcccaggagagtgtcacagagcaggacagcaaggacagcacctacagcctcagcagcaccctgacgctgagcaaagcagactacgagaaacacaaagtctacgcctgcgaagtcacccatcagggcctgagctcgcccgtcacaaagagcttcaacaggggagagtgttga

SEQ ID NO: 94 - protein, 237 aa, Artificial Sequence
  source: /note="Description of Artificial Sequence: Synthetic polypeptide"
MGWSCIILFLVATATGVHSDIQMTQSPSSLSASVGDRVTITCQASQSISSYLAWYQQKPGKAPKLLIYYASTLASGVPSRFSGSGSGTDFTLTISSLQCEDFATYYCLGVYGYSFDDGIAFGSGTKVEIKRTVAAPSVFIFPPSDEQLKSGTASVVCLLNNFYPREAKVQWKVDNALQSGNSQESVTEQDSKDSTYSLSSTLTLSKADYEKHKVYACEVTHQGLSSPVTKSFNRGEC

SEQ ID NO: 95 - DNA, 714 bp, Artificial Sequence
  source: /note="Description of Artificial Sequence: Synthetic polynucleotide"
atgggctggtcctgcatcatcctgtttctggtggccaccgccaccggcgtgcacagcgacattgtgatgacccagactcctctctccctgcccgtgactcctggagaacccgcctcgatctcatgtcaagcgtcgcagagcatctcctcatacttggcttggtacctccaaaagccgggccagagcccacagcttctgatctattacgcctccaccctggcctcgggcgtgccggatcggttttccggttctggaagcggaaccgacttcaccctgaaaatctcccgcgtggagtgcgaggacgtgggcgtgtactactgcctgggagtctacgggtactccttcgatgacggcattgcattcgggtccggtaccaaggtcgaaatcaaacgaactgtggctgcaccatctgtcttcatcttcccgccatctgatgagcagttgaaatctggaactgcctctgttgtgtgcctgctgaataacttctatcccagagaggccaaagtacagtggaaggtggataacgccctccaatcgggtaactcccaggagagtgtcacagagcaggacagcaaggacagcacctacagcctcagcagcaccctgacgctgagcaaagcagactacgagaaacacaaagtctacgcctgcgaagtcacccatcagggcctgagctcgcccgtcacaaagagcttcaacaggggagagtgttga

SEQ ID NO: 96 - protein, 237 aa, Artificial Sequence
  source: /note="Description of Artificial Sequence: Synthetic polypeptide"
MGWSCIILFLVATATGVHSDIVMTQTPLSLPVTPGEPASISCQASQSISSYLAWYLQKPGQSPQLLIYYASTLASGVPDRFSGSGSGTDFTLKISRVECEDVGVYYCLGVYGYSFDDGIAFGSGTKVEIKRTVAAPSVFIFPPSDEQLKSGTASVVCLLNNFYPREAKVQWKVDNALQSGNSQESVTEQDSKDSTYSLSSTLTLSKADYEKHKVYACEVTHQGLSSPVTKSFNRGEC

SEQ ID NO: 97 - DNA, 714 bp, Artificial Sequence
  source: /note="Description of Artificial Sequence: Synthetic polynucleotide"
atgggctggtcctgcatcatcctgtttctggtggccaccgccaccggcgtgcacagcgaaattgtgctcactcaatcccctgccaccctttccttgtcccccggcgaaagagccactctgtcatgtcaagccagccagtcgatctcctcttacctggcttggtaccagcagaagccaggacaggcaccgcgcctgctgatctactacgcgtcgaccctcgcctcgggaatcccggcccggttcagcggatcaggctccggtaccgacttcactctgaccattagctccctggagtgcgaggacttcgcggtgtattactgcctgggggtgtacggctactccttcgatgacggaatcgcctttgggagcggtaccaaggtcgagatcaaacgaactgtggctgcaccatctgtcttcatcttcccgccatctgatgagcagttgaaatctggaactgcctctgttgtgtgcctgctgaataacttctatcccagagaggccaaagtacagtggaaggtggataacgccctccaatcgggtaactcccaggagagtgtcacagagcaggacagcaaggacagcacctacagcctcagcagcaccctgacgctgagcaaagcagactacgagaaacacaaagtctacgcctgcgaagtcacccatcagggcctgagctcgcccgtcacaaagagcttcaacaggggagagtgttga

SEQ ID NO: 98 - protein, 237 aa, Artificial Sequence
  source: /note="Description of Artificial Sequence: Synthetic polypeptide"
MGWSCIILFLVATATGVHSEIVLTQSPATLSLSPGERATLSCQASQSISSYLAWYQQKPGQAPRLLIYYASTLASGIPARFSGSGSGTDFTLTISSLECEDFAVYYCLGVYGYSFDDGIAFGSGTKVEIKRTVAAPSVFIFPPSDEQLKSGTASVVCLLNNFYPREAKVQWKVDNALQSGNSQESVTEQDSKDSTYSLSSTLTLSKADYEKHKVYACEVTHQGLSSPVTKSFNRGEC

SEQ ID NO: 99 - DNA, 714 bp, Artificial Sequence
  source: /note="Description of Artificial Sequence: Synthetic polynucleotide"
atgggctggtcctgcatcatcctgtttctggtggccaccgccaccggcgtgcacagcgatatcgtgatgacccaaagccctgactcccttgccgtgtcactcggagaacgcgccaccatcaactgtcaagcgtcgcagtccatctcctcatacctggcctggtatcagcagaaaccggggcagccgccaaagctgctgatctactacgcttccactctggcctccggcgtgcccgatcggttctccggatcgggctccggcaccgactttactctgaccattagcagcctccagtgcgaggacgtggcggtgtactactgcttgggtgtctacggatactccttcgacgacgggatcgcattcggttcgggaaccaaggtcgagattaaacgaactgtggctgcaccatctgtcttcatcttcccgccatctgatgagcagttgaaatctggaactgcctctgttgtgtgcctgctgaataacttctatcccagagaggccaaagtacagtggaaggtggataacgccctccaatcgggtaactcccaggagagtgtcacagagcaggacagcaaggacagcacctacagcctcagcagcaccctgacgctgagcaaagcagactacgagaaacacaaagtctacgcctgcgaagtcacccatcagggcctgagctcgcccgtcacaaagagcttcaacaggggagagtgttga

SEQ ID NO: 100 - protein, 237 aa, Artificial Sequence
  source: /note="Description of Artificial Sequence: Synthetic polypeptide"
MGWSCIILFLVATATGVHSDIVMTQSPDSLAVSLGERATINCQASQSISSYLAWYQQKPGQPPKLLIYYASTLASGVPDRFSGSGSGTDFTLTISSLQCEDVAVYYCLGVYGYSFDDGIAFGSGTKVEIKRTVAAPSVFIFPPSDEQLKSGTASVVCLLNNFYPREAKVQWKVDNALQSGNSQESVTEQDSKDSTYSLSSTLTLSKADYEKHKVYACEVTHQGLSSPVTKSFNRGEC

SEQ ID NO: 101 - DNA, 714 bp, Artificial Sequence
  source: /note="Description of Artificial Sequence: Synthetic polynucleotide"
atgggctggtcctgcatcatcctgtttctggtggccaccgccaccggcgtgcacagcgaaatcgtcttgacccaaagccctgacttccaatccgtgacccccaaggaaaaggtcaccatcacgtgtcaggcctcccagtcaatttcctcgtaccttgcgtggtaccagcagaagccagaccagtccccgaagctcctgattaagtacgcatccaccctggctagcggagtgccgagccggttctcgggatccggctctggaactgacttcactctgaccatcaactcgctcgagtgcgaagatgccgccacttactattgcctgggggtgtacgggtactcatttgacgatggcatcgccttcggctccggtaccaaagtggagatcaaacgaactgtggctgcaccatctgtcttcatcttcccgccatctgatgagcagttgaaatctggaactgcctctgttgtgtgcctgctgaataacttctatcccagagaggccaaagtacagtggaaggtggataacgccctccaatcgggtaactcccaggagagtgtcacagagcaggacagcaaggacagcacctacagcctcagcagcaccctgacgctgagcaaagcagactacgagaaacacaaagtctacgcctgcgaagtcacccatcagggcctgagctcgcccgtcacaaagagcttcaacaggggagagtgttga

SEQ ID NO: 102 - protein, 237 aa, Artificial Sequence
  source: /note="Description of Artificial Sequence: Synthetic polypeptide"
MGWSCIILFLVATATGVHSEIVLTQSPDFQSVTPKEKVTITCQASQSISSYLAWYQQKPDQSPKLLIKYASTLASGVPSRFSGSGSGTDFTLTINSLECEDAATYYCLGVYGYSFDDGIAFGSGTKVEIKRTVAAPSVFIFPPSDEQLKSGTASVVCLLNNFYPREAKVQWKVDNALQSGNSQESVTEQDSKDSTYSLSSTLTLSKADYEKHKVYACEVTHQGLSSPVTKSFNRGEC

SEQ ID NO: 103 - DNA, 714 bp, Artificial Sequence
  source: /note="Description of Artificial Sequence: Synthetic polynucleotide"
atgggctggtcctgcatcatcctgtttctggtggccaccgccaccggcgtgcacagcgacgtcgtgatgactcaaagccccgcattcctttccgtgactcctggagaaaaggtcaccatcacctgtcaagccagccagtccatttcgtcctacttggcctggtatcagcagaagccagaccaggccccgaagctgctgattaagtacgcctccaccctggccagcggagtgccgtcacggttctccgggtccggctcaggaaccgacttcacgttcaccatctcgtccctcgagtgcgaagatgctgcgacttactactgcctgggcgtgtacggttactcgtttgatgacggcatcgcgttcgggtctggaaccaaagtggagatcaaacgaactgtggctgcaccatctgtcttcatcttcccgccatctgatgagcagttgaaatctggaactgcctctgttgtgtgcctgctgaataacttctatcccagagaggccaaagtacagtggaaggtggataacgccctccaatcgggtaactcccaggagagtgtcacagagcaggacagcaaggacagcacctacagcctcagcagcaccctgacgctgagcaaagcagactacgagaaacacaaagtctacgcctgcgaagtcacccatcagggcctgagctcgcccgtcacaaagagcttcaacaggggagagtgttga

SEQ ID NO: 104 - protein, 237 aa, Artificial Sequence
  source: /note="Description of Artificial Sequence: Synthetic polypeptide"
MGWSCIILFLVATATGVHSDVVMTQSPAFLSVTPGEKVTITCQASQSISSYLAWYQQKPDQAPKLLIKYASTLASGVPSRFSGSGSGTDFTFTISSLECEDAATYYCLGVYGYSFDDGIAFGSGTKVEIKRTVAAPSVFIFPPSDEQLKSGTASVVCLLNNFYPREAKVQWKVDNALQSGNSQESVTEQDSKDSTYSLSSTLTLSKADYEKHKVYACEVTHQGLSSPVTKSFNRGEC

SEQ ID NO: 105 - DNA, 714 bp, Artificial Sequence
  source: /note="Description of Artificial Sequence: Synthetic polynucleotide"
atgggctggtcctgcatcatcctgtttctggtggccaccgccaccggcgtgcacagcgatatcgtcctcactcaatcccccgcttcactcgccgtgtcccctggtcaacgcgccaccattacgtgtcaggcgtcccagtccatttcgagctaccttgcatggtaccagcagaagcctggacagcccccgaaactgctgatctattacgcctccaccttggcctcgggagtgccagcgcggtttagcggttcgggctccggcactgacttcactctgaccatcaacccggtggagtgcgaagataccgccaactactactgcctgggggtgtacggatactcattcgacgacgggatcgccttcggaagcggcaccaaggtcgaaatcaaacgaactgtggctgcaccatctgtcttcatcttcccgccatctgatgagcagttgaaatctggaactgcctctgttgtgtgcctgctgaataacttctatcccagagaggccaaagtacagtggaaggtggataacgccctccaatcgggtaactcccaggagagtgtcacagagcaggacagcaaggacagcacctacagcctcagcagcaccctgacgctgagcaaagcagactacgagaaacacaaagtctacgcctgcgaagtcacccatcagggcctgagctcgcccgtcacaaagagcttcaacaggggagagtgttga

SEQ ID NO: 106 - protein, 237 aa, Artificial Sequence
  source: /note="Description of Artificial Sequence: Synthetic polypeptide"
MGWSCIILFLVATATGVHSDIVLTQSPASLAVSPGQRATITCQASQSISSYLAWYQQKPGQPPKLLIYYASTLASGVPARFSGSGSGTDFTLTINPVECEDTANYYCLGVYGYSFDDGIAFGSGTKVEIKRTVAAPSVFIFPPSDEQLKSGTASVVCLLNNFYPREAKVQWKVDNALQSGNSQESVTEQDSKDSTYSLSSTLTLSKADYEKHKVYACEVTHQGLSSPVTKSFNRGEC

SEQ ID NO: 107 - DNA, 711 bp, Artificial Sequence
  source: /note="Description of Artificial Sequence: Synthetic polynucleotide"
atgggctggtcctgcatcatcctgtttctggtggccaccgccaccggcgtgcactccgagctcgtgatgacccagactccagcctctgtggaggtagctgtgggaggcacagtcaccatcaagtgccaggccagtcagagcattaatacctacttagcctggtatcagcagaaaccagggcagcctcccaagctcctgatctacagggcatccactctggcatctggggtcccatcgcggttcaaaggcagtggatctgggacagagttcactctcaccattagcgacctggagtgtgccgatgctgccacttactactgtcaacagagtgttcgtgttattgatgttgataatactttcggcggagggaccgaggtggtggtcaaacgaactgtggctgcaccatctgtcttcatcttcccgccatctgatgagcagttgaaatctggaactgcctctgttgtgtgcctgctgaataacttctatcccagagaggccaaagtacagtggaaggtggataacgccctccaatcgggtaactcccaggagagtgtcacagagcaggacagcaaggacagcacctacagcctcagcagcaccctgacgctgagcaaagcagactacgagaaacacaaagtctacgcctgcgaagtcacccatcagggcctgagctcgcccgtcacaaagagcttcaacaggggagagtgttga

SEQ ID NO: 108 - protein, 236 aa, Artificial Sequence
  source: /note="Description of Artificial Sequence: Synthetic polypeptide"
MGWSCIILFLVATATGVHSELVMTQTPASVEVAVGGTVTIKCQASQSINTYLAWYQQKPGQPPKLLIYRASTLASGVPSRFKGSGSGTEFTLTISDLECADAATYYCQQSVRVIDVDNTFGGGTEVVVKRTVAAPSVFIFPPSDEQLKSGTASVVCLLNNFYPREAKVQWKVDNALQSGNSQESVTEQDSKDSTYSLSSTLTLSKADYEKHKVYACEVTHQGLSSPVTKSFNRGEC

SEQ ID NO: 109 - DNA, 714 bp, Artificial Sequence
  source: /note="Description of Artificial Sequence: Synthetic polynucleotide"
atgggctggtcctgcatcatcctgtttctggtggccaccgccaccggcgtgcacagcgagctcgtgatgacccagactccatcctacacgtctgcagctgtgggagacacagtcaccatcaagtgccaggccagtcagaccattggtggtagcgacttatcctggtatcagcagaaaccagggcagcctcccaaactcctgatctggtatgcaaccaatctgccatctggggtcccatcgcggttcagtggcagtagatctgggacagagtacactctcaccatcagcggcgtgcagtgtgaggatgctgccacctactactgtctaggtggttatgctgctgcttcttacagaactgctttcggcggagggaccgaggtggtcgtcaaacgaactgtggctgcaccatctgtcttcatcttcccgccatctgatgagcagttgaaatctggaactgcctctgttgtgtgcctgctgaataacttctatcccagagaggccaaagtacagtggaaggtggataacgccctccaatcgggtaactcccaggagagtgtcacagagcaggacagcaaggacagcacctacagcctcagcagcaccctgacgctgagcaaagcagactacgagaaacacaaagtctacgcctgcgaagtcacccatcagggcctgagctcgcccgtcacaaagagcttcaacaggggagagtgttga

SEQ ID NO: 110 - protein, 237 aa, Artificial Sequence
  source: /note="Description of Artificial Sequence: Synthetic polypeptide"
MGWSCIILFLVATATGVHSELVMTQTPSYTSAAVGDTVTIKCQASQTIGGSDLSWYQQKPGQPPKLLIWYATNLPSGVPSRFSGSRSGTEYTLTISGVQCEDAATYYCLGGYAAASYRTAFGGGTEVVVKRTVAAPSVFIFPPSDEQLKSGTASVVCLLNNFYPREAKVQWKVDNALQSGNSQESVTEQDSKDSTYSLSSTLTLSKADYEKHKVYACEVTHQGLSSPVTKSFNRGEC

SEQ ID NO: 111 - DNA, 714 bp, Artificial Sequence
  source: /note="Description of Artificial Sequence: Synthetic polynucleotide"
atgggctggtcctgcatcatcctgtttctggtggccaccgccaccggcgtgcacagcgatattcagatgacccagagcccttccttcctgtcagccagcgtcggggatagagtcacaatcacttgccaggccagccagaccattggcgggagcgacctgtcctggtaccagcagaagcccggaaaagcccctaagctgctgatctactatgctacaaacctgccatctggcgtgcccagccggttctctggaagtggctcagggactgactttaccctgacaattagctccctgcagtgcgaggatttcgccacctactattgtctggggggctatgccgccgcaagctaccgcaccgccttcggaggaggaactaaagtggaaatcaaacgaactgtggctgcaccatctgtcttcatcttcccgccatctgatgagcagttgaaatctggaactgcctctgttgtgtgcctgctgaataacttctatcccagagaggccaaagtacagtggaaggtggataacgccctccaatcgggtaactcccaggagagtgtcacagagcaggacagcaaggacagcacctacagcctcagcagcaccctgacgctgagcaaagcagactacgagaaacacaaagtctacgcctgcgaagtcacccatcagggcctgagctcgcccgtcacaaagagcttcaacaggggagagtgttga

SEQ ID NO: 112 - protein, 237 aa, Artificial Sequence
  source: /note="Description of Artificial Sequence: Synthetic polypeptide"
MGWSCIILFLVATATGVHSDIQMTQSPSFLSASVGDRVTITCQASQTIGGSDLSWYQQKPGKAPKLLIYYATNLPSGVPSRFSGSGSGTDFTLTISSLQCEDFATYYCLGGYAAASYRTAFGGGTKVEIKRTVAAPSVFIFPPSDEQLKSGTASVVCLLNNFYPREAKVQWKVDNALQSGNSQESVTEQDSKDSTYSLSSTLTLSKADYEKHKVYACEVTHQGLSSPVTKSFNRGEC

SEQ ID NO: 113 - DNA, 714 bp, Artificial Sequence
  source: /note="Description of Artificial Sequence: Synthetic polynucleotide"
atgggctggtcctgcatcatcctgtttctggtggccaccgccaccggcgtgcacagcgatattcagatgactcagagcccttccttcctgtccgcttccgtcggggatcgggtcacaatcacttgccaggcctcacagactattggcgggagcgacctgtcctggtaccagcagaagcccggaaaagcacctaagctgctgatctactatgccacaaacctgccatctggcgtgcccagccggttctctggaagtggctcagggactgactttaccctgacaattagctccctgcagtgcgaggatgccgctacctactattgtctggggggctacgccgccgcttcatacaggaccgccttcggaggaggaactaaagtggaaatcaaacgaactgtggctgcaccatctgtcttcatcttcccgccatctgatgagcagttgaaatctggaactgcctctgttgtgtgcctgctgaataacttctatcccagagaggccaaagtacagtggaaggtggataacgccctccaatcgggtaactcccaggagagtgtcacagagcaggacagcaaggacagcacctacagcctcagcagcaccctgacgctgagcaaagcagactacgagaaacacaaagtctacgcctgcgaagtcacccatcagggcctgagctcgcccgtcacaaagagcttcaacaggggagagtgttga

SEQ ID NO: 114 - protein, 237 aa, Artificial Sequence
  source: /note="Description of Artificial Sequence: Synthetic polypeptide"
MGWSCIILFLVATATGVHSDIQMTQSPSFLSASVGDRVTITCQASQTIGGSDLSWYQQKPGKAPKLLIYYATNLPSGVPSRFSGSGSGTDFTLTISSLQCEDAATYYCLGGYAAASYRTAFGGGTKVEIKRTVAAPSVFIFPPSDEQLKSGTASVVCLLNNFYPREAKVQWKVDNALQSGNSQESVTEQDSKDSTYSLSSTLTLSKADYEKHKVYACEVTHQGLSSPVTKSFNRGEC

SEQ ID NO: 115 - DNA, 717 bp, Artificial Sequence
  source: /note="Description of Artificial Sequence: Synthetic polynucleotide"
atgggctggtcctgcatcatcctgtttctggtggccaccgccaccggcgtgcactccgaagtgttgatgacccagactccatcctccgtgtctgcagctgtgggagacacagtcaccatcaagtgccaggccagtcagagcattagtagtgtcttgtcctggtatcagcagaaaccagggcagcctcccaagctcctgatctatctggcatccactctggcatctggggtcccatcgcggttcagcggcagtagatctgggacagagttcactctcaccatcagcgacctggagtgtgacgatgctgccacttactactgtcaaaccaattatggtactagtagtagtaattatggttttgctttcggcggagggaccgaggtggtcgtcaaacgaactgtggctgcaccatctgtcttcatcttcccgccatctgatgagcagttgaaatctggaactgcctctgttgtgtgcctgctgaataacttctatcccagagaggccaaagtacagtggaaggtggataacgccctccaatcgggtaactcccaggagagtgtcacagagcaggacagcaaggacagcacctacagcctcagcagcaccctgacgctgagcaaagcagactacgagaaacacaaagtctacgcctgcgaagtcacccatcagggcctgagctcgcccgtcacaaagagcttcaacaggggagagtgttga

SEQ ID NO: 116 - protein, 238 aa, Artificial Sequence
  source: /note="Description of Artificial Sequence: Synthetic polypeptide"
MGWSCIILFLVATATGVHSEVLMTQTPSSVSAAVGDTVTIKCQASQSISSVLSWYQQKPGQPPKLLIYLASTLASGVPSRFSGSRSGTEFTLTISDLECDDAATYYCQTNYGTSSSNYGFAFGGGTEVVVKRTVAAPSVFIFPPSDEQLKSGTASVVCLLNNFYPREAKVQWKVDNALQSGNSQESVTEQDSKDSTYSLSSTLTLSKADYEKHKVYACEVTHQGLSSPVTKSFNRGEC

SEQ ID NO: 117 - DNA, 717 bp, Artificial Sequence
  source: /note="Description of Artificial Sequence: Synthetic polynucleotide"
atgggctggtcctgcatcatcctgtttctggtggccaccgccaccggcgtgcacagcgacattcagatgacccagtccccaagctcgctgtccgcctccgtgggcgaccgcgtgaccatcacgtgccaggcgtcccagtcaattagcagcgtgctctcctggtaccaacagaagccggggaaagcacccaagctgctgatctacttggcctccactctggcctcgggagtgccttcacggttctccggatcgggatctggtactgatttcaccctcaccatctcgagccttcagtgcgaggacttcgctacttactattgtcaaaccaactacggaacctccagctccaactacggctttgccttcggtggcgggaccaaggtcgaaatcaaacgaactgtggctgcaccatctgtcttcatcttcccgccatctgatgagcagttgaaatctggaactgcctctgttgtgtgcctgctgaataacttctatcccagagaggccaaagtacagtggaaggtggataacgccctccaatcgggtaactcccaggagagtgtcacagagcaggacagcaaggacagcacctacagcctcagcagcaccctgacgctgagcaaagcagactacgagaaacacaaagtctacgcctgcgaagtcacccatcagggcctgagctcgcccgtcacaaagagcttcaacaggggagagtgttga

SEQ ID NO: 118 - protein, 238 aa, Artificial Sequence
  source: /note="Description of Artificial Sequence: Synthetic polypeptide"
MGWSCIILFLVATATGVHSDIQMTQSPSSLSASVGDRVTITCQASQSISSVLSWYQQKPGKAPKLLIYLASTLASGVPSRFSGSGSGTDFTLTISSLQCEDFATYYCQTNYGTSSSNYGFAFGGGTKVEIKRTVAAPSVFIFPPSDEQLKSGTASVVCLLNNFYPREAKVQWKVDNALQSGNSQESVTEQDSKDSTYSLSSTLTLSKADYEKHKVYACEVTHQGLSSPVTKSFNRGEC

SEQ ID NO: 119 - DNA, 717 bp, Artificial Sequence
  source: /note="Description of Artificial Sequence: Synthetic polynucleotide"
atgggctggtcctgcatcatcctgtttctggtggccaccgccaccggcgtgcacagcgacattcagatgacccagtccccaagctcgctgtccgcctccgtgggcgaccgcgtgaccatcacgtgccaggcgtcccagtcaattagcagcgtgctctcctggtaccaacagaagccggggaaagcacccaagctgctgatctacttggcctccactctggcctcgggagtgccttcacggttctccggatcgggatctggtactgatttcaccctcaccatctcgagccttcagtgcgaggacgccgctacttactattgtcaaaccaactacggaacctccagctccaactacggctttgccttcggtggcgggaccaaggtcgaaatcaaacgaactgtggctgcaccatctgtcttcatcttcccgccatctgatgagcagttgaaatctggaactgcctctgttgtgtgcctgctgaataacttctatcccagagaggccaaagtacagtggaaggtggataacgccctccaatcgggtaactcccaggagagtgtcacagagcaggacagcaaggacagcacctacagcctcagcagcaccctgacgctgagcaaagcagactacgagaaacacaaagtctacgcctgcgaagtcacccatcagggcctgagctcgcccgtcacaaagagcttcaacaggggagagtgttga

SEQ ID NO: 120 - protein, 238 aa, Artificial Sequence
  source: /note="Description of Artificial Sequence: Synthetic polypeptide"
MGWSCIILFLVATATGVHSDIQMTQSPSSLSASVGDRVTITCQASQSISSVLSWYQQKPGKAPKLLIYLASTLASGVPSRFSGSGSGTDFTLTISSLQCEDAATYYCQTNYGTSSSNYGFAFGGGTKVEIKRTVAAPSVFIFPPSDEQLKSGTASVVCLLNNFYPREAKVQWKVDNALQSGNSQESVTEQDSKDSTYSLSSTLTLSKADYEKHKVYACEVTHQGLSSPVTKSFNRGEC

SEQ ID NO: 121 - DNA, 717 bp, Artificial Sequence
  source: /note="Description of Artificial Sequence: Synthetic polynucleotide"
atgggctggtcctgcatcatcctgtttctggtggccaccgccaccggcgtgcacagcgacattcagatgacccagtccccaagctcgctgtccgcctccgtgggcgaccgcgtgaccatcacgtgccaggcgtcccagtcaattagcagcgtgctctcctggtaccaacagaagccggggaaagcacccaagctgctgatctacttggcctccactctggcctcgggagtgccttcacggttctccggatcgggatctggtactgatttcaccctcaccatctcgagccttcagtgcgaggacatcgctacttactattgtcaaaccaactacggaacctccagctccaactacggctttgccttcggtggcgggaccaaggtcgaaatcaaacgaactgtggctgcaccatctgtcttcatcttcccgccatctgatgagcagttgaaatctggaactgcctctgttgtgtgcctgctgaataacttctatcccagagaggccaaagtacagtggaaggtggataacgccctccaatcgggtaactcccaggagagtgtcacagagcaggacagcaaggacagcacctacagcctcagcagcaccctgacgctgagcaaagcagactacgagaaacacaaagtctacgcctgcgaagtcacccatcagggcctgagctcgcccgtcacaaagagcttcaacaggggagagtgttga

SEQ ID NO: 122 - protein, 238 aa, Artificial Sequence
  source: /note="Description of Artificial Sequence: Synthetic polypeptide"
MGWSCIILFLVATATGVHSDIQMTQSPSSLSASVGDRVTITCQASQSISSVLSWYQQKPGKAPKLLIYLASTLASGVPSRFSGSGSGTDFTLTISSLQCEDIATYYCQTNYGTSSSNYGFAFGGGTKVEIKRTVAAPSVFIFPPSDEQLKSGTASVVCLLNNFYPREAKVQWKVDNALQSGNSQESVTEQDSKDSTYSLSSTLTLSKADYEKHKVYACEVTHQGLSSPVTKSFNRGEC

SEQ ID NO: 123 - DNA, 705 bp, Artificial Sequence
  source: /note="Description of Artificial Sequence: Synthetic polynucleotide"
atgggctggtcctgcatcatcctgtttctggtggccaccgccaccggcgtgcactccgcattcgaattgacccagactccatcctccgtggaggcagctgtgggaggcacagtcaccatcaagtgccaggccagtcagagcatttacagttatttagcctggtatcagcagaaaccagggcagcctcccaagctcctgatctattctgcatccactctggcatctggggtctcatcgcggttcagaggcagtggatctgggacagaatacactctcaccatcagcgacctggagtgtgccgatgctgccacttactactgtcaaacctattatgatattgttactagtactttcggcggagggaccgaggtggtcgtcaaacgaactgtggctgcaccatctgtcttcatcttcccgccatctgatgagcagttgaaatctggaactgcctctgttgtgtgcctgctgaataacttctatcccagagaggccaaagtacagtggaaggtggataacgccctccaatcgggtaactcccaggagagtgtcacagagcaggacagcaaggacagcacctacagcctcagcagcaccctgacgctgagcaaagcagactacgagaaacacaaagtctacgcctgcgaagtcacccatcagggcctgagctcgcccgtcacaaagagcttcaacaggggagagtgttga

SEQ ID NO: 124 - protein, 234 aa, Artificial Sequence
  source: /note="Description of Artificial Sequence: Synthetic polypeptide"
MGWSCIILFLVATATGVHSAFELTQTPSSVEAAVGGTVTIKCQASQSIYSYLAWYQQKPGQPPKLLIYSASTLASGVSSRFRGSGSGTEYTLTISDLECADAATYYCQTYYDIVTSTFGGGTEVVVKRTVAAPSVFIFPPSDEQLKSGTASVVCLLNNFYPREAKVQWKVDNALQSGNSQESVTEQDSKDSTYSLSSTLTLSKADYEKHKVYACEVTHQGLSSPVTKSFNRGEC

SEQ ID NO: 125 - DNA, 705 bp, Artificial Sequence
  source: /note="Description of Artificial Sequence: Synthetic polynucleotide"
atgggctggtcctgcatcatcctgtttctggtggccaccgccaccggcgtgcactccgcattcgaattgacccagactccatcctccgtggaggcagctgtgggaggcacagtcaccatcaagtgccaggccagtcagagcatttacagttatttagcctggtatcagcagaaaccagggcagcctcccaagctcctgatctattctgcatccactctggcatctggggtctcatcgcggttcagaggcagtggatctgggacagaatacattctcaccatcagcgacctggagtgtgccgatgctgccacttactactgtcaaacctattatgatattgttactagtactttcggcggagggaccgaggtggtggtcaaacgaactgtggctgcaccatctgtcttcatcttcccgccatctgatgagcagttgaaatctggaactgcctctgttgtgtgcctgctgaataacttctatcccagagaggccaaagtacagtggaaggtggataacgccctccaatcgggtaactcccaggagagtgtcacagagcaggacagcaaggacagcacctacagcctcagcagcaccctgacgctgagcaaagcagactacgagaaacacaaagtctacgcctgcgaagtcacccatcagggcctgagctcgcccgtcacaaagagcttcaacaggggagagtgttga

SEQ ID NO: 126 - protein, 234 aa, Artificial Sequence
  source: /note="Description of Artificial Sequence: Synthetic polypeptide"
MGWSCIILFLVATATGVHSAFELTQTPSSVEAAVGGTVTIKCQASQSIYSYLAWYQQKPGQPPKLLIYSASTLASGVSSRFRGSGSGTEYILTISDLECADAATYYCQTYYDIVTSTFGGGTEVVVKRTVAAPSVFIFPPSDEQLKSGTASVVCLLNNFYPREAKVQWKVDNALQSGNSQESVTEQDSKDSTYSLSSTLTLSKADYEKHKVYACEVTHQGLSSPVTKSFNRGEC

SEQ ID NO: 127 - DNA, 705 bp, Artificial Sequence
  source: /note="Description of Artificial Sequence: Synthetic polynucleotide"
atgggctggtcctgcatcatcctgtttctggtggccaccgccaccggcgtgcactccgccgtcgtgctgacccagactgcatcccccgtgtctggagttgtgggaggcacagtcaccatcaagtgccaggccagtcagaacatttacagcaatttagcctggtatcagcagaaaccagggcagcgtcccaagctcctgatgtatgatgcatccactctggcatctggggtcccatcgcggttcaaaggcagtggatctgggacacagttcactctcaccatcagcgacctggagtgtgccgatgctgccacttactactgtcaaagtattagtagtgttgacaataatgttttcggcggagggaccgaggtggtggtcaaacgaactgtggctgcaccatctgtcttcatcttcccgccatctgatgagcagttgaaatctggaactgcctctgttgtgtgcctgctgaataacttctatcccagagaggccaaagtacagtggaaggtggataacgccctccaatcgggtaactcccaggagagtgtcacagagcaggacagcaaggacagcacctacagcctcagcagcaccctgacgctgagcaaagcagactacgagaaacacaaagtctacgcctgcgaagtcacccatcagggcctgagctcgcccgtcacaaagagcttcaacaggggagagtgttga

SEQ ID NO: 128 - protein, 234 aa, Artificial Sequence
  source: /note="Description of Artificial Sequence: Synthetic polypeptide"
MGWSCIILFLVATATGVHSAVVLTQTASPVSGVVGGTVTIKCQASQNIYSNLAWYQQKPGQRPKLLMYDASTLASGVPSRFKGSGSGTQFTLTISDLECADAATYYCQSISSVDNNVFGGGTEVVVKRTVAAPSVFIFPPSDEQLKSGTASVVCLLNNFYPREAKVQWKVDNALQSGNSQESVTEQDSKDSTYSLSSTLTLSKADYEKHKVYACEVTHQGLSSPVTKSFNRGEC

SEQ ID NO: 129 - DNA, 705 bp, Artificial Sequence
  source: /note="Description of Artificial Sequence: Synthetic polynucleotide"
atgggctggtcctgcatcatcctgtttctggtggccaccgccaccggcgtgcactccgtattcgaattgacccagactccatcccccgtgtctgcagctgtgggaggcacagtcaccatcaggtgccaggccagtcagaacattaagagctacttagcctggtatcagcagaaaccagggcagcctcccaaactcctgatctatgaagcatccattctggcatctggggtctcatcgcggttcaaaggcagtggatctgggacagagttcactctcaccatcagcgacctggagtgtgccgatgctgccacttactactgtcaaagctattatgctgctagtagtaatgctttcggcggagggaccgaggtggtggtcaaacgaactgtggctgcaccatctgtcttcatcttcccgccatctgatgagcagttgaaatctggaactgcctctgttgtgtgcctgctgaataacttctatcccagagaggccaaagtacagtggaaggtggataacgccctccaatcgggtaactcccaggagagtgtcacagagcaggacagcaaggacagcacctacagcctcagcagcaccctgacgctgagcaaagcagactacgagaaacacaaagtctacgcctgcgaagtcacccatcagggcctgagctcgcccgtcacaaagagcttcaacaggggagagtgttga

SEQ ID NO: 130 - protein, 234 aa, Artificial Sequence
  source: /note="Description of Artificial Sequence: Synthetic polypeptide"
MGWSCIILFLVATATGVHSVFELTQTPSPVSAAVGGTVTIRCQASQNIKSYLAWYQQKPGQPPKLLIYEASILASGVSSRFKGSGSGTEFTLTISDLECADAATYYCQSYYAASSNAFGGGTEVVVKRTVAAPSVFIFPPSDEQLKSGTASVVCLLNNFYPREAKVQWKVDNALQSGNSQESVTEQDSKDSTYSLSSTLTLSKADYEKHKVYACEVTHQGLSSPVTKSFNRGEC

SEQ ID NO: 131 - DNA, 714 bp, Artificial Sequence
  source: /note="Description of Artificial Sequence: Synthetic polynucleotide"
atgggctggtcctgcatcatcctgtttctggtggccaccgccaccggcgtgcacagcgagctcgtgatgacccagactccatcctccgtgtctgcagctgtgggaggcacagtcaccatcaattgccaggccagtcagagcattagtaactacttatcctggtatcagcagaaaccaggacagcctcccaagctcctgatctttgctgcatccaaactggcatcttgggtcccaaagcggttcagtggcagcagatctgggatagaatacactctcaccattagcggcgtgcagtgtgacgatgctgccacttacttctgtctaggagtttatagtattagtactgatgatggagctgctttcggcggagggaccgaggtggtcgtcaaacgaactgtggctgcaccatctgtcttcatcttcccgccatctgatgagcagttgaaatctggaactgcctctgttgtgtgcctgctgaataacttctatcccagagaggccaaagtacagtggaaggtggataacgccctccaatcgggtaactcccaggagagtgtcacagagcaggacagcaaggacagcacctacagcctcagcagcaccctgacgctgagcaaagcagactacgagaaacacaaagtctacgcctgcgaagtcacccatcagggcctgagctcgcccgtcacaaagagcttcaacaggggagagtgttga

SEQ ID NO: 132 - protein, 237 aa, Artificial Sequence
  source: /note="Description of Artificial Sequence: Synthetic polypeptide"
MGWSCIILFLVATATGVHSELVMTQTPSSVSAAVGGTVTINCQASQSISNYLSWYQQKPGQPPKLLIFAASKLASWVPKRFSGSRSGIEYTLTISGVQCDDAATYFCLGVYSISTDDGAAFGGGTEVVVKRTVAAPSVFIFPPSDEQLKSGTASVVCLLNNFYPREAKVQWKVDNALQSGNSQESVTEQDSKDSTYSLSSTLTLSKADYEKHKVYACEVTHQGLSSPVTKSFNRGEC

SEQ ID NO: 133 - DNA, 714 bp, Artificial Sequence
  source: /note="Description of Artificial Sequence: Synthetic polynucleotide"
atgggctggtcctgcatcatcctgtttctggtggccaccgccaccggcgtgcacagcgatattcagatgacccagtctccttcctccctgtccgcttccgtcggcgatagagtcacaatcacttgccaggcttcccagagcatcagcaactacctgtcctggtatcagcagaagcccggcaaagcacctaagctgctgatctacgccgcttctaaactggcaagcggagtgccaagccggttctctggaagtgggtcaggaactgactttaccctgacaattagctccctgcagtgcgaggatttcgctacctactattgtctgggcgtctattcaatctcaactgacgacggagccgcattcggagggggcaccaaagtggaaatcaaacgaactgtggctgcaccatctgtcttcatcttcccgccatctgatgagcagttgaaatctggaactgcctctgttgtgtgcctgctgaataacttctatcccagagaggccaaagtacagtggaaggtggataacgccctccaatcgggtaactcccaggagagtgtcacagagcaggacagcaaggacagcacctacagcctcagcagcaccctgacgctgagcaaagcagactacgagaaacacaaagtctacgcctgcgaagtcacccatcagggcctgagctcgcccgtcacaaagagcttcaacaggggagagtgttga

SEQ ID NO: 134 - protein, 237 aa, Artificial Sequence
  source: /note="Description of Artificial Sequence: Synthetic polypeptide"
MGWSCIILFLVATATGVHSDIQMTQSPSSLSASVGDRVTITCQASQSISNYLSWYQQKPGKAPKLLIYAASKLASGVPSRFSGSGSGTDFTLTISSLQCEDFATYYCLGVYSISTDDGAAFGGGTKVEIKRTVAAPSVFIFPPSDEQLKSGTASVVCLLNNFYPREAKVQWKVDNALQSGNSQESVTEQDSKDSTYSLSSTLTLSKADYEKHKVYACEVTHQGLSSPVTKSFNRGEC

SEQ ID NO: 135 - DNA, 714 bp, Artificial Sequence
  source: /note="Description of Artificial Sequence: Synthetic polynucleotide"
atgggctggtcctgcatcatcctgtttctggtggccaccgccaccggcgtgcacagcgatattcagatgacccagagcccttcctccctgtccgctagtgtcggggatagagtgaccattacttgccaggccagccagagcattagcaactacctgtcctggtatcagcagaagcccggcaaagctcctaagctgctgatctacgccgcttctaaactggcaagcggagtgccaagccggttctctggaagtgggtcaggaactgactttaccctgacaattagctccctgcagtgcgaggatgcagccacctactattgtctgggcgtctactcaatctcaaccgacgacggagctgcttttggagggggcactaaggtggaaatcaaacgaactgtggctgcaccatctgtcttcatcttcccgccatctgatgagcagttgaaatctggaactgcctctgttgtgtgcctgctgaataacttctatcccagagaggccaaagtacagtggaaggtggataacgccctccaatcgggtaactcccaggagagtgtcacagagcaggacagcaaggacagcacctacagcctcagcagcaccctgacgctgagcaaagcagactacgagaaacacaaagtctacgcctgcgaagtcacccatcagggcctgagctcgcccgtcacaaagagcttcaacaggggagagtgttga

SEQ ID NO: 136 - protein, 237 aa, Artificial Sequence
  source: /note="Description of Artificial Sequence: Synthetic polypeptide"
MGWSCIILFLVATATGVHSDIQMTQSPSSLSASVGDRVTITCQASQSISNYLSWYQQKPGKAPKLLIYAASKLASGVPSRFSGSGSGTDFTLTISSLQCEDAATYYCLGVYSISTDDGAAFGGGTKVEIKRTVAAPSVFIFPPSDEQLKSGTASVVCLLNNFYPREAKVQWKVDNALQSGNSQESVTEQDSKDSTYSLSSTLTLSKADYEKHKVYACEVTHQGLSSPVTKSFNRGEC

SEQ ID NO: 137 - DNA, 993 bp, Artificial Sequence
  source: /note="Description of Artificial Sequence: Synthetic polynucleotide"
gcatccaccaagggcccatcggtcttccccctggcaccctcctccaagagcacctctgggggcacagcggccctgggctgcctggtcaaggactacttccccgaaccggtgacggtgtcgtggaactcaggcgccctgaccagcggcgtgcacaccttcccggctgtcctacagtcctcaggactctactccctcagcagcgtggtgaccgtgccctccagcagcttgggcacccagacctacatctgcaacgtgaatcacaagcccagcaacaccaaggtggacaagaaagttgagcccaaatcttgtgacaaaactcacacatgcccaccgtgcccagcacctgaactcctggggggaccgtcagtcttcctcttccccccaaaacccaaggacaccctcatgatctcccggacccctgaggtcacatgcgtggtggtggacgtgagccacgaagaccctgaggtcaagttcaactggtacgtggacggcgtggaggtgcataatgccaagacaaagccgcgggaggagcagtacaacagcacgtaccgtgtggtcagcgtcctcaccgtcctgcaccaggactggctgaatggcaaggagtacaagtgcaaggtctccaacaaagccctcccagcccccatcgagaaaaccatctccaaagccaaagggcagccccgagaaccacaggtgtacaccctgcccccatcccgggatgagctgaccaagaaccaggtcagcctgacctgcctggtcaaaggcttctatcccagcgacatcgccgtggagtgggagagcaatgggcagccggagaacaactacaagaccacgcctcccgtgctggactccgacggctccttcttcttatattcaaagctcaccgtggacaagagcaggtggcagcaggggaacgtcttctcatgctccgtgatgcatgaggctctgcacaaccactacacgcagaagagcctctccctgtctcccgggaaatga

SEQ ID NO: 138 - protein, 330 aa, Artificial Sequence [sequence omitted]

SEQ ID NO: 139 - DNA, 324 bp, Artificial Sequence
  source: /note="Description of Artificial Sequence: Synthetic polynucleotide"
cgaactgtggctgcaccatctgtcttcatcttcccgccatctgatgagcagttgaaatctggaactgcctctgttgtgtgcctgctgaataacttctatcccagagaggccaaagtacagtggaaggtggataacgccctccaatcgggtaactcccaggagagtgtcacagagcaggacagcaaggacagcacctacagcctcagcagcaccctgacgctgagcaaagcagactacgagaaacacaaagtctacgcctgcgaagtcacccatcagggcctgagctcgcccgtcacaaagagcttcaacaggggagagtgttga

SEQ ID NO: 140 - protein, 107 aa, Artificial Sequence [sequence omitted]

SEQ ID NO: 141 - DNA, 972 bp, Artificial Sequence
  source: /note="Description of Artificial Sequence: Synthetic polynucleotide"
gggcaacctaaggctccatcagtcttcccactggccccctgctgcggggacacacccagctccacggtgaccctgggctgcctggtcaaaggctacctcccggagccagtgaccgtgacctggaactcgggcaccctcaccaatggggtacgcaccttcccgtccgtccggcagtcctcaggcctctactcgctgagcagcgtggtgagcgtgacctcaagcagccagcccgtcacctgcaacgtggcccacccagccaccaacaccaaagtggacaagaccgttgcaccctcgacatgcagcaagcccacgtgcccaccccctgaactcctggggggaccgtctgtcttcatcttccccccaaaacccaaggacaccctcatgatctcacgcacccccgaggtcacatgcgtggtggtggacgtgagccaggatgaccccgaggtgcagttcacatggtacataaacaacgagcaggtgcgcaccgcccggccgccgctacgggagcagcagttcaacagcacgatccgcgtggtcagcaccctccccatcacgcaccaggactggctgaggggcaaggagttcaagtgcaaagtccacaacaaggcactcccggcccccatcgagaaaaccatctccaaagccagagggcagcccctggagccgaaggtctacaccatgggccctccccgggaggagctgagcagcaggtcggtcagcctgacctgcatgatcaacggcttctacccttccgacatctcggtggagtgggagaagaacgggaaggcagaggacaactacaagaccacgccggccgtgctggacagcgacggctcctacttcctctacaacaagctctcagtgcccacgagtgagtggcagcggggcgacgtcttcacctgctccgtgatgcacgaggccttgcacaaccactacacgcagaagtccatctcccgctctccgggtaaatga

SEQ ID NO: 142 - protein, 323 aa, Artificial Sequence
  source: /note="Description of Artificial Sequence: Synthetic polypeptide"
GQPKAPSVFPLAPCCGDTPSSTVTLGCLVKGYLPEPVTVTWNSGTLTNGVRTFPSVRQSSGLYSLSSVVSVTSSSQPVTCNVAHPATNTKVDKTVAPSTCSKPTCPPPELLGGPSVFIFPPKPKDTLMISRTPEVTCVVVDVSQDDPEVQFTWYINNEQVRTARPPLREQQFNSTIRVVSTLPITHQDWLRGKEFKCKVHNKALPAPIEKTISKARGQPLEPKVYTMGPPREELSSRSVSLTCMINGFYPSDISVEWEKNGKAEDNYKTTPAVLDSDGSYFLYNKLSVPTSEWQRGDVFTCSVMHEALHNHYTQKSISRSPGK

SEQ ID NO: 143 - DNA, 315 bp, Artificial Sequence
  source: /note="Description of Artificial Sequence: Synthetic polynucleotide"
ggtgatccagttgcacctactgtcctcatcttcccaccatctgctgatcttgtggcaactggaacagtcaccatcgtgtgtgtggcgaataaatactttcccgatgtcaccgtcacctgggaggtggatggcaccacccaaacaactggcatcgagaacagtaaaacaccgcagaattctgcagattgtacctacaacctcagcagcactctgacactgaccagcacacagtacaacagccacaaagagtacacctgcaaggtgacccagggcacgacctcagtcgtccagagcttcaataggggtgactgttag

SEQ ID NO: 144 - protein, 104 aa, Artificial Sequence
  source: /note="Description of Artificial Sequence: Synthetic polypeptide"
GDPVAPTVLIFPPSADLVATGTVTIVCVANKYFPDVTVTWEVDGTTQTTGIENSKTPQNSADCTYNLSSTLTLTSTQYNSHKEYTCKVTQGTTSVVQSFNRGDC

SEQ ID NO: 145 - DNA, 24 bp, Artificial Sequence
  source: /note="Description of Artificial Sequence: Synthetic oligonucleotide"
ggattctccctcaatagctatgcg

SEQ ID NO: 146 - protein, 8 aa, Artificial Sequence
  source: /note="Description of Artificial Sequence: Synthetic peptide"
GFSLNSYA

SEQ ID NO: 147 - DNA, 21 bp, Artificial Sequence
  source: /note="Description of Artificial Sequence: Synthetic oligonucleotide"
attactactggtggtaccaca

SEQ ID NO: 148 - protein, 7 aa, Artificial Sequence
  source: /note="Description of Artificial Sequence: Synthetic peptide"
ITTGGTT

SEQ ID NO: 149 - DNA, 51 bp, Artificial Sequence
  source: /note="Description of Artificial Sequence: Synthetic oligonucleotide"
gatcgggttaaaagctacgatgactatggtgatttagatgctttcgagccc

SEQ ID NO: 150 - protein, 20 aa, Artificial Sequence
  source: /note="Description of Artificial Sequence: Synthetic peptide"
DRVKSYDDYGDLDAFEPWGP

SEQ ID NO: 151 - DNA, 24 bp, Artificial Sequence
  source: /note="Description of Artificial Sequence: Synthetic oligonucleotide"
ggcttttccctgaacagctacgct

SEQ ID NO: 152 - protein, 8 aa, Artificial Sequence
  source: /note="Description of Artificial Sequence: Synthetic peptide"
GFSLNSYA

SEQ ID NO: 153 - DNA, 21 bp, Artificial Sequence
  source: /note="Description of Artificial Sequence: Synthetic oligonucleotide"
attaccacaggagggactacc

SEQ ID NO: 154 - protein, 7 aa, Artificial Sequence
  source: /note="Description of Artificial Sequence: Synthetic peptide"
ITTGGTT

SEQ ID NO: 155 - DNA, 51 bp, Artificial Sequence
  source: /note="Description of Artificial Sequence: Synthetic oligonucleotide"
gatcgggtgaaatcttacgacgattatggagacctggatgctttcgaacca

SEQ ID NO: 156 - protein, 20 aa, Artificial Sequence
  source: /note="Description of Artificial Sequence: Synthetic peptide"
DRVKSYDDYGDLDAFEPWGP

SEQ ID NO: 157 - DNA, 24 bp, Artificial Sequence
  source: /note="Description of Artificial Sequence: Synthetic oligonucleotide"
ggattctccttcagtagcagctac

SEQ ID NO: 158 - protein, 8 aa, Artificial Sequence
  source: /note="Description of Artificial Sequence: Synthetic peptide"
GFSFSSSY

SEQ ID NO: 159 - DNA, 27 bp, Artificial Sequence
  source: /note="Description of Artificial Sequence: Synthetic oligonucleotide"
atttatggtggtagtagtggtaccact

SEQ ID NO: 160 - protein, 9 aa, Artificial Sequence
  source: /note="Description of Artificial Sequence: Synthetic peptide"
IYGGSSGTT

SEQ ID NO: 161 - DNA, 33 bp, Artificial Sequence
  source: /note="Description of Artificial Sequence: Synthetic oligonucleotide"
gtgactaatggtggtgattgggattttaaattg

SEQ ID NO: 162 - protein, 11 aa, Artificial Sequence
  source: /note="Description of Artificial Sequence: Synthetic peptide"
VTNGGDWDFKL

SEQ ID NO: 163 - DNA, 24 bp, Artificial Sequence
  source: /note="Description of Artificial Sequence: Synthetic oligonucleotide"
ggaatcgacctcagtaattatgca

SEQ ID NO: 164 - protein, 8 aa, Artificial Sequence
  source: /note="Description of Artificial Sequence: Synthetic peptide"
GIDLSNYA

SEQ ID NO: 165 - DNA, 21 bp, Artificial Sequence
  source: /note="Description of Artificial Sequence: Synthetic oligonucleotide"
attagtagtaatgataagaca

SEQ ID NO: 166 - protein, 7 aa, Artificial Sequence
  source: /note="Description of Artificial Sequence: Synthetic peptide"
ISSNDKT

SEQ ID NO: 167 - DNA, 39 bp, Artificial Sequence
  source: /note="Description of Artificial Sequence: Synthetic oligonucleotide"
gctgctatgcctggtggtttaaagaatgctttcgatccc

SEQ ID NO: 168 - protein, 13 aa, Artificial Sequence
  source: /note="Description of Artificial Sequence: Synthetic peptide"
AAMPGGLKNAFDP

SEQ ID NO: 169 - DNA, 24 bp, Artificial Sequence
  source: /note="Description of Artificial Sequence: Synthetic oligonucleotide"
ggcattgatctgtctaactacgct

SEQ ID NO: 170 - protein, 8 aa, Artificial Sequence
  source: /note="Description of Artificial Sequence: Synthetic peptide"
GIDLSNYA

SEQ ID NO: 171 - DNA, 21 bp, Artificial Sequence
  source: /note="Description of Artificial Sequence: Synthetic oligonucleotide"
attagctccaatgacaagacc

SEQ ID NO: 172 - protein, 7 aa, Artificial Sequence
  source: /note="Description of Artificial Sequence: Synthetic peptide"
ISSNDKT

SEQ ID NO: 173 - DNA, 39 bp, Artificial Sequence
  source: /note="Description of Artificial Sequence: Synthetic oligonucleotide"
gccgctatgcctggcggactgaagaacgcatttgatcct

SEQ ID NO: 174 - protein, 13 aa, Artificial Sequence
  source: /note="Description of Artificial Sequence: Synthetic peptide"
AAMPGGLKNAFDP

SEQ ID NO: 175 - DNA, 24 bp, Artificial Sequence
  source: /note="Description of Artificial Sequence: Synthetic oligonucleotide"
ggaatctccctcagtagcgatgca

SEQ ID NO: 176 - protein, 8 aa, Artificial Sequence
  source: /note="Description of Artificial Sequence: Synthetic peptide"
GISLSSDA

SEQ ID NO: 177 - DNA, 21 bp, Artificial Sequence
  source: /note="Description of Artificial Sequence: Synthetic oligonucleotide"
attaatggtggtggtaacaca

SEQ ID NO: 178 - protein, 7 aa, Artificial Sequence
  source: /note="Description of Artificial Sequence: Synthetic peptide"
INGGGNT

SEQ ID NO: 179 - DNA, 54 bp, Artificial Sequence
  source: /note="Description of Artificial Sequence: Synthetic oligonucleotide"
ggcattcaacatggtggtggtaatagtgattattattattacggcatggacctc

SEQ ID NO: 180 - protein, 18 aa, Artificial Sequence
  source: /note="Description of Artificial Sequence: Synthetic peptide"
GIQHGGGNSDYYYYGMDL

SEQ ID NO: 181 - DNA, 24 bp, Artificial Sequence
  source: /note="Description of Artificial Sequence: Synthetic oligonucleotide"
ggaatttccctctcctccgacgcg

SEQ ID NO: 182 - protein, 8 aa, Artificial Sequence
  source: /note="Description of Artificial Sequence: Synthetic peptide"
GISLSSDA

SEQ ID NO: 183 - DNA, 21 bp, Artificial Sequence
  source: /note="Description of Artificial Sequence: Synthetic oligonucleotide"
atcaacggcggcggaaacacc

SEQ ID NO: 184 - protein, 7 aa, Artificial Sequence
  source: /note="Description of Artificial Sequence: Synthetic peptide"
INGGGNT

SEQ ID NO: 185 - DNA, 54 bp, Artificial Sequence
  source: /note="Description of Artificial Sequence: Synthetic oligonucleotide"
ggcatccagcacggtggtggaaacagcgactactactactatgggatggatctg

SEQ ID NO: 186 - protein, 18 aa, Artificial Sequence
  source: /note="Description of Artificial Sequence: Synthetic peptide"
GIQHGGGNSDYYYYGMDL

SEQ ID NO: 187 - DNA, 24 bp, Artificial Sequence
  source: /note="Description of Artificial Sequence: Synthetic oligonucleotide"
ggattctccctcagtaactatgca

SEQ ID NO: 188 - protein, 8 aa, Artificial Sequence
  source: /note="Description of Artificial Sequence: Synthetic peptide"
GFSLSNYA

SEQ ID NO: 189 - DNA, 21 bp, Artificial Sequence
  source: /note="Description of Artificial Sequence: Synthetic oligonucleotide"
attagtactggcggtatcaca

SEQ ID NO: 190 - protein, 7 aa, Artificial Sequence
  source: /note="Description of Artificial Sequence: Synthetic peptide"
ISTGGIT

SEQ ID NO: 191 - DNA, 39 bp, Artificial Sequence
  source: /note="Description of Artificial Sequence: Synthetic oligonucleotide"
aatgctggtggtagttatattttctattattttgacttg

SEQ ID NO: 192 - protein, 13 aa, Artificial Sequence
  source: /note="Description of Artificial Sequence: Synthetic peptide"
NAGGSYIFYYFDL

SEQ ID NO: 193 - DNA, 24 bp, Artificial Sequence
  source: /note="Description of Artificial Sequence: Synthetic oligonucleotide"
ggattctccctcagtaactatgca

SEQ ID NO: 194 - protein, 8 aa, Artificial Sequence
  source: /note="Description of Artificial Sequence: Synthetic peptide"
GFSLSNYA

SEQ ID NO: 195 - DNA, 21 bp, Artificial Sequence
  source: /note="Description of Artificial Sequence: Synthetic oligonucleotide"
attagtactggcggtatcaca

SEQ ID NO: 196 - protein, 7 aa, Artificial Sequence
  source: /note="Description of Artificial Sequence: Synthetic peptide"
ISTGGIT

SEQ ID NO: 197 - DNA, 39 bp, Artificial Sequence
  source: /note="Description of Artificial Sequence: Synthetic oligonucleotide"
aatgctggtggtagttatattttctattatttcgacttg

SEQ ID NO: 198 - protein, 13 aa, Artificial Sequence
  source: /note="Description of Artificial Sequence: Synthetic peptide"
NAGGSYIFYYFDL

SEQ ID NO: 199 - DNA, 24 bp, Artificial Sequence
  source: /note="Description of Artificial Sequence: Synthetic oligonucleotide"
ggattctccctcagtagttaccac

SEQ ID NO: 200 - protein, 8 aa, Artificial Sequence
  source: /note="Description of Artificial Sequence: Synthetic peptide"
GFSLSSYH

SEQ ID NO: 201 - DNA, 21 bp, Artificial Sequence
  source: /note="Description of Artificial Sequence: Synthetic oligonucleotide"
attactgctatgagtcgcaca

SEQ ID NO: 202 - protein, 7 aa, Artificial Sequence
  source: /note="Description of Artificial Sequence: Synthetic peptide"
ITAMSRT

SEQ ID NO: 203 - DNA, 24 bp, Artificial Sequence
  source: /note="Description of Artificial Sequence: Synthetic oligonucleotide"
gaacctggttttgttagtaacatc

SEQ ID NO: 204 - protein, 8 aa, Artificial Sequence
  source: /note="Description of Artificial Sequence: Synthetic peptide"
EPGFVSNI

SEQ ID NO: 205 - DNA, 24 bp, Artificial Sequence
  source: /note="Description of Artificial Sequence: Synthetic oligonucleotide"
ggattctccctcagtagctatgca

SEQ ID NO: 206 - protein, 8 aa, Artificial Sequence
  source: /note="Description of Artificial Sequence: Synthetic peptide"
GFSLSSYA

SEQ ID NO: 207 - DNA, 21 bp, Artificial Sequence
  source: /note="Description of Artificial Sequence: Synthetic oligonucleotide"
attagtactggtggtattaca

SEQ ID NO: 208 - protein, 7 aa, Artificial Sequence
  source: /note="Description of Artificial Sequence: Synthetic peptide"
ISTGGIT

SEQ ID NO: 209 - DNA, 39 bp, Artificial Sequence
  source: /note="Description of Artificial Sequence: Synthetic oligonucleotide"
gtgggtagtagtggttatcttttctacttctttaacttg

SEQ ID NO: 210 - protein, 13 aa, Artificial Sequence
  source: /note="Description of Artificial Sequence: Synthetic peptide"
VGSSGYLFYFFNL

SEQ ID NO: 211 - DNA, 24 bp, Artificial Sequence
  source: /note="Description of Artificial Sequence: Synthetic oligonucleotide"
ggattctccctcagtaggtataca

SEQ ID NO: 212 - protein, 8 aa, Artificial Sequence
  source: /note="Description of Artificial Sequence: Synthetic peptide"
GFSLSRYT

SEQ ID NO: 213 - DNA, 21 bp, Artificial Sequence
  source: /note="Description of Artificial Sequence: Synthetic oligonucleotide"
atagatagtagtagtagtgca

SEQ ID NO: 214 - protein, 7 aa, Artificial Sequence
  source: /note="Description of Artificial Sequence: Synthetic peptide"
IDSSSSA

SEQ ID NO: 215 - DNA, 54 bp, Artificial Sequence
  source: /note="Description of Artificial Sequence: Synthetic oligonucleotide"
gacagagtcctaagctacgatgactatggtgatttgcccgatggtttcgatccc

SEQ ID NO: 216 - protein, 18 aa, Artificial Sequence
  source: /note="Description of Artificial Sequence: Synthetic peptide"
DRVLSYDDYGDLPDGFDP

SEQ ID NO: 217 - DNA, 24 bp, Artificial Sequence
  source: /note="Description of Artificial Sequence: Synthetic oligonucleotide"
gggtttagcctgtcccgatacacc

SEQ ID NO: 218 - protein, 8 aa, Artificial Sequence
  source: /note="Description of Artificial Sequence: Synthetic peptide"
GFSLSRYT

SEQ ID NO: 219 - DNA, 21 bp, Artificial Sequence
  source: /note="Description of Artificial Sequence: Synthetic oligonucleotide"
attgacagctcctctagtgcc

SEQ ID NO: 220 - protein, 7 aa, Artificial Sequence
  source: /note="Description of Artificial Sequence: Synthetic peptide"
IDSSSSA

SEQ ID NO: 221 - DNA, 54 bp, Artificial Sequence
  source: /note="Description of Artificial Sequence: Synthetic oligonucleotide"
gatagagtcctgagctacgacgattatggggacctgcctgacggctttgatcct

SEQ ID NO: 222 - protein, 18 aa, Artificial Sequence
  source: /note="Description of Artificial Sequence: Synthetic peptide"
DRVLSYDDYGDLPDGFDP

SEQ ID NO: 223 - DNA, 18 bp, Artificial Sequence
  source: /note="Description of Artificial Sequence: Synthetic oligonucleotide"
cagagcattagtagctac

SEQ ID NO: 224 - protein, 6 aa, Artificial Sequence
  source: /note="Description of Artificial Sequence: Synthetic peptide"
QSISSY

SEQ ID NO: 225 - DNA, 9 bp, Artificial Sequence
  source: /note="Description of Artificial Sequence: Synthetic oligonucleotide"
tatgcatcc

SEQ ID NO: 226 - protein, 3 aa, Artificial Sequence
  source: /note="Description of Artificial Sequence: Synthetic peptide"
YAS

SEQ ID NO: 227 - DNA, 39 bp, Artificial Sequence
  source: /note="Description of Artificial Sequence: Synthetic oligonucleotide"
ctaggtgtttatggttatagttttgatgatggtattgct

SEQ ID NO: 228 - protein, 13 aa, Artificial Sequence
  source: /note="Description of Artificial Sequence: Synthetic peptide"
LGVYGYSFDDGIA

SEQ ID NO: 229 - DNA, 18 bp, Artificial Sequence
  source: /note="Description of Artificial Sequence: Synthetic oligonucleotide"
cagagtatttccagctac

SEQ ID NO: 230 - protein, 6 aa, Artificial Sequence
  source: /note="Description of Artificial Sequence: Synthetic peptide"
QSISSY

SEQ ID NO: 231 - DNA, 9 bp, Artificial Sequence
  source: /note="Description of Artificial Sequence: Synthetic oligonucleotide"
tatgctagt

SEQ ID NO: 232 - protein, 3 aa, Artificial Sequence
  source: /note="Description of Artificial Sequence: Synthetic peptide"
YAS

SEQ ID NO: 233 - DNA, 39 bp, Artificial Sequence
  source: /note="Description of Artificial Sequence: Synthetic oligonucleotide"
ctgggggtgtacggttattctttcgacgatggcatcgca

SEQ ID NO: 234 - protein, 13 aa, Artificial Sequence
  source: /note="Description of Artificial Sequence: Synthetic peptide"
LGVYGYSFDDGIA

SEQ ID NO: 235 - DNA, 18 bp, Artificial Sequence
  source: /note="Description of Artificial Sequence: Synthetic oligonucleotide"
cagagtatttccagctac

SEQ ID NO: 236 - protein, 6 aa, Artificial Sequence
  source: /note="Description of Artificial Sequence: Synthetic peptide"
QSISSY

SEQ ID NO: 237 - DNA, 9 bp, Artificial Sequence
  source: /note="Description of Artificial Sequence: Synthetic oligonucleotide"
tatgctagt

SEQ ID NO: 238 - protein, 3 aa, Artificial Sequence
  source: /note="Description of Artificial Sequence: Synthetic peptide"
YAS

SEQ ID NO: 239 - DNA, 39 bp, Artificial Sequence; identical to SEQ ID NO: 233
  source: /note="Description of Artificial Sequence: Synthetic oligonucleotide"

SEQ ID NO: 240 - protein, 13 aa, Artificial Sequence
  source: /note="Description of Artificial Sequence: Synthetic peptide"
LGVYGYSFDDGIA

SEQ ID NO: 241 - DNA, 18 bp, Artificial Sequence
  source: /note="Description of Artificial Sequence: Synthetic oligonucleotide"
cagagtatttccagctac

SEQ ID NO: 242 - protein, 6 aa, Artificial Sequence
  source: /note="Description of Artificial Sequence: Synthetic peptide"
QSISSY

SEQ ID NO: 243 - DNA, 9 bp, Artificial Sequence
  source: /note="Description of Artificial Sequence: Synthetic oligonucleotide"
tatgctagt

SEQ ID NO: 244 - protein, 3 aa, Artificial Sequence
  source: /note="Description of Artificial Sequence: Synthetic peptide"
YAS

SEQ ID NO: 245 - DNA, 39 bp, Artificial Sequence; identical to SEQ ID NO: 233
  source: /note="Description of Artificial Sequence: Synthetic oligonucleotide"

SEQ ID NO: 246 - protein, 13 aa, Artificial Sequence
  source: /note="Description of Artificial Sequence: Synthetic peptide"
LGVYGYSFDDGIA

SEQ ID NO: 247 - DNA, 18 bp, Artificial Sequence
  source: /note="Description of Artificial Sequence: Synthetic oligonucleotide"
cagagtatttccagctac

SEQ ID NO: 248 - protein, 6 aa, Artificial Sequence
  source: /note="Description of Artificial Sequence: Synthetic peptide"
QSISSY

SEQ ID NO: 249 - DNA, 9 bp, Artificial Sequence
  source: /note="Description of Artificial Sequence: Synthetic oligonucleotide"
tatgctagt

SEQ ID NO: 250 - protein, 3 aa, Artificial Sequence
  source: /note="Description of Artificial Sequence: Synthetic peptide"
YAS

SEQ ID NO: 251 - DNA, 39 bp, Artificial Sequence; identical to SEQ ID NO: 233
  source: /note="Description of Artificial Sequence: Synthetic oligonucleotide"

SEQ ID NO: 252 - protein, 13 aa, Artificial Sequence
  source: /note="Description of Artificial Sequence: Synthetic peptide"
LGVYGYSFDDGIA

SEQ ID NO: 253 - DNA, 18 bp, Artificial Sequence
  source: /note="Description of Artificial Sequence: Synthetic oligonucleotide"
cagagtatttccagctac

SEQ ID NO: 254 - protein, 6 aa, Artificial Sequence
  source: /note="Description of Artificial Sequence: Synthetic peptide"
QSISSY

SEQ ID NO: 255 - DNA, 9 bp, Artificial Sequence
  source: /note="Description of Artificial Sequence: Synthetic oligonucleotide"
tatgctagt

SEQ ID NO: 256 - protein, 3 aa, Artificial Sequence
  source: /note="Description of Artificial Sequence: Synthetic peptide"
YAS

SEQ ID NO: 257 - DNA, 39 bp, Artificial Sequence; identical to SEQ ID NO: 233
  source: /note="Description of Artificial Sequence: Synthetic oligonucleotide"

SEQ ID NO: 258 - protein, 13 aa, Artificial Sequence
  source: /note="Description of Artificial Sequence: Synthetic peptide"
LGVYGYSFDDGIA

SEQ ID NO: 259 - DNA, 18 bp, Artificial Sequence
  source: /note="Description of Artificial Sequence: Synthetic oligonucleotide"
cagagtatttccagctac

SEQ ID NO: 260 - protein, 6 aa, Artificial Sequence
  source: /note="Description of Artificial Sequence: Synthetic peptide"
QSISSY

SEQ ID NO: 261 - DNA, 9 bp, Artificial Sequence
  source: /note="Description of Artificial Sequence: Synthetic oligonucleotide"
tatgctagt

SEQ ID NO: 262 - protein, 3 aa, Artificial Sequence
  source: /note="Description of Artificial Sequence: Synthetic peptide"
YAS

SEQ ID NO: 263 - DNA, 39 bp, Artificial Sequence; identical to SEQ ID NO: 233
  source: /note="Description of Artificial Sequence: Synthetic oligonucleotide"

SEQ ID NO: 264 - protein, 13 aa, Artificial Sequence
  source: /note="Description of Artificial Sequence: Synthetic peptide"
LGVYGYSFDDGIA

SEQ ID NO: 265 - DNA, 18 bp, Artificial Sequence
  source: /note="Description of Artificial Sequence: Synthetic oligonucleotide"
cagagtatttccagctac

SEQ ID NO: 266 - protein, 6 aa, Artificial Sequence
  source: /note="Description of Artificial Sequence: Synthetic peptide"
QSISSY

SEQ ID NO: 267 - DNA, 9 bp, Artificial Sequence
  source: /note="Description of Artificial Sequence: Synthetic oligonucleotide"
tatgctagt

SEQ ID NO: 268 - protein, 3 aa, Artificial Sequence
  source: /note="Description of Artificial Sequence: Synthetic peptide"
YAS

SEQ ID NO: 269 - DNA, 39 bp, Artificial Sequence; identical to SEQ ID NO: 233
  source: /note="Description of Artificial Sequence: Synthetic oligonucleotide"

SEQ ID NO: 270 - protein, 13 aa, Artificial Sequence
  source: /note="Description of Artificial Sequence: Synthetic peptide"
LGVYGYSFDDGIA

SEQ ID NO: 271 - DNA, 18 bp, Artificial Sequence
  source: /note="Description of Artificial Sequence: Synthetic oligonucleotide"
cagtccatctcctcctac

SEQ ID NO: 272 - protein, 6 aa, Artificial Sequence
  source: /note="Description of Artificial Sequence: Synthetic peptide"
QSISSY

SEQ ID NO: 273 - DNA, 9 bp, Artificial Sequence
  source: /note="Description of Artificial Sequence: Synthetic oligonucleotide"
tacgcctcc

SEQ ID NO: 274 - protein, 3 aa, Artificial Sequence
  source: /note="Description of Artificial Sequence: Synthetic peptide"
YAS

SEQ ID NO: 275 - DNA, 39 bp, Artificial Sequence
  source: /note="Description of Artificial Sequence: Synthetic oligonucleotide"
ctgggggtgtatggttactcgttcgacgatggaatcgca

SEQ ID NO: 276 - protein, 13 aa, Artificial Sequence
  source: /note="Description of Artificial Sequence: Synthetic peptide"
LGVYGYSFDDGIA

SEQ ID NO: 277 - DNA, 18 bp, Artificial Sequence
  source: /note="Description of Artificial Sequence: Synthetic oligonucleotide"
cagagcatctcctcatac

SEQ ID NO: 278 - protein, 6 aa, Artificial Sequence
  source: /note="Description of Artificial Sequence: Synthetic peptide"
QSISSY

SEQ ID NO: 279 - DNA, 9 bp, Artificial Sequence
  source: /note="Description of Artificial Sequence: Synthetic oligonucleotide"
tacgcctcc

SEQ ID NO: 280 - protein, 3 aa, Artificial Sequence
  source: /note="Description of Artificial Sequence: Synthetic peptide"
YAS

SEQ ID NO: 281 - DNA, 39 bp, Artificial Sequence
  source: /note="Description of Artificial Sequence: Synthetic oligonucleotide"
ctgggagtctacgggtactccttcgatgacggcattgca

SEQ ID NO: 282 - protein, 13 aa, Artificial Sequence
  source: /note="Description of Artificial Sequence: Synthetic peptide"
LGVYGYSFDDGIA

SEQ ID NO: 283 - DNA, 18 bp, Artificial Sequence
  source: /note="Description of Artificial Sequence: Synthetic oligonucleotide"
cagtcgatctcctcttac

SEQ ID NO: 284 - protein, 6 aa, Artificial Sequence
  source: /note="Description of Artificial Sequence: Synthetic peptide"
QSISSY

SEQ ID NO: 285 - DNA, 9 bp, Artificial Sequence
  source: /note="Description of Artificial Sequence: Synthetic oligonucleotide"
tacgcgtcg

SEQ ID NO: 286 - protein, 3 aa, Artificial Sequence
  source: /note="Description of Artificial Sequence: Synthetic peptide"
YAS

SEQ ID NO: 287 - DNA, 39 bp, Artificial Sequence
  source: /note="Description of Artificial Sequence: Synthetic oligonucleotide"
ctgggggtgtacggctactccttcgatgacggaatcgcc

SEQ ID NO: 288 - protein, 13 aa, Artificial Sequence
  source: /note="Description of Artificial Sequence: Synthetic peptide"
LGVYGYSFDDGIA

SEQ ID NO: 289 - DNA, 18 bp, Artificial Sequence
  source: /note="Description of Artificial Sequence: Synthetic oligonucleotide"
cagtccatctcctcatac

SEQ ID NO: 290 - protein, 6 aa, Artificial Sequence
  source: /note="Description of Artificial Sequence: Synthetic peptide"
QSISSY

SEQ ID NO: 291 - DNA, 9 bp, Artificial Sequence
  source: /note="Description of Artificial Sequence: Synthetic oligonucleotide"
tacgcttcc

SEQ ID NO: 292 - protein, 3 aa, Artificial Sequence
  source: /note="Description of Artificial Sequence: Synthetic peptide"
YAS

SEQ ID NO: 293 - DNA, 39 bp, Artificial Sequence
  source: /note="Description of Artificial Sequence: Synthetic oligonucleotide"
ttgggtgtctacggatactccttcgacgacgggatcgca

SEQ ID NO: 294 - protein, 13 aa, Artificial Sequence
  source: /note="Description of Artificial Sequence: Synthetic peptide"
LGVYGYSFDDGIA

SEQ ID NO: 295 - DNA, 18 bp, Artificial Sequence
  source: /note="Description of Artificial Sequence: Synthetic oligonucleotide"
cagtcaatttcctcgtac

SEQ ID NO: 296 - protein, 6 aa, Artificial Sequence
  source: /note="Description of Artificial Sequence: Synthetic peptide"
QSISSY

SEQ ID NO: 297 - DNA, 9 bp, Artificial Sequence
  source: /note="Description of Artificial Sequence: Synthetic oligonucleotide"
tacgcatcc

SEQ ID NO: 298 - protein, 3 aa, Artificial Sequence
  source: /note="Description of Artificial Sequence: Synthetic peptide"
YAS

SEQ ID NO: 299 - DNA, 39 bp, Artificial Sequence
  source: /note="Description of Artificial Sequence: Synthetic oligonucleotide"
ctgggggtgtacgggtactcatttgacgatggcatcgcc

SEQ ID NO: 300 - protein, 13 aa, Artificial Sequence
  source: /note="Description of Artificial Sequence: Synthetic peptide"
LGVYGYSFDDGIA

SEQ ID NO: 301 - DNA, 18 bp, Artificial Sequence
  source: /note="Description of Artificial Sequence: Synthetic oligonucleotide"
cagtccatttcgtcctac

SEQ ID NO: 302 - protein, 6 aa, Artificial Sequence
  source: /note="Description of Artificial Sequence: Synthetic peptide"
QSISSY

SEQ ID NO: 303 - DNA, 9 bp, Artificial Sequence
  source: /note="Description of Artificial Sequence: Synthetic oligonucleotide"
tacgcctcc

SEQ ID NO: 304 - protein, 3 aa, Artificial Sequence
  source: /note="Description of Artificial Sequence: Synthetic peptide"
YAS

SEQ ID NO: 305 - DNA, 39 bp, Artificial Sequence
  source: /note="Description of Artificial Sequence: Synthetic oligonucleotide"
ctgggcgtgtacggttactcgtttgatgacggcatcgcg

SEQ ID NO: 306 - protein, 13 aa, Artificial Sequence
  source: /note="Description of Artificial Sequence: Synthetic peptide"
LGVYGYSFDDGIA

SEQ ID NO: 307 - DNA, 18 bp, Artificial Sequence
  source: /note="Description of Artificial Sequence: Synthetic oligonucleotide"
cagtccatttcgagctac

SEQ ID NO: 308 - protein, 6 aa, Artificial Sequence
  source: /note="Description of Artificial Sequence: Synthetic peptide"
QSISSY

SEQ ID NO: 309 - DNA, 9 bp, Artificial Sequence
  source: /note="Description of Artificial Sequence: Synthetic oligonucleotide"
tacgcctcc

SEQ ID NO: 310 - protein, 3 aa, Artificial Sequence
  source: /note="Description of Artificial Sequence: Synthetic peptide"
YAS

SEQ ID NO: 311 - DNA, 39 bp, Artificial Sequence
  source: /note="Description of Artificial Sequence: Synthetic oligonucleotide"
ctgggggtgtacggatactcattcgacgacgggatcgcc

SEQ ID NO: 312 - protein, 13 aa, Artificial Sequence
  source: /note="Description of Artificial Sequence: Synthetic peptide"
LGVYGYSFDDGIA

SEQ ID NO: 313 - DNA, 18 bp, Artificial Sequence
  source: /note="Description of Artificial Sequence: Synthetic oligonucleotide"
cagagcattaatacctac

SEQ ID NO: 314 - protein, 6 aa, Artificial Sequence
  source: /note="Description of Artificial Sequence: Synthetic peptide"
QSINTY

SEQ ID NO: 315 - DNA, 9 bp, Artificial Sequence
  source: /note="Description of Artificial Sequence: Synthetic oligonucleotide"
agggcatcc

SEQ ID NO: 316 - protein, 3 aa, Artificial Sequence
  source: /note="Description of Artificial Sequence: Synthetic peptide"
RAS

SEQ ID NO: 317 - DNA, 36 bp, Artificial Sequence
  source: /note="Description of Artificial Sequence: Synthetic oligonucleotide"
caacagagtgttcgtgttattgatgttgataatact

SEQ ID NO: 318 - protein, 12 aa, Artificial Sequence
  source: /note="Description of Artificial Sequence: Synthetic peptide"
QQSVRVIDVDNT

SEQ ID NO: 319 - DNA, 21 bp, Artificial Sequence
  source: /note="Description of Artificial Sequence: Synthetic oligonucleotide"
cagaccattggtggtagcgac

SEQ ID NO: 320 - protein, 7 aa, Artificial Sequence
  source: /note="Description of Artificial Sequence: Synthetic peptide"
QTIGGSD

SEQ ID NO: 321 - DNA, 9 bp, Artificial Sequence
  source: /note="Description of Artificial Sequence: Synthetic oligonucleotide"
tatgcaacc

SEQ ID NO: 322 - protein, 3 aa, Artificial Sequence
  source: /note="Description of Artificial Sequence: Synthetic peptide"
YAT

SEQ ID NO: 323 - DNA, 36 bp, Artificial Sequence
  source: /note="Description of Artificial Sequence: Synthetic oligonucleotide"
ctaggtggttatgctgctgcttcttacagaactgct

SEQ ID NO: 324 - protein, 12 aa, Artificial Sequence
  source: /note="Description of Artificial Sequence: Synthetic peptide"
LGGYAAASYRTA

SEQ ID NO: 325 - DNA, 21 bp, Artificial Sequence
  source: /note="Description of Artificial Sequence: Synthetic oligonucleotide"
cagaccattggcgggagcgac

SEQ ID NO: 326 - protein, 7 aa, Artificial Sequence
  source: /note="Description of Artificial Sequence: Synthetic peptide"
QTIGGSD

SEQ ID NO: 327 - DNA, 9 bp, Artificial Sequence
  source: /note="Description of Artificial Sequence: Synthetic oligonucleotide"
tatgctaca

SEQ ID NO: 328 - protein, 3 aa, Artificial Sequence
  source: /note="Description of Artificial Sequence: Synthetic peptide"
YAT

SEQ ID NO: 329 - DNA, 36 bp, Artificial Sequence
  source: /note="Description of Artificial Sequence: Synthetic oligonucleotide"
ctggggggctatgccgccgcaagctaccgcaccgcc

SEQ ID NO: 330 - protein, 12 aa, Artificial Sequence
  source: /note="Description of Artificial Sequence: Synthetic peptide"
LGGYAAASYRTA

SEQ ID NO: 331 - DNA, 21 bp, Artificial Sequence
  source: /note="Description of Artificial Sequence: Synthetic oligonucleotide"
cagaccattggcgggagcgac

SEQ ID NO: 332 - protein, 7 aa, Artificial Sequence
  source: /note="Description of Artificial Sequence: Synthetic peptide"
QTIGGSD

SEQ ID NO: 333 - DNA, 9 bp, Artificial Sequence
  source: /note="Description of Artificial Sequence: Synthetic oligonucleotide"
tatgctaca

SEQ ID NO: 334 - protein, 3 aa, Artificial Sequence
  source: /note="Description of Artificial Sequence: Synthetic peptide"
YAT

SEQ ID NO: 335 - DNA, 36 bp, Artificial Sequence; identical to SEQ ID NO: 329
  source: /note="Description of Artificial Sequence: Synthetic oligonucleotide"

SEQ ID NO: 336 - protein, 12 aa, Artificial Sequence
  source: /note="Description of Artificial Sequence: Synthetic peptide"
LGGYAAASYRTA

SEQ ID NO: 337 - DNA, 18 bp, Artificial Sequence
  source: /note="Description of Artificial Sequence: Synthetic oligonucleotide"
cagagcattagtagtgtc

SEQ ID NO: 338 - protein, 6 aa, Artificial Sequence
  source: /note="Description of Artificial Sequence: Synthetic peptide"
QSISSV

SEQ ID NO: 339 - DNA, 9 bp, Artificial Sequence
  source: /note="Description of Artificial Sequence: Synthetic oligonucleotide"
ctggcatcc

SEQ ID NO: 340 - protein, 3 aa, Artificial Sequence
  source: /note="Description of Artificial Sequence: Synthetic peptide"
LAS

SEQ ID NO: 341 - DNA, 42 bp, Artificial Sequence
  source: /note="Description of Artificial Sequence: Synthetic oligonucleotide"
caaaccaattatggtactagtagtagtaattatggttttgct

SEQ ID NO: 342 - protein, 14 aa, Artificial Sequence
  source: /note="Description of Artificial Sequence: Synthetic peptide"
QTNYGTSSSNYGFA

SEQ ID NO: 343 - DNA, 18 bp, Artificial Sequence
  source: /note="Description of Artificial Sequence: Synthetic oligonucleotide"
cagtcaattagcagcgtg

SEQ ID NO: 344 - protein, 6 aa, Artificial Sequence
  source: /note="Description of Artificial Sequence: Synthetic peptide"
QSISSV

SEQ ID NO: 345 - DNA, 9 bp, Artificial Sequence
  source: /note="Description of Artificial Sequence: Synthetic oligonucleotide"
ttggcctcc

SEQ ID NO: 346 - protein, 3 aa, Artificial Sequence
  source: /note="Description of Artificial Sequence: Synthetic peptide"
LAS

SEQ ID NO: 347 - DNA, 42 bp, Artificial Sequence
  source: /note="Description of Artificial Sequence: Synthetic oligonucleotide"
caaaccaactacggaacctccagctccaactacggctttgcc

SEQ ID NO: 348 - protein, 14 aa, Artificial Sequence
  source: /note="Description of Artificial Sequence: Synthetic peptide"
QTNYGTSSSNYGFA

SEQ ID NO: 349 - DNA, 18 bp, Artificial Sequence
  source: /note="Description of Artificial Sequence: Synthetic oligonucleotide"
cagtcaattagcagcgtg

SEQ ID NO: 350 - protein, 6 aa, Artificial Sequence
  source: /note="Description of Artificial Sequence: Synthetic peptide"
QSISSV

SEQ ID NO: 351 - DNA, 9 bp, Artificial Sequence
  source: /note="Description of Artificial Sequence: Synthetic oligonucleotide"
ttggcctcc

SEQ ID NO: 352 - protein, 3 aa, Artificial Sequence
  source: /note="Description of Artificial Sequence: Synthetic peptide"
LAS

SEQ ID NO: 353 - DNA, 42 bp, Artificial Sequence; identical to SEQ ID NO: 347
  source: /note="Description of Artificial Sequence: Synthetic oligonucleotide"

SEQ ID NO: 354 - protein, 14 aa, Artificial Sequence
  source: /note="Description of Artificial Sequence: Synthetic peptide"
QTNYGTSSSNYGFA

SEQ ID NO: 355 - DNA, 18 bp, Artificial Sequence
  source: /note="Description of Artificial Sequence: Synthetic oligonucleotide"
cagtcaattagcagcgtg

SEQ ID NO: 356 - protein, 6 aa, Artificial Sequence
  source: /note="Description of Artificial Sequence: Synthetic peptide"
QSISSV

SEQ ID NO: 357 - DNA, 9 bp, Artificial Sequence
  source: /note="Description of Artificial Sequence: Synthetic oligonucleotide"
ttggcctcc

SEQ ID NO: 358 - protein, 3 aa, Artificial Sequence
  source: /note="Description of Artificial Sequence: Synthetic peptide"
LAS

SEQ ID NO: 359 - DNA, 42 bp, Artificial Sequence; identical to SEQ ID NO: 347
  source: /note="Description of Artificial Sequence: Synthetic oligonucleotide"

SEQ ID NO: 360 - protein, 14 aa, Artificial Sequence
  source: /note="Description of Artificial Sequence: Synthetic peptide"
QTNYGTSSSNYGFA

SEQ ID NO: 361 - DNA, 18 bp, Artificial Sequence
  source: /note="Description of Artificial Sequence: Synthetic oligonucleotide"
cagagcatttacagttat

SEQ ID NO: 362 - protein, 6 aa, Artificial Sequence
  source: /note="Description of Artificial Sequence: Synthetic peptide"
QSIYSY

SEQ ID NO: 363 - DNA, 9 bp, Artificial Sequence
  source: /note="Description of Artificial Sequence: Synthetic oligonucleotide"
tctgcatcc

SEQ ID NO: 364 - protein, 3 aa, Artificial Sequence
  source: /note="Description of Artificial Sequence: Synthetic peptide"
SAS

SEQ ID NO: 365 - DNA, 30 bp, Artificial Sequence
  source: /note="Description of Artificial Sequence: Synthetic oligonucleotide"
caaacctattatgatattgttactagtact

SEQ ID NO: 366 - protein, 10 aa, Artificial Sequence
  source: /note="Description of Artificial Sequence: Synthetic peptide"
QTYYDIVTST

SEQ ID NO: 367 - DNA, 18 bp, Artificial Sequence
  source: /note="Description of Artificial Sequence: Synthetic oligonucleotide"
cagagcatttacagttat

SEQ ID NO: 368 - protein, 6 aa, Artificial Sequence
  source: /note="Description of Artificial Sequence: Synthetic peptide"
QSIYSY

SEQ ID NO: 369 - DNA, 9 bp, Artificial Sequence
  source: /note="Description of Artificial Sequence: Synthetic oligonucleotide"
tctgcatcc

SEQ ID NO: 370 - protein, 3 aa, Artificial Sequence
  source: /note="Description of Artificial Sequence: Synthetic peptide"
SAS

SEQ ID NO: 371 - DNA, 30 bp, Artificial Sequence; identical to SEQ ID NO: 365
  source: /note="Description of Artificial Sequence: Synthetic oligonucleotide"

SEQ ID NO: 372 - protein, 10 aa, Artificial Sequence
  source: /note="Description of Artificial Sequence: Synthetic peptide"
QTYYDIVTST

SEQ ID NO: 373 - DNA, 18 bp, Artificial Sequence
  source: /note="Description of Artificial Sequence: Synthetic oligonucleotide"
cagaacatttacagcaat

SEQ ID NO: 374 - protein, 6 aa, Artificial Sequence
  source: /note="Description of Artificial Sequence: Synthetic peptide"
QNIYSN

SEQ ID NO: 375 - DNA, 9 bp, Artificial Sequence
  source: /note="Description of Artificial Sequence: Synthetic oligonucleotide"
gatgcatcc

SEQ ID NO: 376 - protein, 3 aa, Artificial Sequence
  source: /note="Description of Artificial Sequence: Synthetic peptide"
DAS

SEQ ID NO: 377 - DNA, 30 bp, Artificial Sequence
  source: /note="Description of Artificial Sequence: Synthetic oligonucleotide"
caaagtattagtagtgttgacaataatgtt

SEQ ID NO: 378 - protein, 10 aa, Artificial Sequence
  source: /note="Description of Artificial Sequence: Synthetic peptide"
QSISSVDNNV

SEQ ID NO: 379 - DNA, 18 bp, Artificial Sequence
  source: /note="Description of Artificial Sequence: Synthetic oligonucleotide"
cagaacattaagagctac

SEQ ID NO: 380 - protein, 6 aa, Artificial Sequence
  source: /note="Description of Artificial Sequence: Synthetic peptide"
QNIKSY

SEQ ID NO: 381 - DNA, 9 bp, Artificial Sequence
  source: /note="Description of Artificial Sequence: Synthetic oligonucleotide"
gaagcatcc

SEQ ID NO: 382 - protein, 3 aa, Artificial Sequence
  source: /note="Description of Artificial Sequence: Synthetic peptide"
EAS

SEQ ID NO: 383 - DNA, 30 bp, Artificial Sequence
  source: /note="Description of Artificial Sequence: Synthetic oligonucleotide"
caaagctattatgctgctagtagtaatgct

SEQ ID NO: 384 - protein, 10 aa, Artificial Sequence
  source: /note="Description of Artificial Sequence: Synthetic peptide"
QSYYAASSNA

SEQ ID NO: 385 - DNA, 18 bp, Artificial Sequence
  source: /note="Description of Artificial Sequence: Synthetic oligonucleotide"
cagagcattagtaactac

SEQ ID NO: 386 - protein, 6 aa, Artificial Sequence
  source: /note="Description of Artificial Sequence: Synthetic peptide"
QSISNY

SEQ ID NO: 387 - DNA, 9 bp, Artificial Sequence
  source: /note="Description of Artificial Sequence: Synthetic oligonucleotide"
gctgcatcc

SEQ ID NO: 388 - protein, 3 aa, Artificial Sequence
  source: /note="Description of Artificial Sequence: Synthetic peptide"
AAS

SEQ ID NO: 389 - DNA, 39 bp, Artificial Sequence
  source: /note="Description of Artificial Sequence: Synthetic oligonucleotide"
ctaggagtttatagtattagtactgatgatggagctgct

SEQ ID NO: 390 - protein, 13 aa, Artificial Sequence
  source: /note="Description of Artificial Sequence: Synthetic peptide"
LGVYSISTDDGAA

SEQ ID NO: 391 - DNA, 18 bp, Artificial Sequence
  source: /note="Description of Artificial Sequence: Synthetic oligonucleotide"
cagagcatcagcaactac

SEQ ID NO: 392 - protein, 6 aa, Artificial Sequence
  source: /note="Description of Artificial Sequence: Synthetic peptide"
QSISNY

SEQ ID NO: 393 - DNA, 9 bp, Artificial Sequence
  source: /note="Description of Artificial Sequence: Synthetic oligonucleotide"
gccgcttct

SEQ ID NO: 394 - protein, 3 aa, Artificial Sequence
  source: /note="Description of Artificial Sequence: Synthetic peptide"
AAS

SEQ ID NO: 395 - DNA, 39 bp, Artificial Sequence
  source: /note="Description of Artificial Sequence: Synthetic oligonucleotide"
ctgggcgtctattcaatctcaactgacgacggagccgca

SEQ ID NO: 396 - protein, 13 aa, Artificial Sequence
  source: /note="Description of Artificial Sequence: Synthetic peptide"
LGVYSISTDDGAA

SEQ ID NO: 397 - DNA, 18 bp, Artificial Sequence
  source: /note="Description of Artificial Sequence: Synthetic oligonucleotide"
cagagcatcagcaactac

SEQ ID NO: 398 - protein, 6 aa, Artificial Sequence
  source: /note="Description of Artificial Sequence: Synthetic peptide"
QSISNY

SEQ ID NO: 399 - DNA, 9 bp, Artificial Sequence
  source: /note="Description of Artificial Sequence: Synthetic oligonucleotide"
gccgcttct

SEQ ID NO: 400 - protein, 3 aa, Artificial Sequence
  source: /note="Description of Artificial Sequence: Synthetic peptide"
AAS

SEQ ID NO: 401 - DNA, 39 bp, Artificial Sequence; identical to SEQ ID NO: 395
  source: /note="Description of Artificial Sequence: Synthetic oligonucleotide"

SEQ ID NO: 402 - protein, 13 aa, Artificial Sequence
  source: /note="Description of Artificial Sequence: Synthetic peptide"
LGVYSISTDDGAA

SEQ ID NO: 403 - protein, 100 aa, Oryctolagus cuniculus
AQVLTQTESPVSAPVGGTVTINCQASQSVYDNNWLSWYQQKPGQPPKLLIYDASKLASGVPSRFSGSGSGTQFTLTISGVQCDDAATYYCQGSYYSSGWY

SEQ ID NO: 404 - protein, 95 aa, Homo sapiens
DIQMTQSPSTLSASVGDRVTITCRASQSISSWLAWYQQKPGKAPKLLIYDASSLESGVPSRFSGSGSGTEFTLTISSLQPDDFATYYCQQYNSYS

SEQ ID NO: 405 - protein, 103 aa, Oryctolagus cuniculus
DPVAPTVLIFPPAADQVATGTVTIVCVANKYFPDVTVTWEVDGTTQTTGIENSKTPQNSADCTYNLSSTLTLTSTQYNSHKEYTCKVTQGTTSVVQSFNRGDC

SEQ ID NO: 406 - protein, 107 aa, Homo sapiens [sequence omitted]

SEQ ID NO: 407 - protein, 70 aa, Artificial Sequence
  source: /note="Description of Artificial Sequence: Synthetic polypeptide"
ALVMTQTPSPVSAAVGGTVTISCWFQQKPGQPPKLLIYGVPSRFKGSGSGTQFTLTISGVECDDAATYYC

SEQ ID NO: 408 - protein, 70 aa, Artificial Sequence
  source: /note="Description of Artificial Sequence: Synthetic polypeptide"
AQVLTQTESPVSAPVGGTVTINCWYQQKPGQPPKLLIYGVPSRFSGSGSGTQFTLTISGVQCDDAATYYC

SEQ ID NO: 409 - protein, 70 aa, Artificial Sequence; identical to SEQ ID NO: 408
  source: /note="Description of Artificial Sequence: Synthetic polypeptide"

SEQ ID NO: 410 - protein, 70 aa, Artificial Sequence
  source: /note="Description of Artificial Sequence: Synthetic polypeptide"
AQVLTQTPASVSAAVGGTVTINCWYQQKLGQPPKLLIYGVPSRFKGSGSGTEYTLTISGVQCDDAATYYC

SEQ ID NO: 411 - protein, 70 aa, Artificial Sequence
  source: /note="Description of Artificial Sequence: Synthetic polypeptide"
AQVMTQTPASVSAAVGGTVTIICWYQQKLGQPPKLLIYGVPSRFKGSGSGTEYTLTISGVQCDDAATYYC

SEQ ID NO: 412 - protein, 70 aa, Artificial Sequence
  source: /note="Description of Artificial Sequence: Synthetic polypeptide"
AIDMTQTPASVEAAVGGTITINCWYQQKPGQPPKLLIYGVPSRFSGSGSGTQFTLTISGVQCDDAATYYC

SEQ ID NO: 413 - protein, 70 aa, Artificial Sequence
  source: /note="Description of Artificial Sequence: Synthetic polypeptide"
DPVMTQTPSSTSAAVGGTVTINCWFQQKPGQPPKLLIYGVPSRFSGSGSGKQFTLTISGVQCDDAATYYC

SEQ ID NO: 414 - protein, 70 aa, Artificial Sequence
  source: /note="Description of Artificial Sequence: Synthetic polypeptide"
DGVMTQTPAPVSAAVGGTVTINCWYQQKPGQPPKLLIYGVPSRFNGSGSGTQFTLTISGVQCDDAATYYC

SEQ ID NO: 415 - protein, 70 aa, Artificial Sequence
  source: /note="Description of Artificial Sequence: Synthetic polypeptide"
DVVMTQTPSPVSAAVGGTVTINCWYQQKPGQPPKLLIYGVPSRFSGSGSGTQFTLTISGVQCDDAATYYC

SEQ ID NO: 416 - protein, 70 aa, Artificial Sequence
  source: /note="Description of Artificial Sequence: Synthetic polypeptide"
DPMLTQTASPVSAAVGSTVTISCWFQQKPGQPPKLLIYGVPSRFKGSGSGTQFTLTINGVQCDDAATYYC

SEQ ID NO: 417 - protein, 70 aa, Artificial Sequence
  source: /note="Description of Artificial Sequence: Synthetic polypeptide"
AAVLTQTPSPVSVAVGGTVTINCWFQQKPGQPPKLLIYGVSSRFKGSGSGTQFTLTISGVQCDDAATYYC

SEQ ID NO: 418 - protein, 70 aa, Artificial Sequence
  source: /note="Description of Artificial Sequence: Synthetic polypeptide"
DVVMTQTPSSKSAAVGDTVTIKCWYQQKPGQPPKLLIYGVPSRFKGSGSGTQFTLTISDLECADAATYYC

SEQ ID NO: 419 - protein, 70 aa, Artificial Sequence; identical to SEQ ID NO: 416
  source: /note="Description of Artificial Sequence: Synthetic polypeptide"

SEQ ID NO: 420 - protein, 70 aa, Artificial Sequence
  source: /note="Description of Artificial Sequence: Synthetic polypeptide"
DPVLTQTASPVSAAVGGTVTISCWYQQKPGQPPKLLIYGVPSRFKGSGSGTQFTLTISGVQCDDAATYYC

SEQ ID NO: 421 - protein, 26 aa, Artificial Sequence
  source: /note="Description of Artificial Sequence: Synthetic peptide"
ALVMTQTPSPVSAAVGSTVTISCWFQ

SEQ ID NO: 422 - protein, 43 aa, Artificial Sequence
  source: /note="Description of Artificial Sequence: Synthetic polypeptide"
KPGQPPKLLIYGVPSRFKGSGFGTQFTLTISGAQCDDAATYYC

SEQ ID NO: 423 - protein, 70 aa, Artificial Sequence
  source: /note="Description of Artificial Sequence: Synthetic polypeptide"
DPMLTQTASPVSAAVGSTVTISCWYQQKPGQPPKLLIYGVPSRFKGSGSGTQFTLTISGVQCDDAATYYC

SEQ ID NO: 424 - protein, 70 aa, Artificial Sequence
  source: /note="Description of Artificial Sequence: Synthetic polypeptide"
AQGPTQTPSSVSAAVGGTVTINCWYQQKPGQPPKLLIYGVPSRFKGSGSGTQFTLTISDVQCDDAATYYC

SEQ ID NO: 425 - protein, 70 aa, Artificial Sequence
  source: /note="Description of Artificial Sequence: Synthetic polypeptide"
DPMLTQTASPVSAAVGSTVTISCWFQQKPGQPPKLLIYGVSSRFKGSGSGTQFTLTISGVQCDDAATYYC

SEQ ID NO: 426 - protein, 70 aa, Artificial Sequence
  source: /note="Description of Artificial Sequence: Synthetic polypeptide"
ALVMTQTPASVEAAVGGTVTIKCWYQQKPGQPPKLLIYGVSSRFKGSGSGTEYTLTISGVQCADAATYYC

SEQ ID NO: 427 - protein, 70 aa, Artificial Sequence
  source: /note="Description of Artificial Sequence: Synthetic polypeptide"
AAVMTQTPSPVSVAVGGTVTINCWFQQKPGQPPKLLIYGVSSRFKGSGSGTQFTLTISGVQCDDAATYYC

SEQ ID NO: 428 - protein, 70 aa, Artificial Sequence
  source: /note="Description of Artificial Sequence: Synthetic polypeptide"
AAVLTQTPSPVSAAVGGTVTIKCWYQQKPGQPPKLLIYGVPDRFSGSGSGTQFTLTISGVQCDDAATYYC

SEQ ID NO: 429 - protein, 70 aa, Artificial Sequence; identical to SEQ ID NO: 423
  source: /note="Description of Artificial Sequence: Synthetic polypeptide"

SEQ ID NO: 430 - protein, 70 aa, Artificial Sequence
  source: /note="Description of Artificial Sequence: Synthetic polypeptide"
YVMMTQTPSSVSEAVGGTVTIYCWYQQKPGQPPKLLIYGVPSRFRGSGSGTQFTLTISGMKAEDVATYYC

SEQ ID NO: 431 - protein, 70 aa, Artificial Sequence
  source: /note="Description of Artificial Sequence: Synthetic polypeptide"
DPMLTQTASPVSAAVGSTVTISCWFQQKPGQPPKLLIYGVPSRFKGSGSGTQFTLTISGVQCDDAATYYC

SEQ ID NO: 432 - protein, 70 aa, Artificial Sequence
  source: /note="Description of Artificial Sequence: Synthetic polypeptide"
DVVMTQTPSPVSAAVGGTVTINCWFQQKPGQPPKLLIYGVPSRFKGSGSGTQFTLTINGVQCDDAATYYC

SEQ ID NO: 433 - protein, 70 aa, Artificial Sequence; identical to SEQ ID NO: 416
  source: /note="Description of Artificial Sequence: Synthetic polypeptide"

SEQ ID NO: 434 - protein, 70 aa, Artificial Sequence; identical to SEQ ID NO: 431
  source: /note="Description of Artificial Sequence: Synthetic polypeptide"

SEQ ID NO: 435 - protein, 70 aa, Artificial Sequence
  source: /note="Description of Artificial Sequence: Synthetic polypeptide"
DPMLTQTASPVSAAVGGTVTINCWYQQKPGQPPKLLIYGVPSRFKGSGSGTQFTLTINGVQCDDAATYYC

SEQ ID NO: 436 - protein, 70 aa, Artificial Sequence
  source: /note="Description of Artificial Sequence: Synthetic polypeptide"
YVMMTQTPSSVSEAVGGTVTIYCWYQQKPGQPPKLLIYGVPSRFKGSGSGTEYTLTISGVQCDDAATYYC

SEQ ID NO: 437 - protein, 70 aa, Artificial Sequence
  source: /note="Description of Artificial Sequence: Synthetic polypeptide"
DPMLTQTASPVSAAVGGTVTINCWYQQKPGQPPKLLIYGVPSRFSGSGSGTQFTLTISGVQCDDAATYYC

SEQ ID NO: 438 - protein, 70 aa, Artificial Sequence
  source: /note="Description of Artificial Sequence: Synthetic polypeptide"
DVVMTQTPSPVSAAVGGTVTINCWYQQKPGQPPKLLIYGVPSRFKGSGSGTQFTLTINGVQCDDAATYYC

SEQ ID NO: 439 - protein, 70 aa, Artificial Sequence; identical to SEQ ID NO: 416
  source: /note="Description of Artificial Sequence: Synthetic polypeptide"

SEQ ID NO: 440 - protein, 70 aa, Artificial Sequence
  source: /note="Description of Artificial Sequence: Synthetic polypeptide"
DIVLTQTASPVSAAVGSTVTISCWFQQKPGQPPKLLIYGVPSRFKGSGSGTQFTLTINGVQCDDAATYYC

SEQ ID NO: 441 - protein, 70 aa, Artificial Sequence
  source: /note="Description of Artificial Sequence: Synthetic polypeptide"
AVVLTQTASPVSAAVGGTVTINCWYQQKPGQRPKLLIYGVPSRFKGSGSGTQFTLTISGVQCDDAATYYC

SEQ ID NO: 442 - protein, 70 aa, Artificial Sequence
  source: /note="Description of Artificial Sequence: Synthetic polypeptide"
DPMLTQTASPVSAAVGSTVTISCWYQQKPGQPPKLLIYGVPSRFSGSGSGTQFTLTISGVQCDDAATYYC

SEQ ID NO: 443 - protein, 70 aa, Artificial Sequence
  source: /note="Description of Artificial Sequence: Synthetic polypeptide"
DVVMTQTPSPVSAAVGGTVTINCWYQQKPGQPPKLLIYGVPSRFSGSGSGTEFTLTISDLECADAATYYC

SEQ ID NO: 444 - protein, 70 aa, Artificial Sequence
  source: /note="Description of Artificial Sequence: Synthetic polypeptide"
DVVMTQTPSPVSAAVGGTVTINCWYQQKPGQPPKLLIYGVPSRFRGSGSGTQFTLTISGMKAEDVATYYC

SEQ ID NO: 445 - protein, 70 aa, Artificial Sequence
  source: /note="Description of Artificial Sequence: Synthetic polypeptide"
DVVMTQTPSPVSAAVGGTVTINCWYQQKPGQPPKLLIYGVPSRFKGSRSGTEFTLTISDLECADAATYYC

SEQ ID NO: 446 - protein, 70 aa, Artificial Sequence
  source: /note="Description of Artificial Sequence: Synthetic polypeptide"
DVVMTQTPSPVSAAVGGTVTINCWYQQKPGQPPKLLIYGVPSRFKGSGSGTQFTLTISDLECADAATYYC

SEQ ID NO: 447 - protein, 70 aa, Artificial Sequence; identical to SEQ ID NO: 415
  source: /note="Description of Artificial Sequence: Synthetic polypeptide"

SEQ ID NO: 448 - protein, 70 aa, Artificial Sequence; identical to SEQ ID NO: 420
  source: /note="Description of Artificial Sequence: Synthetic polypeptide"

SEQ ID NO: 449 - protein, 70 aa, Artificial Sequence; identical to SEQ ID NO: 417
  source: /note="Description of Artificial Sequence: Synthetic polypeptide"

SEQ ID NO: 450 - protein, 70 aa, Artificial Sequence
  source: /note="Description of Artificial Sequence: Synthetic polypeptide"
DPMLTQTPSPVSAAVGGTVTINCWYQQKPGQPPKLLIYGVPPRFKGSGSGTEFTLTISDLECADAATYYC

SEQ ID NO: 451 - protein, 70 aa, Artificial Sequence
  source: /note="Description of Artificial Sequence: Synthetic polypeptide"
AAVLTQTPSPVSVAVGGTVTINCWFQQKPGQPPKLLIYGVSSRFKGSGSGTQFTLTISGVQPGDAATYYC

SEQ ID NO: 452 - protein, 70 aa, Artificial Sequence
  source: /note="Description of Artificial Sequence: Synthetic polypeptide"
DPMLTQTASPVSAAVGSTVTISCWYQQKPGQPPKLLIYGVPSRFSGSGSGTEYTLTISGVQCDDAATYYC

SEQ ID NO: 453 - protein, 70 aa, Artificial Sequence
  source: /note="Description of Artificial Sequence: Synthetic polypeptide"
DPVLTQTASPVSAAVGGTVTISCWFQQKPGQPPKLLIYGVSSRFKGSGSGTQFTLTISGVQCDDAATYYC

SEQ ID NO: 454 - protein, 70 aa, Artificial Sequence
  source: /note="Description of Artificial Sequence: Synthetic polypeptide"
AIKMTQTPSSVSAAVGGTVTINCWYQQKPGQPPKLLIYGVPSRFKGSGSGTQFTLTINGVQCDDAATYYC

SEQ ID NO: 455 - protein, 70 aa, Artificial Sequence; identical to SEQ ID NO: 425
  source: /note="Description of Artificial Sequence: Synthetic polypeptide"

SEQ ID NO: 456 - protein, 70 aa, Artificial Sequence
  source: /note="Description of Artificial Sequence: Synthetic polypeptide"
DPVLTQTPSSACEPVGGTVTIKCWYQQKPGQSPKLLIYGVPSRFKGSGSGTEYTLTISDLECADAATYYC

SEQ ID NO: 457 - protein, 70 aa, Artificial Sequence; identical to SEQ ID NO: 425
  source: /note="Description of Artificial Sequence: Synthetic polypeptide"

SEQ ID NO: 458 - protein, 70 aa, Artificial Sequence
  source: /note="Description of Artificial Sequence: Synthetic polypeptide"
YVMMTQTPSSVSEAVGGTVTIYCWYQQKPGQPPKLLIYGVPSRFKGSGSGTQFTLTINGVQCDDAATYYC

SEQ ID NO: 459 - protein, 70 aa, Artificial Sequence
  source: /note="Description of Artificial Sequence: Synthetic polypeptide"
DPMLTQTASPVSAAVGGTVTISCWYQQKPGQPPKLLIYGVPSRFKGSGSGTQFTLTINGVQCDDAATYYC

SEQ ID NO: 460 - protein, 70 aa, Artificial Sequence
  source: /note="Description of Artificial Sequence: Synthetic polypeptide"
YVMMTQTPSSVSEAVGGTVTISCWFQQKPGQPPKLLIYGVPSRFKGSGSGTQFTLTINGVQCDDAATYYC

SEQ ID NO: 461 - protein, 70 aa, Artificial Sequence
  source: /note="Description of Artificial Sequence: Synthetic polypeptide"
DVVMTQTPSPVSAAVGSTVTISCWFQQKPGQPPKLLIYGVPSRFKGSGSGTQFTLTISGVQCDDAATYYC

SEQ ID NO: 462 - protein, 70 aa, Artificial Sequence
  source: /note="Description of Artificial Sequence: Synthetic polypeptide"
DPMLTQTASPVSAAVGSTVTISCWFQQKPGQPPKLLIYGVPSRFSGSGSGTQFTLTISGVQCDDAATYYC

SEQ ID NO: 463 - protein, 70 aa, Artificial Sequence
  source: /note="Description of Artificial Sequence: Synthetic polypeptide"
DPVLTQTASPVSAAVGGTVTISCWFQQKPGQPPKLLIYGVPSRFKGSGSGTQFTLTINGVQCDDAATYYC

SEQ ID NO: 464 - protein, 70 aa, Artificial Sequence
  source: /note="Description of Artificial Sequence: Synthetic polypeptide"
DPMLTQTASPVSAAVGSTVTISCWFQQKPGQPPKLLIYGVPSWVSSSGSGTEFTLTISGVQPGDAATYYC

SEQ ID NO: 465 - protein, 70 aa, Artificial Sequence; identical to SEQ ID NO: 415
  source: /note="Description of Artificial Sequence: Synthetic polypeptide"

SEQ ID NO: 466 - protein, 70 aa, Artificial Sequence
  source: /note="Description of Artificial Sequence: Synthetic polypeptide"
AAVLTQTPSPVSVAVGGTVTISCWYQQKPGQPPKLLIYGVSSRFKGSGSGTQFTLTISGVQCDDAATYYC

SEQ ID NO: 467 - protein, 70 aa, Artificial Sequence
  source: /note="Description of Artificial Sequence: Synthetic polypeptide"
DPVLTQTPSPVSVAVGGTVTINCWFQQKPGQPPKLLIYGVSSRFKGSGSGTQFTLTISGVQCDDAATYYC

SEQ ID NO: 468 - protein, 70 aa, Artificial Sequence
  source: /note="Description of Artificial Sequence: Synthetic polypeptide"
ALVMTQTPSSTSEPVGGTVTINCWFQQKPGQPPKLLIYGVSSRFKGSGSGTQFTLTISGVQCDDAATYYC

SEQ ID NO: 469 - protein, 70 aa, Artificial Sequence
  source: /note="Description of Artificial Sequence: Synthetic polypeptide"
DVVMTQTASPVSAAVGSTVTISCWFQQKPGQPPKLLIYGVPSRFKGSGSGTQFTLTINGVQCDDAATYYC

SEQ ID NO: 470 - protein, 70 aa, Artificial Sequence
  source: /note="Description of Artificial Sequence: Synthetic polypeptide"
AAVLTQTPSPVSVAVGGTVTINCWFQQKPGQPPKLLIYGVPSRFKGSGSGTQFTLTINGVQCDDAATYYC

SEQ ID NO: 471 - protein, 70 aa, Artificial Sequence; identical to SEQ ID NO: 463
  source: /note="Description of Artificial Sequence: Synthetic polypeptide"

SEQ ID NO: 472 - protein, 70 aa, Artificial Sequence
  source: /note="Description of Artificial Sequence: Synthetic polypeptide"
YVMMTQTPSSVSEAVGGTVTIYCWYQQKPGQPPKLLIYGVPSRFRGSGSGTQFTLTINGVQCDDAATYYC

SEQ ID NO: 473 - protein, 70 aa, Artificial Sequence
  source: /note="Description of Artificial Sequence: Synthetic polypeptide"
DPMLTQTASPVSAAVGSTVTISCWFQQKPGQPRKLLIYGVPSRFKGSGSGTQFTLTINGVQCDDAATYYC

SEQ ID NO: 474 - protein, 70 aa, Artificial Sequence
  source: /note="Description of Artificial Sequence: Synthetic polypeptide"
DVVMTQTPSSKSAAVGDTVTIKCWYQQKPGQPPKLLIYGVPSRFKGSGSGTQFTLTINGVQCDDAATYYC

SEQ ID NO: 475 - protein, 70 aa, Artificial Sequence
  source: /note="Description of Artificial Sequence: Synthetic polypeptide"
AAVLTQTPSPVSVAVGGTVTINCWFQQKPGQPPKLLIYGVSSRFKGSGSGTQFTLTINGVQCDDAATYYC

SEQ ID NO: 476 - protein, 94 aa, Artificial Sequence
  source: /note="Description of Artificial Sequence: Synthetic polypeptide"
QSVKESGGRLVTPGTPLTLTCTVSGFSLNSYAMIWVRQAPGEGLEYIGFITTGGTTYYASWAKGRFTISRTSTTVDLKLTRPTTEDTATYFCAR

SEQ ID NO: 477 - protein, 98 aa, Artificial Sequence
  source: /note="Description of Artificial Sequence: Synthetic polypeptide"
QVQLVESGGGLVQPGGSLRLSCSASGFTFSSYAMHWVRQAPGKGLEYVSAISSNGGSTYYADSVKGRFTISRDNSKNTLYLQMNSLRAEDTAVYYCAR

SEQ ID NO: 478 - protein, 95 aa, Artificial Sequence
  source: /note="Description of Artificial Sequence: Synthetic polypeptide"
ESGGGLVQPGRSLRLSCTASGFTFGDYAMSWVRQAPGKGLEWVGFIRSKAYGGTTEYAASVKGRFTISRDDSKSIAYLQMNSLKTEDTAVYYCTR

SEQ ID NO: 479 - protein, 93 aa, Artificial Sequence
  source: /note="Description of Artificial Sequence: Synthetic polypeptide"
ESGGGLVQPGGSLRLSCAASGFTFSSYAMHWVRQAPGKGLEYVSAISSNGGSTYYANSVKGRFTISRDNSKNTLYLQMGSLRAEDMAVYYCAR

SEQ ID NO: 480 - protein, 95 aa, Artificial Sequence
  source: /note="Description of Artificial Sequence: Synthetic polypeptide"
ELVMTQTPSSVSAAVGGTVTINCQASQSISSYLAWYQQKPGQPPKLLIYYASTLASGVPSRFKGSGSGTEFTLTITGVQCDDAATYYCLGVYGYS

SEQ ID NO: 481 - protein, 95 aa, Artificial Sequence
  source: /note="Description of Artificial Sequence: Synthetic polypeptide"
DIQMTQSPSTLSASVGDRVTITCRASQSISSWLAWYQQKPGKAPKLLIYKASSLESGVPSRFSGSGSGTEFTLTISSLQPDDFATYYCQQYNSYS

SEQ ID NO: 482 - protein, 95 aa, Artificial Sequence; identical to SEQ ID NO: 404
  source: /note="Description of Artificial Sequence: Synthetic polypeptide"

SEQ ID NO: 483 - protein, 91 aa, Artificial Sequence
  source: /note="Description of Artificial Sequence: Synthetic polypeptide"
MTQSPSSFSASTGDRVTITCRASQGISSYLAWYQQKPGKAPKLLIYAASTLQSGVPSRFSGSGSGTDFTLTISCLQSEDFATYYCQQYYSY

SEQ ID NO: 484 - protein, 111 aa, Artificial Sequence
  source: /note="Description of Artificial Sequence: Synthetic polypeptide"
ELVMTQTPSSVSAAVGGTVTINCQASQSISSYLAWYQQKPGQPPKLLIYYASTLASGVPSRFKGSGSGTEFTLTITGVQCDDAATYYCLGVYGYSFDDGIAFGGGTELEIK

SEQ ID NO: 485 - protein, 111 aa, Artificial Sequence
  source: /note="Description of Artificial Sequence: Synthetic polypeptide"
DIQMTQSPSTLSASVGDRVTITCQASQSISSYLAWYQQKPGKAPKLLIYYASTLASGVPSRFSGSGSGTEFTLTISSLQCDDFATYYCLGVYGYSFDDGIAFGGGTKVEIK

SEQ ID NO: 486 - protein, 111 aa, Artificial Sequence
  source: /note="Description of Artificial Sequence: Synthetic polypeptide"
ELVMTQTPSYTSAAVGDTVTIKCQASQTIGGSDLSWYQQKPGQPPKLLIWYATNLPSGVPSRFSGSRSGTEYTLTISGVQCEDAATYYCLGGYAAASYRTAFGGGTEVVVK

SEQ ID NO: 487 - protein, 111 aa, Artificial Sequence
  source: /note="Description of Artificial Sequence: Synthetic polypeptide"
DIQMTQSPSFLSASVGDRVTITCQASQTIGGSDLSWYQQKPGKAPKLLIYYATNLPSGVPSRFSGSGSGTDFTLTISSLQCEDFATYYCLGGYAAASYRTAFGGGTKVEIK

SEQ ID NO: 488 - protein, 111 aa, Artificial Sequence
  source: /note="Description of Artificial Sequence: Synthetic polypeptide"
ELVMTQTPSSVSAAVGGTVTINCQASQSISNYLSWYQQKPGQPPKLLIFAASKLASWVPKRFSGSRSGIEYTLTISGVQCDDAATYFCLGVYSISTDDGAAFGGGTEVVVK

SEQ ID NO: 489 - protein, 111 aa, Artificial Sequence
  source: /note="Description of Artificial Sequence: Synthetic polypeptide"
DIQMTQSPSSLSASVGDRVTITCQASQSISNYLSWYQQKPGKAPKLLIYAASKLASGVPSRFSGSGSGTDFTLTISSLQCEDFATYYCLGVYSISTDDGAAFGGGTKVEIK

SEQ ID NO: 490 - protein, 112 aa, Artificial Sequence
  source: /note="Description of Artificial Sequence: Synthetic polypeptide"
EVLMTQTPSSVSAAVGDTVTIKCQASQSISSVLSWYQQKPGQPPKLLIYLASTLASGVPSRFSGSRSGTEFTLTISDLECDDAATYYCQTNYGTSSSNYGFAFGGGTEVVVK

SEQ ID NO: 491 - protein, 112 aa, Artificial Sequence
  source: /note="Description of Artificial Sequence: Synthetic polypeptide"
DIQMTQSPSSLSASVGDRVTITCQASQSISSVLSWYQQKPGKAPKLLIYLASTLASGVPSRFSGSGSGTDFTLTISSLQPEDFATYYCQTNYGTSSSNYGFAFGGGTKVEIK